European Patent Specification EP 3 578 664 B1, published October 30, 2024. Title: Fibrosis Biomarker Assay. Applicant: Nordic Bioscience A/S. Application US 12/749652. The sequence listing filed with the application follows.

SEQUENCE LISTING (2248 sequences)

SEQ ID NO: 1 - protein, 10 aa, Homo sapiens
PGIPGRNGDP

SEQ ID NO: 2 - protein, 10 aa, Homo sapiens
ESCPTGPQNY

SEQ ID NO: 3 - protein, 10 aa, Homo sapiens
PKGDTGPRGP

SEQ ID NO: 4 - protein, 25 aa, Homo sapiens
  MOD_RES (16)..(17): proline or hydroxyproline
  MOD_RES (20)..(20): proline or hydroxyproline
VPGPMGPSGPRGLPGXXGAXGPQGF

SEQ ID NO: 5 - protein, 26 aa, Homo sapiens
  MOD_RES (17)..(18): proline or hydroxyproline
  MOD_RES (21)..(21): proline or hydroxyproline
SVPGPMGPSGPRGLPGXXGAXGPQGF

SEQ ID NO: 6 - protein, 28 aa, Homo sapiens
  MOD_RES (8)..(8): methionine or oxidised methionine
  MOD_RES (19)..(20): proline or hydroxyproline
  MOD_RES (23)..(23): proline or hydroxyproline
GISVPGPXGPSGPRGLPGXXGAXGPQGF

SEQ ID NO: 7 - protein, 29 aa, Homo sapiens
  MOD_RES (23)..(24): proline or hydroxy proline
  MOD_RES (26)..(26): proline or hydroxy proline
GFQGPPGEPGEPGASGPMGPRGXXGXPGK

SEQ ID NO: 8 - protein, 25 aa, Homo sapiens
  MOD_RES (5)..(5): methionine or oxidised methionine
  MOD_RES (17)..(17): proline or hydroxyproline
  MOD_RES (20)..(20): proline or hydroxyproline
VPGPXGPSGPRGLPGPXGAXGPQGF

SEQ ID NO: 9 - protein, 37 aa, Homo sapiens
  MOD_RES (17)..(17): lysine or hydroxylysine
  MOD_RES (23)..(23): proline or hydroxyproline
  MOD_RES (29)..(29): proline or hydroxyproline
FSGLDGAKGDAGPAGPXGEPGSXGENGAXGQMGPRGL

SEQ ID NO: 10 - protein, 17 aa, Homo sapiens
  MOD_RES (3)..(3): proline or hydroxyproline
  MOD_RES (9)..(9): proline or hydroxyproline
  MOD_RES (12)..(12): proline or hydroxyproline
GLXGERGRXGAXGPAGA

SEQ ID NO: 11 - protein, 23 aa, Homo sapiens
  MOD_RES (6)..(6): proline or hydroxyproline
  MOD_RES (9)..(9): proline or hydroxyproline
  MOD_RES (20)..(20): proline or hydroxyproline
GLTGSXGSXGPDGKTGPPGXAGQ

SEQ ID NO: 12 - protein, 31 aa, Homo sapiens
  MOD_RES (5)..(5): proline or hydroxyproline
  MOD_RES (14)..(14): proline or hydroxyproline
  MOD_RES (20)..(20): proline or hydroxyproline
  MOD_RES (26)..(26): proline or hydroxyproline
ERGSXGPAGPKGSXGEAGRXGEAGLXGAKGL

SEQ ID NO: 13 - protein, 32 aa, Homo sapiens
  MOD_RES (6)..(6): proline or hydroxyproline
  MOD_RES (8)..(8): proline or hydroxyproline
  MOD_RES (21)..(21): proline or hydroxyproline
  MOD_RES (27)..(27): proline or hydroxyproline
  MOD_RES (31)..(31): proline or hydroxyproline
GERGSXGXAGPKGSPGEAGRXGEAGLXGAKGL

SEQ ID NO: 14 - protein, 23 aa, Homo sapiens
  MOD_RES (6)..(6): proline or hydroxyproline
  MOD_RES (9)..(9): proline or hydroxyproline
  MOD_RES (20)..(20): proline or hydroxyproline
GLTGSXGSXGPDGKTGPPGXAGQ

SEQ ID NO: 15 - protein, 35 aa, Homo sapiens
GLTGSPGSPGPDGKTGPPGPAGQDGRPGPPGPPGA

SEQ ID NO: 16 - protein, 38 aa, Homo sapiens
GLTGSPGSPGPDGKTGPPGPAGQDGRPGPPGPPGARGQ

SEQ ID NO: 17 - protein, 17 aa, Homo sapiens
GQDGRPGPPGPPGARGQ

SEQ ID NO: 18 - protein, 38 aa, Homo sapiens; identical to SEQ ID NO: 16

SEQ ID NO: 19 - protein, 33 aa, Homo sapiens
  MOD_RES (12)..(12): proline or hydroxyproline
  MOD_RES (30)..(30): proline or hydroxyproline
GKDGEAGAQGPXGPAGPAGERGEQGPAGSXGFQ

SEQ ID NO: 20 - protein, 15 aa, Homo sapiens
  MOD_RES (12)..(12): proline or hydroxyproline
GERGEQGPAGSXGFQ

SEQ ID NO: 21 - protein, 47 aa, Homo sapiens
  MOD_RES (5)..(5): proline or hydroxyproline
  MOD_RES (7)..(7): proline or hydroxyproline
  MOD_RES (40)..(40): proline or hydroxyproline
  MOD_RES (44)..(44): proline or hydroxyproline
ERGVXGXPGAVGPAGKDGEAGAQGPPGPAGPAGERGEQGXAGSXGFQ

SEQ ID NO: 22 - protein, 10 aa, Homo sapiens
PKGDTGPRGP

SEQ ID NO: 23 - protein, 6 aa, Homo sapiens
ISVPGP

SEQ ID NO: 24 - protein, 6 aa, Homo sapiens
VPGPMG

SEQ ID NO: 25 - protein, 6 aa, Homo sapiens
PGPMGP

SEQ ID NO: 26 - protein, 6 aa, Homo sapiens
LPGPGG

SEQ ID NO: 27 - protein, 6 aa, Homo sapiens
FQGPPG

SEQ ID NO: 28 - protein, 6 aa, Homo sapiens
KNGDDG

SEQ ID NO: 29 - protein, 6 aa, Homo sapiens
ARGLPG

SEQ ID NO: 30 - protein, 6 aa, Homo sapiens
SGLDGA

SEQ ID NO: 31 - protein, 6 aa, Homo sapiens
LDGAKG

SEQ ID NO: 32 - protein, 6 aa, Homo sapiens
LPGERG

SEQ ID NO: 33 - protein, 6 aa, Homo sapiens
VRGEPG

SEQ ID NO: 34 - protein, 6 aa, Homo sapiens
PGAKGA

SEQ ID NO: 35 - protein, 6 aa, Homo sapiens
GGPPGP

SEQ ID NO: 36 - protein, 6 aa, Homo sapiens
NSGEPG

SEQ ID NO: 37 - protein, 6 aa, Homo sapiens
DGVAGP

SEQ ID NO: 38 - protein, 6 aa, Homo sapiens
ERGSPG

SEQ ID NO: 39 - protein, 6 aa, Homo sapiens
LTGSPG

SEQ ID NO: 40 - protein, 6 aa, Homo sapiens
QDGRPG

SEQ ID NO: 41 - protein, 6 aa, Homo sapiens
RGVPGP

SEQ ID NO: 42 - protein, 6 aa, Homo sapiens
VGPAGK

SEQ ID NO: 43 - protein, 6 aa, Homo sapiens
ERGEQG

SEQ ID NO: 44 - protein, 6 aa, Homo sapiens
RGEQGP

SEQ ID NO: 45 - protein, 6 aa, Homo sapiens
PGERGV

SEQ ID NO: 46 - protein, 6 aa, Homo sapiens
ANGAPG

SEQ ID NO: 47 - protein, 6 aa, Homo sapiens
ARGAPG

SEQ ID NO: 48 - protein, 6 aa, Homo sapiens
PGDRGE

SEQ ID NO: 49 - protein, 6 aa, Homo sapiens
AKGDAG

SEQ ID NO: 50 - protein, 6 aa, Homo sapiens
PIGNVG

SEQ ID NO: 51 - protein, 6 aa, Homo sapiens
AAGRVG

SEQ ID NO: 52 - protein, 6 aa, Homo sapiens
  MOD_RES (2)..(2): proline or hydroxyproline
  MOD_RES (4)..(4): proline or hydroxyproline
PXGXAG

SEQ ID NO: 53 - protein, 6 aa, Homo sapiens
GADGPA

SEQ ID NO: 54 - protein, 6 aa, Homo sapiens
GPQGIA

SEQ ID NO: 55 - protein, 6 aa, Homo sapiens
GQRGVV

SEQ ID NO: 56 - protein, 6 aa, Homo sapiens
QRGVVG

SEQ ID NO: 57 - protein, 6 aa, Homo sapiens
GLPGQR

SEQ ID NO: 58 - protein, 6 aa, Homo sapiens
PGLPGP

SEQ ID NO: 59 - protein, 6 aa, Homo sapiens
PMGPPG

SEQ ID NO: 60 - protein, 6 aa, Homo sapiens
MGPPGL

SEQ ID NO: 61 - protein, 6 aa, Homo sapiens
DKGETG

SEQ ID NO: 62 - protein, 6 aa, Homo sapiens
  MOD_RES (5)..(5): proline or hydroxyproline
LQGPXG

SEQ ID NO: 63 - protein, 6 aa, Homo sapiens
SAGAPG

SEQ ID NO: 64 - protein, 6 aa, Homo sapiens
RTGDAG

SEQ ID NO: 65 - protein, 5 aa, Homo sapiens
FDFSF

SEQ ID NO: 66 - protein, 5 aa, Homo sapiens
FDFSF

SEQ ID NO: 67 - protein, 6 aa, Homo sapiens
ATGAAG

SEQ ID NO: 68 - protein, 6 aa, Homo sapiens
AKGEAG

SEQ ID NO: 69 - protein, 6 aa, Homo sapiens
GIAGAP

SEQ ID NO: 70 - protein, 6 aa, Homo sapiens
IAGAPG

SEQ ID NO: 71 - protein, 6 aa, Homo sapiens
VQGPPG

SEQ ID NO: 72 - protein, 6 aa, Homo sapiens
  MOD_RES (4)..(5): proline or hydroxproline
LPGXXG

SEQ ID NO: 73 - protein, 6 aa, Homo sapiens
AGPKGS

SEQ ID NO: 74 - protein, 6 aa, Homo sapiens
RGSPGP

SEQ ID NO: 75 - protein, 6 aa, Homo sapiens
FAGPPG

SEQ ID NO: 76 - protein, 6 aa, Homo sapiens
QAGVMG

SEQ ID NO: 77 - protein, 6 aa, Homo sapiens
ARGQAG

SEQ ID NO: 78 - protein, 6 aa, Homo sapiens
NVGAPG

SEQ ID NO: 79 - protein, 6 aa, Homo sapiens
PAGERG

SEQ ID NO: 80 - protein, 6 aa, Homo sapiens
KDGEAG

SEQ ID NO: 81 - protein, 6 aa, Homo sapiens
GEVGPP

SEQ ID NO: 82 - protein, 6 aa, Homo sapiens
ARGERG

SEQ ID NO: 83 - protein, 6 aa, Homo sapiens
QGLPGP

SEQ ID NO: 84 - protein, 6 aa, Homo sapiens
IAGQRG

SEQ ID NO: 85 - protein, 6 aa, Homo sapiens
LTGPIG

SEQ ID NO: 86 - protein, 6 aa, Homo sapiens
AGLPGP

SEQ ID NO: 87 - protein, 6 aa, Homo sapiens
RGVVGL

SEQ ID NO: 88 - protein, 6 aa, Homo sapiens
AGPPGA

SEQ ID NO: 89 - protein, 6 aa, Homo sapiens
LAGPPG

SEQ ID NO: 90 - protein, 6 aa, Homo sapiens
EPGKQG

SEQ ID NO: 91 - protein, 6 aa, Homo sapiens
ATGFPG

SEQ ID NO: 92 - protein, 6 aa, Homo sapiens
PSGASG

SEQ ID NO: 93 - protein, 6 aa, Homo sapiens
GKQGPS

SEQ ID NO: 94 - protein, 6 aa, Homo sapiens
GPPGPA

SEQ ID NO: 95 - protein, 6 aa, Homo sapiens
AGQRGV

SEQ ID NO: 96 - protein, 6 aa, Homo sapiens
ARGPAG

SEQ ID NO: 97 - protein, 6 aa, Homo sapiens
ASGPAG

SEQ ID NO: 98 - protein, 6 aa, Homo sapiens
VVGLPG

SEQ ID NO: 99 - protein, 6 aa, Homo sapiens
VGPPGP

SEQ ID NO: 100 - protein, 6 aa, Homo sapiens
  MOD_RES (2)..(2): proline or hydroxyproline
  MOD_RES (5)..(5): proline or hydroxyproline
  MOD_RES (6)..(6): proline or hydroxyproline
GXPGXX

SEQ ID NO: 101 - protein, 6 aa, Homo sapiens
QLSYGY

SEQ ID NO: 102 - protein, 6 aa, Homo sapiens
EKSTGG

SEQ ID NO: 103 - protein, 6 aa, Homo sapiens
PPGPQG

SEQ ID NO: 104 - protein, 6 aa, Homo sapiens
KGHRGF

SEQ ID NO: 105 - protein, 6 aa, Homo sapiens
PSGPRG

SEQ ID NO: 106 - protein, 6 aa, Homo sapiens
APGPQG

SEQ ID NO: 107 - protein, 6 aa, Homo sapiens
APGPAG

SEQ ID NO: 108 - protein, 6 aa, Homo sapiens
FPGAVG

SEQ ID NO: 109 - protein, 6 aa, Homo sapiens
SEGPQG

SEQ ID NO: 110 - protein, 6 aa, Homo sapiens
GANGAP

SEQ ID NO: 111 - protein, 6 aa, Homo sapiens
GARGLA

SEQ ID NO: 112 - protein, 6 aa, Homo sapiens
SGPQGP

SEQ ID NO: 113 - protein, 6 aa, Homo sapiens
EPGPVG

SEQ ID NO: 114 - protein, 6 aa, Homo sapiens
EPGPTG

SEQ ID NO: 115 - protein, 6 aa, Homo sapiens
RGFPGA

SEQ ID NO: 116 - protein, 6 aa, Homo sapiens
KGPAGE

SEQ ID NO: 117 - protein, 6 aa, Homo sapiens
IPGAPG

SEQ ID NO: 118 - protein, 6 aa, Homo sapiens
LPGAKG

SEQ ID NO: 119 - protein, 6 aa, Homo sapiens
  MOD_RES (1)..(2): proline or hydroxyproline
  MOD_RES (4)..(5): proline or hydroxyproline
XXGXXG

SEQ ID NO: 120 - protein, 6 aa, Homo sapiens
PPGARG

SEQ ID NO: 121 - protein, 6 aa, Homo sapiens
PGKAGE

SEQ ID NO: 122 - protein, 6 aa, Homo sapiens
AVGPAG

SEQ ID NO: 123 - protein, 6 aa, Homo sapiens
PAGPAG

SEQ ID NO: 124 - protein, 6 aa, Homo sapiens
AGPAGE

SEQ ID NO: 125 - protein, 6 aa, Homo sapiens
APGPDG

SEQ ID NO: 126 - protein, 6 aa, Homo sapiens
RGERGF

SEQ ID NO: 127 - protein, 6 aa, Homo sapiens
PAGPRG

SEQ ID NO: 128 - protein, 6 aa, Homo sapiens
KDGVRG

SEQ ID NO: 129 - protein, 6 aa, Homo sapiens
PAGPTG

SEQ ID NO: 130 - protein, 6 aa, Homo sapiens
TGARGA

SEQ ID NO: 131 - protein, 6 aa, Homo sapiens
PGPAGF

SEQ ID NO: 132 - protein, 6 aa, Homo sapiens
EPGDAG

SEQ ID NO: 133 - protein, 6 aa, Homo sapiens
PAGPPG

SEQ ID NO: 134 - protein, 6 aa, Homo sapiens
SAGPPG

SEQ ID NO: 135 - protein, 6 aa, Homo sapiens
DGTSGH

SEQ ID NO: 136 - protein, 6 aa, Homo sapiens
NAGPPG

SEQ ID NO: 137 - protein, 6 aa, Homo sapiens
FRGPAG

SEQ ID NO: 138 - protein, 6 aa, Homo sapiens
GEKGSP

SEQ ID NO: 139 - protein, 6 aa, Homo sapiens
GAPGTP

SEQ ID NO: 140 - protein, 6 aa, Homo sapiens
PGPQGI

SEQ ID NO: 141 - protein, 6 aa, Homo sapiens
PQGIAG

SEQ ID NO: 142 - protein, 6 aa, Homo sapiens
AIGSPG

SEQ ID NO: 143 - protein, 6 aa, Homo sapiens
QPGVMG

SEQ ID NO: 144 - protein, 6 aa, Homo sapiens
AGPPGM

SEQ ID NO: 145 - protein, 6 aa, Homo sapiens
GPSGEP

SEQ ID NO: 146 - protein, 6 aa, Homo sapiens
ERGPPG

SEQ ID NO: 147 - protein, 6 aa, Homo sapiens
RGPPGP

SEQ ID NO: 148 - protein, 6 aa, Homo sapiens
PVGPVG

SEQ ID NO: 149 - protein, 6 aa, Homo sapiens
PQGPRG

SEQ ID NO: 150 - protein, 6 aa, Homo sapiens
HRGFSG

SEQ ID NO: 151 - protein, 6 aa, Homo sapiens
EQGPSG

SEQ ID NO: 152 - protein, 6 aa, Homo sapiens
PRGPPG

SEQ ID NO: 153 - protein, 6 aa, Homo sapiens
PPGPRG

SEQ ID NO: 154 - protein, 6 aa, Homo sapiens
  MOD_RES (2)..(2): Hydroxyproline
  MOD_RES (5)..(6): Hydroxyproline
VGGLAG

SEQ ID NO: 155 - protein, 6 aa, Homo sapiens
GPPSAG

SEQ ID NO: 156 - protein, 6 aa, Homo sapiens
PPSAGF

SEQ ID NO: 157 - skipped

SEQ ID NO: 158 - protein, 6 aa, Homo sapiens
VKGERG

SEQ ID NO: 159 - protein, 6 aa, Homo sapiens
TPGPQG

SEQ ID NO: 160 - protein, 6 aa, Homo sapiens
QMGPRG

SEQ ID NO: 161 - protein, 6 aa, Homo sapiens
PGPPGA

SEQ ID NO: 162 - protein, 6 aa, Homo sapiens
QGIAGQ

SEQ ID NO: 163 - protein, 6 aa, Homo sapiens
PGADGQ

SEQ ID NO: 164 - protein, 6 aa, Homo sapiens
AGSPGF

SEQ ID NO: 165 - protein, 6 aa, Homo sapiens
LPGPSG

SEQ ID NO: 166 - protein, 6 aa, Homo sapiens
PPGPKG

SEQ ID NO: 167 - protein, 6 aa, Homo sapiens
PGERGA

SEQ ID NO: 168 - protein, 6 aa, Homo sapiens
IKGPAG

SEQ ID NO: 169 - protein, 6 aa, Homo sapiens
PKGPAG

SEQ ID NO: 170 - protein, 6 aa, Homo sapiens
GRNGDP

SEQ ID NO: 171 - protein, 6 aa, Homo sapiens
SPGEQG

SEQ ID NO: 172 - protein, 6 aa, Homo sapiens
GPAGRP

SEQ ID NO: 173 - protein, 6 aa, Homo sapiens
  MOD_RES (2)..(2): proline or hydroxyproline
PXGPIG

SEQ ID NO: 174 - protein, 6 aa, Homo sapiens
TGDAGP

SEQ ID NO: 175 - protein, 6 aa, Homo sapiens
LSGERG

SEQ ID NO: 176 - protein, 6 aa, Homo sapiens
TGPRGP

SEQ ID NO: 177 - protein, 20 aa, Homo sapiens
AGIPGAPGLMGARGPPGPAG

SEQ ID NO: 178 - protein, 19 aa, Homo sapiens
KGDPGPPGIPGRNGDPGIP

SEQ ID NO: 179 - protein, 20 aa, Homo sapiens
GLAGPPGMPGPRGSPGPQGV

SEQ ID NO: 180 - protein, 21 aa, Homo sapiens
GERGLPGPPGIKGPAGIPGFP

SEQ ID NO: 181 - protein, 22 aa, Homo sapiens
GIAGITGARGLAGPPGMPGPRG

SEQ ID NO: 182 - protein, 23 aa, Homo sapiens
GIKGHRGFPGNPGAPGSPGPAGQ

SEQ ID NO: 183 - protein, 23 aa, Homo sapiens
ARGLAGPPGMPGPRGSPGPQGVK

SEQ ID NO: 184 - protein, 25 aa, Homo sapiens
ITGARGLAGPPGMPGPRGSPGPQGV

SEQ ID NO: 185 - protein, 26 aa, Homo sapiens
ITGARGLAGPPGMPGPRGSPGPQGVK

SEQ ID NO: 186 - protein, 26 aa, Homo sapiens
GITGARGLAGPPGMPGPRGSPGPQGV

SEQ ID NO: 187 - protein, 26 aa, Homo sapiens
GVKGESGKPGANGLSGERGPPGPQGL

SEQ ID NO: 188 - protein, 26 aa, Homo sapiens
GSRGAPGPQGPRGDKGETGERGAAGI

SEQ ID NO: 189 - protein, 28 aa, Homo sapiens
PKGDAGQPGEKGSPGAQGPPGAPGPLGI

SEQ ID NO: 190 - protein, 27 aa, Homo sapiens
GITGARGLAGPPGMPGPRGSPGPQGVK

SEQ ID NO: 191 - protein, 32 aa, Homo sapiens
GLRGGAGPPGPEGGKGAAGPPGPPGAAGTPGL

SEQ ID NO: 192 - protein, 35 aa, Homo sapiens
GHAGAQGPPGPPGINGSPGGKGEMGPAGIPGAPGL

SEQ ID NO: 193 - protein, 48 aa, Homo sapiens
AGKSGDRGESGPAGPAGAPGPAGSRGAPGPQGPRGDKGETGERGAAGI

SEQ ID NO: 194 - protein, 50 aa, Homo sapiens
GLQGLPGTGGPPGENGKPGEPGPKGDAGAPGAPGGKGDAGAPGERGPPGL

SEQ ID NO: 195 - protein, 21 aa, Homo sapiens
GERGLPGPPGIKGPAGIPGFP

SEQ ID NO: 196 - protein, 24 aa, Homo sapiens
AVGGLAGYPGPAGPPGPPGPPGTS

SEQ ID NO: 197 - protein, 24 aa, Homo sapiens
KDGTSGHPGPIGPPGPRGNRGERG

SEQ ID NO: 198 - protein, 29 aa, Homo sapiens
AVGGLAGYPGPAGPPGPPGPPGTSGHPGS

SEQ ID NO: 199 - protein, 29 aa, Homo sapiens
GIAGITGARGLAGPPGMPGPRGSPGPQGV

SEQ ID NO: 200 - protein, 31 aa, Homo sapiens
APGAPGGKGDAGAPGERGPPGLAGAPGLRGG

SEQ ID NO: 201 - protein, 32 aa, Homo sapiens
AVGGLAGYPGPAGPPGPPGPPGTSGHPGSPGS

SEQ ID NO: 202 - protein, 22 aa, Homo sapiens
AIGSPGPAGPRGPVGPSGPPGK

SEQ ID NO: 203 - protein, 23 aa, Homo sapiens
GAIGSPGPAGPRGPVGPSGPPGK

SEQ ID NO: 204 - protein, 15 aa, Homo sapiens
PAGQQGAIGSPGPAG

SEQ ID NO: 205 - protein, 20 aa, Homo sapiens
GGPPGVAGPPGGSGPAGPPG

SEQ ID NO: 206 - protein, 19 aa, Homo sapiens
LAGPPGMPGPRGSPGPQGV

SEQ ID NO: 207 - protein, 19 aa, Homo sapiens
GLSGERGPPGPQGLPGLAG

SEQ ID NO: 208 - protein, 21 aa, Homo sapiens
RGLAGPPGMPGPRGSPGPQGV

SEQ ID NO: 209 - protein, 21 aa, Homo sapiens
GLAGPPGMPGPRGSPGPQGVK

SEQ ID NO: 210 - protein, 22 aa, Homo sapiens
RGLAGPPGMPGPRGSPGPQGVK

SEQ ID NO: 211 - protein, 21 aa, Homo sapiens
GPQGPPGKNGETGPQGPPGPT

SEQ ID NO: 212 - protein, 22 aa, Homo sapiens
GVKGERGSPGGPGAAGFPGARG

SEQ ID NO: 213 - protein, 22 aa, Homo sapiens
ARGLAGPPGMPGPRGSPGPQGV

SEQ ID NO: 214 - protein, 23 aa, Homo sapiens
NGLSGERGPPGPQGLPGLAGTAG

SEQ ID NO: 215 - protein, 24 aa, Homo sapiens
AVGGLAGYPGPAGPPGPPGPPGTS

SEQ ID NO: 216 - protein, 24 aa, Homo sapiens
GSPGGKGEMGPAGIPGAPGLMGAR

SEQ ID NO: 217 - protein, 24 aa, Homo sapiens
TGARGLAGPPGMPGPRGSPGPQGV

SEQ ID NO: 218 - protein, 25 aa, Homo sapiens
VKGESGKPGANGLSGERGPPGPQGL

SEQ ID NO: 219 - protein, 53 aa, Homo sapiens
GVKGERGSPGGPGAAGFPGARGLPGPPGSNGNPGPPGPSGSPGKDGPPGPAGN

SEQ ID NO: 220 - protein, 32 aa, Homo sapiens
GSPGAQGPPGAPGPLGIAGITGARGLAGPPGM

SEQ ID NO: 221 - protein, 32 aa, Homo sapiens
RGAPGEKGEGGPPGVAGPPGGSGPAGPPGPQG

SEQ ID NO: 222 - protein, 32 aa, Homo sapiens; identical to SEQ ID NO: 221

SEQ ID NO: 223 - protein, 29 aa, Homo sapiens
GIAGITGARGLAGPPGMPGPRGSPGPQGV

SEQ ID NO: 224 - protein, 14 aa, Homo sapiens
GIKGPAGIPGFPGM

SEQ ID NO: 225 - protein, 14 aa, Homo sapiens
GQPGVMGFPGPKGN

SEQ ID NO: 226 - protein, 16 aa, Homo sapiens
GIKGPAGIPGFPGMKG

SEQ ID NO: 227 - protein, 17 aa, Homo sapiens
GIKGPAGIPGFPGMKGH

SEQ ID NO: 228 - protein, 19 aa, Homo sapiens
IPGAPGLMGARGPPGPAGA

SEQ ID NO: 229 - protein, 19 aa, Homo sapiens
GERGLPGPPGIKGPAGIPG

SEQ ID NO: 230 - protein, 20 aa, Homo sapiens
GIPGAPGLMGARGPPGPAGA

SEQ ID NO: 231 - protein, 20 aa, Homo sapiens
GFRGPAGPNGIPGEKGPAGE

SEQ ID NO: 232 - protein, 20 aa, Homo sapiens
PGIPGQPGSPGSPGPPGICE

SEQ ID NO: 233 - protein, 21 aa, Homo sapiens
GERGLPGPPGIKGPAGIPGFP

SEQ ID NO: 234 - protein, 23 aa, Homo sapiens
AVGGLAGYPGPAGPPGPPGPPGT

SEQ ID NO: 235 - protein, 23 aa, Homo sapiens
GVKGERGSPGGPGAAGFPGARGL

SEQ ID NO: 236 - protein, 26 aa, Homo sapiens
GDAGAPGAPGGKGDAGAPGERGPPGL

SEQ ID NO: 237 - protein, 25 aa, Homo sapiens
QGPPGPTGPGGDKGDTGPPGPQGLQ

SEQ ID NO: 238 - protein, 25 aa, Homo sapiens
GINGSPGGKGEMGPAGIPGAPGLMG

SEQ ID NO: 239 - protein, 26 aa, Homo sapiens
QGPPGEPGQAGPSGPPGPPGAIGPSG

SEQ ID NO: 240 - protein, 26 aa, Homo sapiens
PGPPGINGSPGGKGEMGPAGIPGAPG

SEQ ID NO: 241 - protein, 33 aa, Homo sapiens
RGLPGPPGSNGNPGPPGPSGSPGKDGPPGPAGN

SEQ ID NO: 242 - protein, 32 aa, Homo sapiens
GKNGETGPQGPPGPTGPGGDKGDTGPPGPQGL

SEQ ID NO: 243 - protein, 32 aa, Homo sapiens
GLPGIAGPRGSPGERGETGPPGPAGFPGAPGQ

SEQ ID NO: 244 - protein, 35 aa, Homo sapiens
GINGSPGGKGEMGPAGIPGAPGLMGARGPPGPAGA

SEQ ID NO: 245 - protein, 36 aa, Homo sapiens
PGINGSPGGKGEMGPAGIPGAPGLMGARGPPGPAGA

SEQ ID NO: 246 - protein, 40 aa, Homo sapiens
PPGENGKPGEPGPKGDAGAPGAPGGKGDAGAPGERGPPGL

SEQ ID NO: 247 - protein, 38 aa, Homo sapiens
GLKGENGLPGENGAPGPMGPRGAPGERGRPGLPGAAGA

SEQ ID NO: 248 - protein, 41 aa, Homo sapiens
GNTGAPGSPGVSGPKGDAGQPGEKGSPGAQGPPGAPGPLGI

SEQ ID NO: 249 - protein, 41 aa, Homo sapiens
GLMGARGPPGPAGANGAPGLRGGAGEPGKNGAKGEPGPRGE

SEQ ID NO: 250 - protein, 50 aa, Homo sapiens
GLRGGAGPPGPEGGKGAAGPPGPPGAAGTPGLQGMPGERGGLGSPGPKGD

SEQ ID NO: 251 - protein, 26 aa, Homo sapiens
GQQGAIGSPGPAGPRGPVGPSGPPGK

SEQ ID NO: 252 - protein, 24 aa, Homo sapiens
KGDPGPPGIPGRNGDPGIPGQPGS

SEQ ID NO: 253 - protein, 26 aa, Homo sapiens
GLRGGAGPPGPEGGKGAAGPPGPPGA

SEQ ID NO: 254 - protein, 32 aa, Homo sapiens; identical to SEQ ID NO: 242

SEQ ID NO: 255 - protein, 23 aa, Homo sapiens
GYQGPPGEPGQAGPSGPPGPPGA

SEQ ID NO: 256 - protein, 20 aa, Homo sapiens
GVAGPPGGSGPAGPPGPQGV

SEQ ID NO: 257 - protein, 35 aa, Homo sapiens
GDKGEPGGPGADGVPGKDGPRGPTGPIGPPGPAGQ

SEQ ID NO: 258 - protein, 17 aa, Homo sapiens
QGHAGAQGPPGPPGING

SEQ ID NO: 259 - protein, 11 aa, Homo sapiens
AGERGAPGPAG

SEQ ID NO: 260 - protein, 11 aa, Homo sapiens
AGIPGFPGMKG

SEQ ID NO: 261 - protein, 12 aa, Homo sapiens
FPGMKGHRGFDG

SEQ ID NO: 262 - protein, 14 aa, Homo sapiens
GFPGARGLPGPPGS

SEQ ID NO: 263 - protein, 15 aa, Homo sapiens
AGFPGARGLPGPPGS

SEQ ID NO: 264 - protein, 15 aa, Homo sapiens
PPGPPGPPGTSGHPG

SEQ ID NO: 265 - protein, 13 aa, Homo sapiens
GFPGMKGHRGFDG

SEQ ID NO: 266 - protein, 17 aa, Homo sapiens
QPGDKGEGGAPGLPGIA

SEQ ID NO: 267 - protein, 17 aa, Homo sapiens
RGDKGETGERGAAGIKG

SEQ ID NO: 268 - protein, 17 aa, Homo sapiens
DGRNGEKGETGAPGLKG

SEQ ID NO: 269 - protein, 20 aa, Homo sapiens
AGQPGDKGEGGAPGLPGIAG

SEQ ID NO: 270 - protein, 19 aa, Homo sapiens
GGPPGENGKPGEPGPKGDA

SEQ ID NO: 271 - protein, 17 aa, Homo sapiens
AGIPGFPGMKGHRGFDG

SEQ ID NO: 272 - protein, 20 aa, Homo sapiens
RGGAGEPGKNGAKGEPGPRG

SEQ ID NO: 273 - protein, 26 aa, Homo sapiens
KGERGSPGGPGAAGFPGARGLPGPPG

SEQ ID NO: 274 - protein, 27 aa, Homo sapiens
IPGVPGAKGEDGKDGSPGEPGANGLPG

SEQ ID NO: 275 - protein, 28 aa, Homo sapiens
GAAGFPGARGLPGPPGSNGNPGPPGPSG

SEQ ID NO: 276 - protein, 26 aa, Homo sapiens
RPGPPGPSGPRGQPGVMGFPGPKGND

SEQ ID NO: 277 - protein, 29 aa, Homo sapiens
QGPPGPPGINGSPGGKGEMGPAGIPGAPG

SEQ ID NO: 278 - protein, 26 aa, Homo sapiens
AGKDGESGRPGRPGERGLPGPPGIKG

SEQ ID NO: 279 - protein, 30 aa, Homo sapiens
AGARGNDGARGSDGQPGPPGPPGTAGFPGS

SEQ ID NO: 280 - protein, 31 aa, Homo sapiens
SPGVSGPKGDAGQPGEKGSPGAQGPPGAPGP

SEQ ID NO: 281 - protein, 32 aa, Homo sapiens
RGSDGQPGPPGPPGTAGFPGSPGAKGEVGPAG

SEQ ID NO: 282 - protein, 32 aa, Homo sapiens
QGPPGPPGINGSPGGKGEMGPAGIPGAPGLMG

SEQ ID NO: 283 - protein, 33 aa, Homo sapiens
AGPPGPPGPPGTSGHPGSPGSPGYQGPPGEPGQ

SEQ ID NO: 284 - protein, 33 aa, Homo sapiens
FPGAPGQNGEPGGKGERGAPGEKGEGGPPGVAG

SEQ ID NO: 285 - protein, 33 aa, Homo sapiens
AGFPGAPGQNGEPGGKGERGAPGEKGEGGPPGV

SEQ ID NO: 286 - protein, 41 aa, Homo sapiens
AGARGNDGARGSDGQPGPPGPPGTAGFPGSPGAKGEVGPAG

SEQ ID NO: 287 - protein, 53 aa, Homo sapiens
RGAAGEPGRDGVPGGPGMRGMPGSPGGPGSDGKPGPPGSQGESGRPGPPGPSG

SEQ ID NO: 288 - protein, 12 aa, Homo sapiens
GIAGITGARGLA

SEQ ID NO: 289 - protein, 18 aa, Homo sapiens
AGPPGPPGAAGTPGLQGM

SEQ ID NO: 290 - protein, 18 aa, Homo sapiens
NGLSGERGPPGPQGLPGL

SEQ ID NO: 291 - protein, 20 aa, Homo sapiens
MGARGPPGPAGANGAPGLRG

SEQ ID NO: 292 - protein, 20 aa, Homo sapiens
NGLSGERGPPGPQGLPGLAG

SEQ ID NO: 293 - protein, 23 aa, Homo sapiens
GIAGITGARGLAGPPGMPGPRGS

SEQ ID NO: 294 - protein, 29 aa, Homo sapiens
GIAGITGARGLAGPPGMPGPRGSPGPQGV

SEQ ID NO: 295 - protein, 32 aa, Homo sapiens
RGGAGPPGPEGGKGAAGPPGPPGAAGTPGLQG

SEQ ID NO: 296 - protein, 30 aa, Homo sapiens
SGPKGDAGQPGEKGSPGAQGPPGAPGPLGI

SEQ ID NO: 297 - protein, 31 aa, Homo sapiens
GIAGITGARGLAGPPGMPGPRGSPGPQGVKG

SEQ ID NO: 298 - protein, 30 aa, Homo sapiens; identical to SEQ ID NO: 296

SEQ ID NO: 299 - protein, 31 aa, Homo sapiens; identical to SEQ ID NO: 297

SEQ ID NO: 300 - protein, 37 aa, Homo sapiens
AVGGLAGYPGPAGPPGPPGPPGTSGHPGSPGSPGYQG

SEQ ID NO: 301 - protein, 40 aa, Homo sapiens
EPGPQGHAGAQGPPGPPGINGSPGGKGEMGPAGIPGAPGL

SEQ ID NO: 302 - protein, 12 aa, Homo sapiens
IPGFPGMKGHRG

SEQ ID NO: 303 - protein, 17 aa, Homo sapiens
RGSPGGPGAAGFPGARG

SEQ ID NO: 304 - protein, 17 aa, Homo sapiens
KGPAGIPGFPGMKGHRG

SEQ ID NO: 305 - protein, 20 aa, Homo sapiens
RGLAGPPGMPGPRGSPGPQG

SEQ ID NO: 306 - protein, 20 aa, Homo sapiens
AGITGARGLAGPPGMPGPRG

SEQ ID NO: 307 - protein, 23 aa, Homo sapiens
LGIAGITGARGLAGPPGMPGPRG

SEQ ID NO: 308 - protein, 23 aa, Homo sapiens
TGARGLAGPPGMPGPRGSPGPQG

SEQ ID NO: 309 - protein, 24 aa, Homo sapiens
QGPPGPPGINGSPGGKGEMGPAGI

SEQ ID NO: 310 - protein, 24 aa, Homo sapiens
LPGPPGIKGPAGIPGFPGMKGHRG

SEQ ID NO: 311 - protein, 26 aa, Homo sapiens
AGITGARGLAGPPGMPGPRGSPGPQG

SEQ ID NO: 312 - protein, 26 aa, Homo sapiens
TGARGLAGPPGMPGPRGSPGPQGVKG

SEQ ID NO: 313 - protein, 26 aa, Homo sapiens
RGLPGPPGIKGPAGIPGFPGMKGHRG

SEQ ID NO: 314 - protein, 29 aa, Homo sapiens
GRPGLPGAAGARGNDGARGSDGQPGPPGP

SEQ ID NO: 315 - protein, 29 aa, Homo sapiens
NGAPGPMGPRGAPGERGRPGLPGAAGARG

SEQ ID NO: 316 - protein, 29 aa, Homo sapiens
AGSRGAPGPQGPRGDKGETGERGAAGIKG

SEQ ID NO: 317 - protein, 32 aa, Homo sapiens
RGLAGPPGMPGPRGSPGPQGVKGESGKPGANG

SEQ ID NO: 318 - protein, 34 aa, Homo sapiens
RGLAGPPGMPGPRGSPGPQGVKGESGKPGANGLS

SEQ ID NO: 319 - protein, 37 aa, Homo sapiens
PGPPGSNGNPGPPGPSGSPGKDGPPGPAGNTGAPGSP

SEQ ID NO: 320 - protein, 35 aa, Homo sapiens
TGARGLAGPPGMPGPRGSPGPQGVKGESGKPGANG

SEQ ID NO: 321 - protein, 38 aa, Homo sapiens
RGAPGEKGEGGPPGVAGPPGGSGPAGPPGPQGVKGERG

SEQ ID NO: 322 - protein, 40 aa, Homo sapiens
GGPPGVAGPPGGSGPAGPPGPQGVKGERGSPGGPGAAGFP

SEQ ID NO: 323 - protein, 48 aa, Homo sapiens
KSGDRGESGPAGPAGAPGPAGSRGAPGPQGPRGDKGETGERGAAGIKG

SEQ ID NO: 324 - protein, 12 aa, Homo sapiens
IPGFPGMKGHRG

SEQ ID NO: 325 - protein, 14 aa, Homo sapiens
RGLAGPPGMPGPRG

SEQ ID NO: 326 - protein, 16 aa, Homo sapiens
GPQGLQGLPGTGGPPG

SEQ ID NO: 327 - protein, 17 aa, Homo sapiens
KGPAGIPGFPGMKGHRG

SEQ ID NO: 328 - protein, 21 aa, Homo sapiens
RGLAGPPGMPGPRGSPGPQGV

SEQ ID NO: 329 - protein, 23 aa, Homo sapiens
GGPPGENGKPGEPGPKGDAGAPG

SEQ ID NO: 330 - protein, 24 aa, Homo sapiens
APGFRGPAGPNGIPGEKGPAGERG

SEQ ID NO: 331 - protein, 27 aa, Homo sapiens
EKGSPGAQGPPGAPGPLGIAGITGARG

SEQ ID NO: 332 - protein, 24 aa, Homo sapiens
LPGPPGIKGPAGIPGFPGMKGHRG

SEQ ID NO: 333 - protein, 26 aa, Homo sapiens
RGAPGFRGPAGPNGIPGEKGPAGERG

SEQ ID NO: 334 - protein, 26 aa, Homo sapiens
RGLPGPPGIKGPAGIPGFPGMKGHRG

SEQ ID NO: 335 - protein, 29 aa, Homo sapiens
RGPVGPSGPPGKDGTSGHPGPIGPPGPRG

SEQ ID NO: 336 - protein, 27 aa, Homo sapiens
APGPQGPRGDKGETGERGAAGIKGHRG

SEQ ID NO: 337 - protein, 29 aa, Homo sapiens
RGAPGPQGPRGDKGETGERGAAGIKGHRG

SEQ ID NO: 338 - protein, 32 aa, Homo sapiens
RGFPGNPGAPGSPGPAGQQGAIGSPGPAGPRG

SEQ ID NO: 339 - protein, 29 aa, Homo sapiens
LPGPPGIKGPAGIPGFPGMKGHRGFDGRN

SEQ ID NO: 340 - protein, 33 aa, Homo sapiens
DAGQPGEKGSPGAQGPPGAPGPLGIAGITGARG

SEQ ID NO: 341 - protein, 35 aa, Homo sapiens
RGPTGPIGPPGPAGQPGDKGEGGAPGLPGIAGPRG

SEQ ID NO: 342 - protein, 35 aa, Homo sapiens
KGDAGQPGEKGSPGAQGPPGAPGPLGIAGITGARG

SEQ ID NO: 343 - protein, 33 aa, Homo sapiens
RNGEKGETGAPGLKGENGLPGENGAPGPMGPRG

SEQ ID NO: 344 - protein, 35 aa, Homo sapiens
APGFRGPAGPNGIPGEKGPAGERGAPGPAGPRGAA

SEQ ID NO: 345 - protein, 35 aa, Homo sapiens
RGAPGFRGPAGPNGIPGEKGPAGERGAPGPAGPRG

SEQ ID NO: 346 - protein, 35 aa, Homo sapiens
RGSPGERGETGPPGPAGFPGAPGQNGEPGGKGERG

SEQ ID NO: 347 - protein, 38 aa, Homo sapiens
GHAGAQGPPGPPGINGSPGGKGEMGPAGIPGAPGLMGA

SEQ ID NO: 348 - protein, 38 aa, Homo sapiens
RGLAGPPGMPGPRGSPGPQGVKGESGKPGANGLSGERG

SEQ ID NO: 349 - protein, 13 aa, Homo sapiens
LGIAGITGARGLA

SEQ ID NO: 350 - protein, 12 aa, Homo sapiens
IPGFPGMKGHRG

SEQ ID NO: 351 - protein, 14 aa, Homo sapiens
RGLAGPPGMPGPRG

SEQ ID NO: 352 - protein, 20 aa, Homo sapiens
QGPPGAPGPLGIAGITGARG

SEQ ID NO: 353 - protein, 20 aa, Homo sapiens
AGITGARGLAGPPGMPGPRG

SEQ ID NO: 354 - protein, 23 aa, Homo sapiens
AGIPGAPGLMGARGPPGPAGANG

SEQ ID NO: 355 - protein, 24 aa, Homo sapiens
RGLAGPPGMPGPRGSPGPQGVKGE

SEQ ID NO: 356 - protein, 26 aa, Homo sapiens
KGSPGAQGPPGAPGPLGIAGITGARG

SEQ ID NO: 357 - protein, 24 aa, Homo sapiens
LPGPPGIKGPAGIPGFPGMKGHRG

SEQ ID NO: 358 - protein, 24 aa, Homo sapiens
KDGTSGHPGPIGPPGPRGNRGERG

SEQ ID NO: 359 - protein, 26 aa, Homo sapiens
AGITGARGLAGPPGMPGPRGSPGPQG

SEQ ID NO: 360 - protein, 27 aa, Homo sapiens
RGLAGPPGMPGPRGSPGPQGVKGESGK

SEQ ID NO: 361 - protein, 32 aa, Homo sapiens; identical to SEQ ID NO: 317

SEQ ID NO: 362 - protein, 34 aa, Homo sapiens; identical to SEQ ID NO: 318

SEQ ID NO: 363 - protein, 37 aa, Homo sapiens; identical to SEQ ID NO: 319

SEQ ID NO: 364 - protein, 38 aa, Homo sapiens; identical to SEQ ID NO: 321

SEQ ID NO: 365 - protein, 44 aa, Homo sapiens
KSGDRGESGPAGPAGAPGPAGSRGAPGPQGPRGDKGETGERGAA

SEQ ID NO: 366 - protein, 53 aa, Homo sapiens
RGAPGEKGEGGPPGVAGPPGGSGPAGPPGPQGVKGERGSPGGPGAAGFPGARG

SEQ ID NO: 367 - protein, 6 aa, Homo sapiens
AIGPSG

SEQ ID NO: 368 - protein, 10 aa, Homo sapiens
PGIPGRNGDP

SEQ ID NO: 369 - protein, 10 aa, Homo sapiens
ESCPTGPQNY

SEQ ID NO: 370 - protein, 10 aa, Homo sapiens
PKGDTGPRGP

SEQ ID NO: 371 - protein, 6 aa, Homo sapiens
GIPGAP

SEQ ID NO: 372 - protein, 6 aa, Homo sapiens
  MOD_RES (3)..(3): proline or hydroxyproline
  MOD_RES (5)..(6): proline or hydroxyproline
GDXGXX

SEQ ID NO: 373 - protein, 6 aa, Homo sapiens
KGESGK

SEQ ID NO: 374 - protein, 6 aa, Homo sapiens
IAGITG

SEQ ID NO: 375 - protein, 6 aa, Homo sapiens
IKGHRG

SEQ ID NO: 376 - protein, 6 aa, Homo sapiens
RGLAGP

SEQ ID NO: 377 - protein, 6 aa, Homo sapiens
TGARGL

SEQ ID NO: 378 - protein, 6 aa, Homo sapiens
ITGARG

SEQ ID NO: 379 - protein, 6 aa, Homo sapiens
VKGESG

SEQ ID NO: 380 - protein, 6 aa, Homo sapiens
KGDAGQ

SEQ ID NO: 381 - protein, 6 aa, Homo sapiens
LRGGAG

SEQ ID NO: 382 - protein, 6 aa, Homo sapiens
GKSGDR

SEQ ID NO: 383 - protein, 6 aa, Homo sapiens
LQGLPG

SEQ ID NO: 384 - protein, 6 aa, Homo sapiens
ERGLPG

SEQ ID NO: 385 - protein, 6 aa, Homo sapiens
IGSPGP

SEQ ID NO: 386 - protein, 6 aa, Homo sapiens
GAPGEK

SEQ ID NO: 387 - protein, 6 aa, Homo sapiens
GLSGER

SEQ ID NO: 388 - protein, 6 aa, Homo sapiens
GLAGPP

SEQ ID NO: 389 - protein, 6 aa, Homo sapiens
PQGPPG

SEQ ID NO: 390 - protein, 6 aa, Homo sapiens
QQGAIG

SEQ ID NO: 391 - protein, 6 aa, Homo sapiens
GPPGPT

SEQ ID NO: 392 - protein, 6 aa, Homo sapiens
INGSPG

SEQ ID NO: 393 - protein, 6 aa, Homo sapiens
GPPGEP

SEQ ID NO: 394 - protein, 6 aa, Homo sapiens
GLPGPP

SEQ ID NO: 395 - protein, 6 aa, Homo sapiens
KNGETG

SEQ ID NO: 396 - protein, 6 aa, Homo sapiens
LPGIAG

SEQ ID NO: 397 - protein, 6 aa, Homo sapiens
GINGSP

SEQ ID NO: 398 - protein, 6 aa, Homo sapiens
GINGSP

SEQ ID NO: 399 - protein, 6 aa, Homo sapiens
LKGENG

SEQ ID NO: 400 - protein, 6 aa, Homo sapiens
LMGARG

SEQ ID NO: 401 - protein, 6 aa, Homo sapiens
YQGPPG

SEQ ID NO: 402 - protein, 6 aa, Homo sapiens
GERGAP

SEQ ID NO: 403 - protein, 6 aa, Homo sapiens
DKGEPG

SEQ ID NO: 404 - protein, 6 aa, Homo sapiens
GHAGAQ

SEQ ID NO: 405 - protein, 6 aa, Homo sapiens
GSDGQP

SEQ ID NO: 406 - protein, 6 aa, Homo sapiens
PGMKGH

SEQ ID NO: 407 - protein, 6 aa, Homo sapiens
FPGARG

SEQ ID NO: 408 - protein, 6 aa, Homo sapiens
GFPGAR

SEQ ID NO: 409 - protein, 6 aa, Homo sapiens
FPGMKG

SEQ ID NO: 410 - protein, 6 aa, Homo sapiens
PGDKGE

SEQ ID NO: 411 - protein, 6 aa, Homo sapiens
GDKGET

SEQ ID NO: 412 - protein, 6 aa, Homo sapiens
GQPGDK

SEQ ID NO: 413 - protein, 6 aa, Homo sapiens
GPPGEN

SEQ ID NO: 414 - protein, 6 aa, Homo sapiens
GIPGFP

SEQ ID NO: 415 - protein, 6 aa, Homo sapiens
GERGSP

SEQ ID NO: 416 - protein, 6 aa, Homo sapiens
PGVPGA

SEQ ID NO: 417 - protein, 6 aa, Homo sapiens
AAGFPG

SEQ ID NO: 418 - protein, 6 aa, Homo sapiens
GKDGES

SEQ ID NO: 419 - protein, 6 aa, Homo sapiens
GARGND

SEQ ID NO: 420 - protein, 6 aa, Homo sapiens
GFPGAP

SEQ ID NO: 421 - protein, 6 aa, Homo sapiens
GAAGEP

SEQ ID NO: 422 - protein, 6 aa, Homo sapiens
GARGPP

SEQ ID NO: 423 - protein, 6 aa, Homo sapiens
GPPGSN

SEQ ID NO: 424 - protein, 6 aa, Homo sapiens
GPKGDA

SEQ ID NO: 425 - protein, 6 aa, Homo sapiens
GGAGPP

SEQ ID NO: 426 - protein, 6 aa, Homo sapiens
PGPQGH

SEQ ID NO: 427 - protein, 6 aa, Homo sapiens
PGFPGM

SEQ ID NO: 428 - protein, 6 aa, Homo sapiens
GSPGGP

SEQ ID NO: 429 - protein, 6 aa, Homo sapiens
SGDRGE

SEQ ID NO: 430 - protein, 6 aa, Homo sapiens
GITGAR

SEQ ID NO: 431 - protein, 6 aa, Homo sapiens
GIAGIT

SEQ ID NO: 432 - protein, 6 aa, Homo sapiens
PGPPGI

SEQ ID NO: 433 - protein, 6 aa, Homo sapiens
ESCPTG

SEQ ID NO: 434 - protein, 6 aa, Homo sapiens
HAGAQG

SEQ ID NO: 435 - protein, 6 aa, Homo sapiens
GAPGFR

SEQ ID NO: 436 - protein, 6 aa, Homo sapiens
RPGLPG

SEQ ID NO: 437 - protein, 6 aa, Homo sapiens
NTGAPG

SEQ ID NO: 438 - protein, 6 aa, Homo sapiens
GAPGPM

SEQ ID NO: 439 - protein, 6 aa, Homo sapiens
GSPGER

SEQ ID NO: 440 - protein, 6 aa, Homo sapiens
PQGLQG

SEQ ID NO: 441 - protein, 6 aa, Homo sapiens
GPAGIP

SEQ ID NO: 442 - protein, 6 aa, Homo sapiens
DRGPQG

SEQ ID NO: 443 - protein, 6 aa, Homo sapiens
PGFRGP

SEQ ID NO: 444 - protein, 6 aa, Homo sapiens
KGSPGA

SEQ ID NO: 445 - protein, 6 aa, Homo sapiens
GAPGPQ

SEQ ID NO: 446 - protein, 6 aa, Homo sapiens
GFPGNP

SEQ ID NO: 447 - protein, 6 aa, Homo sapiens
GPVGPS

SEQ ID NO: 448 - protein, 6 aa, Homo sapiens
GPTGPI

SEQ ID NO: 449 - protein, 6 aa, Homo sapiens
GDAGQP

SEQ ID NO: 450 - protein, 6 aa, Homo sapiens
NGEKGE

SEQ ID NO: 451 - protein, 6 aa, Homo sapiens
SRGAPG

SEQ ID NO: 452 - protein, 6 aa, Homo sapiens
VAGPPG

SEQ ID NO: 453 - protein, 6 aa, Homo sapiens
PGPQGP

SEQ ID NO: 454 - protein, 6 aa, Homo sapiens
AGQPGE

SEQ ID NO: 455 - protein, 6 aa, Homo sapiens
PGAPGG

SEQ ID NO: 456 - protein, 6 aa, Homo sapiens
PGAPGQ

SEQ ID NO: 457 - protein, 6 aa, Homo sapiens
AGQQGA

SEQ ID NO: 458 - protein, 6 aa, Homo sapiens
  MOD_RES (1)..(1): proline or hydroxyproline
  MOD_RES (3)..(3): proline or hydroxyproline
  MOD_RES (6)..(6): proline or hydroxyproline
XGXPGX

SEQ ID NO: 459 - protein, 6 aa, Homo sapiens
SPGGKG

SEQ ID NO: 460 - protein, 6 aa, Homo sapiens
GRNGEK

SEQ ID NO: 461 - protein, 6 aa, Homo sapiens
GPPGAP

SEQ ID NO: 462 - protein, 6 aa, Homo sapiens
GSRGAP

SEQ ID NO: 463 - protein, 6 aa, Homo sapiens
GGAGEP

SEQ ID NO: 464 - protein, 6 aa, Homo sapiens
GSPGAQ

SEQ ID NO: 465 - protein, 6 aa, Homo sapiens
SPGAQG

SEQ ID NO: 466 - protein, 6 aa, Homo sapiens
PGVSGP

SEQ ID NO: 467 - protein, 6 aa, Homo sapiens
PGAPGL

SEQ ID NO: 468 - protein, 6 aa, Homo sapiens
GIPGQP

SEQ ID NO: 469 - protein, 6 aa, Homo sapiens
DAGAPG

SEQ ID NO: 470 - protein, 6 aa, Homo sapiens
GPPGIN

SEQ ID NO: 471 - protein, 6 aa, Homo sapiens
NGDPGI

SEQ ID NO: 472 - protein, 6 aa, Homo sapiens
SPGPQG

SEQ ID NO: 473 - protein, 6 aa, Homo sapiens
GMPGPR

SEQ ID NO: 474 - protein, 6 aa, Homo sapiens
SPGPAG

SEQ ID NO: 475 - protein, 6 aa, Homo sapiens
PGPQGV

SEQ ID NO: 476 - protein, 6 aa, Homo sapiens
ERGAAG

SEQ ID NO: 477 - protein, 6 aa, Homo sapiens
PGPLGI

SEQ ID NO: 478 - protein, 6 aa, Homo sapiens
AAGTPG

SEQ ID NO: 479 - protein, 6 aa, Homo sapiens
PGPPGT

SEQ ID NO: 480 - protein, 6 aa, Homo sapiens
GNRGER

SEQ ID NO: 481 - protein, 6 aa, Homo sapiens
APGLRG

SEQ ID NO: 482 - protein, 6 aa, Homo sapiens
HPGSPG

SEQ ID NO: 483 - protein, 6 aa, Homo sapiens
PSGPPG

SEQ ID NO: 484 - protein, 6 aa, Homo sapiens
GSPGPA

SEQ ID NO: 485 - protein, 6 aa, Homo sapiens
GPAGPP

SEQ ID NO: 486 - protein, 6 aa, Homo sapiens
GLPGLA

SEQ ID NO: 487 - protein, 6 aa, Homo sapiens
QGPPGP

SEQ ID NO: 488 - protein, 6 aa, Homo sapiens
GLAGTA

SEQ ID NO: 489 - protein, 6 aa, Homo sapiens
PGLMGA

SEQ ID NO: 490 - protein, 6 aa, Homo sapiens
GPPGPQ

SEQ ID NO: 491 - protein, 6 aa, Homo sapiens
  MOD_RES (2)..(2): proline or hydroxyproline
  MOD_RES (4)..(4): proline or hydroxyproline
FXGXKG

SEQ ID NO: 492 - protein, 6 aa, Homo sapiens
IPGFPG

SEQ ID NO: 493 - protein, 6 aa, Homo sapiens
GFPGMK

SEQ ID NO: 494 - protein, 6 aa, Homo sapiens
FPGAPG

SEQ ID NO: 495 - protein, 6 aa, Homo sapiens
GAIGPS

SEQ ID NO: 496 - protein, 6 aa, Homo sapiens
AGIPGF

SEQ ID NO: 497 - protein, 6 aa, Homo sapiens
PGPQGL

SEQ ID NO: 498 - protein, 6 aa, Homo sapiens
GAPGLM

SEQ ID NO: 499 - protein, 6 aa, Homo sapiens
SPGPKG

SEQ ID NO: 500 - protein, 6 aa, Homo sapiens
GEPGPR

SEQ ID NO: 501 - protein, 6 aa, Homo sapiens
IPGQPG

SEQ ID NO: 502 - protein, 6 aa, Homo sapiens
TGAPGS

SEQ ID NO: 503 - protein, 6 aa, Homo sapiens
GHRGFD

SEQ ID NO: 504 - protein, 6 aa, Homo sapiens
PGLPGI

SEQ ID NO: 505 - protein, 6 aa, Homo sapiens
GAAGIK

SEQ ID NO: 506 - protein, 6 aa, Homo sapiens
PGPKGD

SEQ ID NO: 507 - protein, 6 aa, Homo sapiens
GLPGIA

SEQ ID NO: 508 - protein, 6 aa, Homo sapiens
PQGLPG

SEQ ID NO: 509 - protein, 6 aa, Homo sapiens
GAPGLR

SEQ ID NO: 510 - protein, 6 aa, Homo sapiens
GANGLP

SEQ ID NO: 511 - protein, 6 aa, Homo sapiens
GPPGPS

SEQ ID NO: 512 - protein, 6 aa, Homo sapiens
GPPGIK

SEQ ID NO: 513 - protein, 6 aa, Homo sapiens
TAGFPG

SEQ ID NO: 514 - protein, 6 aa, Homo sapiens
GEVGPA

SEQ ID NO: 515 - protein, 6 aa, Homo sapiens
EKGPAG

SEQ ID NO: 516 - protein, 6 aa, Homo sapiens
  MOD_RES (2)..(2): proline or hydroxyproline
EXGPRG

SEQ ID NO: 517 - protein, 6 aa, Homo sapiens
PPGAPG

SEQ ID NO: 518 - protein, 6 aa, Homo sapiens
TSGHPG

SEQ ID NO: 519 - protein, 6 aa, Homo sapiens
GAPGPA

SEQ ID NO: 520 - protein, 6 aa, Homo sapiens
TPGLQG

SEQ ID NO: 521 - protein, 6 aa, Homo sapiens
GTPGLQ

SEQ ID NO: 522 - protein, 6 aa, Homo sapiens
GTSGHP

SEQ ID NO: 523 - protein, 6 aa, Homo sapiens
MPGPRG

SEQ ID NO: 524 - protein, 6 aa, Homo sapiens
GPQGVK

SEQ ID NO: 525 - protein, 6 aa, Homo sapiens
GAPGLK

SEQ ID NO: 526 - protein, 6 aa, Homo sapiens
GSPGYQ

SEQ ID NO: 527 - protein, 6 aa, Homo sapiens
  MOD_RES (1)..(1): proline or hydroxyproline
  MOD_RES (4)..(4): lysine or hydroxylysine
XGPXGN

SEQ ID NO: 528 - protein, 6 aa, Homo sapiens
GAAGAR

SEQ ID NO: 529 - protein, 6 aa, Homo sapiens
PGANGL

SEQ ID NO: 530 - protein, 6 aa, Homo sapiens
GTGGPP

SEQ ID NO: 531 - protein, 6 aa, Homo sapiens
GMKGHR

SEQ ID NO: 532 - protein, 6 aa, Homo sapiens
EGGPPG

SEQ ID NO: 533 - protein, 6 aa, Homo sapiens
GSPGPQ

SEQ ID NO: 534 - protein, 6 aa, Homo sapiens
EMGPAG

SEQ ID NO: 535 - protein, 6 aa, Homo sapiens
GIAGPR

SEQ ID NO: 536 - protein, 6 aa, Homo sapiens
QPGPPG

SEQ ID NO: 537 - protein, 6 aa, Homo sapiens
GKPGAN

SEQ ID NO: 538 - protein, 6 aa, Homo sapiens
GVKGER

SEQ ID NO: 539 - protein, 6 aa, Homo sapiens
PGAAGF

SEQ ID NO: 540 - protein, 6 aa, Homo sapiens
TGERGA

SEQ ID NO: 541 - protein, 6 aa, Homo sapiens
PQGVKG

SEQ ID NO: 542 - protein, 6 aa, Homo sapiens
GDAGAP

SEQ ID NO: 543 - protein, 6 aa, Homo sapiens
GPAGER

SEQ ID NO: 544 - protein, 6 aa, Homo sapiens
GPPGPR

SEQ ID NO: 545 - protein, 6 aa, Homo sapiens
GPAGPR

SEQ ID NO: 546 - protein, 6 aa, Homo sapiens
RGFDGR

SEQ ID NO: 547 - protein, 6 aa, Homo sapiens
AGPRGA

SEQ ID NO: 548 - protein, 6 aa, Homo sapiens
GGKGER

SEQ ID NO: 549 - protein, 6 aa, Homo sapiens
APGLMG

SEQ ID NO: 550 - protein, 6 aa, Homo sapiens
GPAGAN

SEQ ID NO: 551 - protein, 12 aa, Homo sapiens
DIDGYRGPPGPQ

SEQ ID NO: 552 - protein, 15 aa, Homo sapiens
SMGPPGTPSVDHGFL

SEQ ID NO: 553 - protein, 20 aa, Homo sapiens
PDGLPGSMGPPGTPSVDHGF

SEQ ID NO: 554 - protein, 21 aa, Homo sapiens
PDGLPGSMGPPGTPSVDHGFL

SEQ ID NO: 555 - protein, 22 aa, Homo sapiens
PDGLPGSMGPPGTPSVDHGFLV

SEQ ID NO: 556 - protein, 23 aa, Homo sapiens
PSGRDGLPGPPGSPGPPGQPGYT

SEQ ID NO: 557 - protein, 25 aa, Homo sapiens
PSGRDGLPGPPGSPGPPGQPGYTNG

SEQ ID NO: 558 - protein, 26 aa, Homo sapiens
PSGRDGLPGPPGSPGPPGQPGYTNGI

SEQ ID NO: 559 - protein, 26 aa, Homo sapiens
IPGSKGEQGFMGPPGPQGQPGLPGSP

SEQ ID NO: 560 - protein, 27 aa, Homo sapiens
PRGFPGPPGPDGLPGSMGPPGTPSVDH

SEQ ID NO: 561 - protein, 16 aa, Homo sapiens
EPGPPGLPGSVGSPGV

SEQ ID NO: 562 - protein, 14 aa, Homo sapiens
IDGYRGPPGPQGPP

SEQ ID NO: 563 - protein, 19 aa, Homo sapiens
PRGFPGPPGPDGLPGSMGP

SEQ ID NO: 564 - protein, 20 aa, Homo sapiens
DGLPGSMGPPGTPSVDHGFL

SEQ ID NO: 565 - protein, 21 aa, Homo sapiens
DGLPGSMGPPGTPSVDHGFLV

SEQ ID NO: 566 - protein, 29 aa, Homo sapiens
PGLPGQQGAPGIPGFPGSKGEMGVMGTPG

SEQ ID NO: 567 - protein, 31 aa, Homo sapiens
IGIPGMPGSPGLKGSPGSVGYPGSPGLPGEK

SEQ ID NO: 568 - protein, 37 aa, Homo sapiens
PGPPGPPGEKGQMGLSFQGPKGDKGDQGVSGPPGVPG

SEQ ID NO: 569 - protein, 39 aa, Homo sapiens
PGIGPPGARGPPGGQGPPGLSGPPGIKGEKGFPGFPGLD

SEQ ID NO: 570 - protein, 15 aa, Homo sapiens
EPGLPGIPGVSGPKG

SEQ ID NO: 571 - protein, 19 aa, Homo sapiens
GEKGQKGDTGPPGPPGLVI

SEQ ID NO: 572 - protein, 38 aa, Homo sapiens
LPGIGVQGPPGPPGIPGPIGQPGLHGIPGEKGDPGPPG

SEQ ID NO: 573 - protein, 14 aa, Homo sapiens
GSPGIPGHQGEMGP

SEQ ID NO: 574 - protein, 14 aa, Homo sapiens
EPGMQGEPGPPGPP

SEQ ID NO: 575 - protein, 18 aa, Homo sapiens
GPPGRLGAPGTPGLPGPR

SEQ ID NO: 576 - protein, 14 aa, Homo sapiens
PPGPKGFPGIPGPP

SEQ ID NO: 577 - protein, 14 aa, Homo sapiens
AKGQPGLPGFPGTP

SEQ ID NO: 578 - protein, 17 aa, Homo sapiens
DRGPPGPPGIRGPPGPP

SEQ ID NO: 579 - protein, 19 aa, Homo sapiens
PGPPGEKGKPGQDGIPGPA

SEQ ID NO: 580 - protein, 26 aa, Homo sapiens
LLGSKGEKGEPGLPGIPGVSGPKGYQ

SEQ ID NO: 581 - protein, 19 aa, Homo sapiens
DGLPGSMGPPGTPSVDHGF

SEQ ID NO: 582 - protein, 22 aa, Homo sapiens
TGPLGEKGERGYPGTPGPRGEP

SEQ ID NO: 583 - protein, 43 aa, Homo sapiens
GLQGIRGEPGPPGLPGSVGSPGVPGIGPPGARGPPGGQGPPGL

SEQ ID NO: 584 - protein, 28 aa, Homo sapiens
DPGLKGDKGDVGLPGKPGSMDKVDMGSM

SEQ ID NO: 585 - protein, 17 aa, Homo sapiens
LPGPMGPPGLPGIDGVK

SEQ ID NO: 586 - protein, 28 aa, Homo sapiens
GIRGEPGPPGLPGSVGSPGVPGIGPPGA

SEQ ID NO: 587 - protein, 28 aa, Homo sapiens
GFPGPPGPDGLPGSMGPPGTPSVDHGFL

SEQ ID NO: 588 - protein, 31 aa, Homo sapiens
GLQGIRGEPGPPGLPGSVGSPGVPGIGPPGA

SEQ ID NO: 589 - protein, 40 aa, Homo sapiens
GIRGEPGPPGLPGSVGSPGVPGIGPPGARGPPGGQGPPGL

SEQ ID NO: 590 - protein, 17 aa, Homo sapiens
EDGVIGMMGFPGAIGPP

SEQ ID NO: 591 - protein, 34 aa, Homo sapiens
YPGNPGILGPPGEDGVIGMMGFPGAIGPPGPPGN

SEQ ID NO: 592 - protein, 16 aa, Homo sapiens
IPPSDEICEPGPPGPP

SEQ ID NO: 593 - protein, 26 aa, Homo sapiens
LPGLPGPKGEPGLPGYPGNPGIKGSV

SEQ ID NO: 594 - protein, 19 aa, Homo sapiens
GIKGDKGSMGHPGPKGPPG

SEQ ID NO: 595 - protein, 22 aa, Homo sapiens
TPGSPGCAGSPGLPGSPGPPGP

SEQ ID NO: 596 - protein, 46 aa, Homo sapiens
PGAPGPQGLPGPPGFPGPVGPPGPPGFFGFPGAMGPRGPKGHMGER

SEQ ID NO: 597 - protein, 11 aa, Homo sapiens
GLPGFAGNPGP

SEQ ID NO: 598 - protein, 17 aa, Homo sapiens
GAEGLPGSPGFPGPQGD

SEQ ID NO: 599 - protein, 17 aa, Homo sapiens
MGPPGVPGFQGPKGLPG

SEQ ID NO: 600 - protein, 17 aa, Homo sapiens
DIDGYRGPPGPQGPPGE

SEQ ID NO: 601 - protein, 18 aa, Homo sapiens
GDQGDQGVPGAKGLPGPP

SEQ ID NO: 602 - protein, 18 aa, Homo sapiens
GDRGPQGQPGLPGLPGPM

SEQ ID NO: 603 - protein, 27 aa, Homo sapiens
EKGSIGIPGMPGSPGLKGSPGSVGYPG

SEQ ID NO: 604 - protein, 49 aa, Homo sapiens
GLQGIRGEPGPPGLPGSVGSPGVPGIGPPGARGPPGGQGPPGLSGPPGI

SEQ ID NO: 605 - protein, 19 aa, Homo sapiens
PGPPGLMGPPGPPGLPGPK

SEQ ID NO: 606 - protein, 23 aa, Homo sapiens
GERGSPGIPGAPGPIGPPGSPGL

SEQ ID NO: 607 - protein, 44 aa, Homo sapiens
PGIPGAPGAPGFPGSKGEPGDILTFPGMKGDKGELGSPGAPGLP

SEQ ID NO: 608 - protein, 18 aa, Homo sapiens
CDGGVPNTGPPGEPGPPG

SEQ ID NO: 609 - protein, 6 aa, Homo sapiens
IDGYRG

SEQ ID NO: 610 - protein, 6 aa, Homo sapiens
MGPPGT

SEQ ID NO: 611 - protein, 6 aa, Homo sapiens
DGLPGS

SEQ ID NO: 612 - protein, 6 aa, Homo sapiens
PGSKGE

SEQ ID NO: 613 - protein, 6 aa, Homo sapiens
RGFPGP

SEQ ID NO: 614 - protein, 6 aa, Homo sapiens
PGPPGL

SEQ ID NO: 615 - protein, 6 aa, Homo sapiens
GLPGSM

SEQ ID NO: 616 - protein, 6 aa, Homo sapiens
GLPGQQ

SEQ ID NO: 617 - protein, 6 aa, Homo sapiens
LGSKGE

SEQ ID NO: 618 - protein, 6 aa, Homo sapiens
PGIGVQ

SEQ ID NO: 619 - protein, 6 aa, Homo sapiens
SPGIPG

SEQ ID NO: 620 - protein, 6 aa, Homo sapiens
PGMQGE

SEQ ID NO: 621 - protein, 6 aa, Homo sapiens
PGPKGF

SEQ ID NO: 622 - protein, 6 aa, Homo sapiens
KGQPGL

SEQ ID NO: 623 - protein, 6 aa, Homo sapiens
PPSDEI

SEQ ID NO: 624 - protein, 6 aa, Homo sapiens
PGLKGD

SEQ ID NO: 625 - protein, 6 aa, Homo sapiens
GPLGEK

SEQ ID NO: 626 - protein, 6 aa, Homo sapiens
IRGEPG

SEQ ID NO: 627 - protein, 6 aa, Homo sapiens
FPGPPG

SEQ ID NO: 628 - protein, 6 aa, Homo sapiens
LQGIRG

SEQ ID NO: 629 - protein, 6 aa, Homo sapiens
DGVIGM

SEQ ID NO: 630 - protein, 6 aa, Homo sapiens
PGNPGI

SEQ ID NO: 631 - protein, 6 aa, Homo sapiens
IKGDKG

SEQ ID NO: 632 - protein, 6 aa, Homo sapiens
PGSPGC

SEQ ID NO: 633 - protein, 6 aa, Homo sapiens
GPPGVP

SEQ ID NO: 634 - protein, 6 aa, Homo sapiens
DQGDQG

SEQ ID NO: 635 - protein, 6 aa, Homo sapiens
KGSIGI

SEQ ID NO: 636 - protein, 6 aa, Homo sapiens
PPGRLG

SEQ ID NO: 637 - protein, 6 aa, Homo sapiens
EKGQKG

SEQ ID NO: 638 - protein, 6 aa, Homo sapiens
DGGVPN

SEQ ID NO: 639 - protein, 6 aa, Homo sapiens
SGRDGL

SEQ ID NO: 640 - protein, 6 aa, Homo sapiens
  MOD_RES (2)..(3): Proline or hydroxyproline
GXXGEK

SEQ ID NO: 641 - protein, 6 aa, Homo sapiens
AEGLPG

SEQ ID NO: 642 - protein, 6 aa, Homo sapiens
DGYRGP

SEQ ID NO: 643 - protein, 6 aa, Homo sapiens
GPPGLM

SEQ ID NO: 644 - protein, 6 aa, Homo sapiens
LPGFAG

SEQ ID NO: 645 - protein, 6 aa, Homo sapiens
GIPGMP

SEQ ID NO: 646 - protein, 6 aa, Homo sapiens
SVDHGF

SEQ ID NO: 647 - protein, 6 aa, Homo sapiens
PSVDHG

SEQ ID NO: 648 - protein, 6 aa, Homo sapiens
VDHGFL

SEQ ID NO: 649 - protein, 6 aa, Homo sapiens
PGQPGY

SEQ ID NO: 650 - protein, 6 aa, Homo sapiens
QPGYTN

SEQ ID NO: 651 - protein, 6 aa, Homo sapiens
PGLPGS

SEQ ID NO: 652 - protein, 6 aa, Homo sapiens
GTPSVD

SEQ ID NO: 653 - protein, 6 aa, Homo sapiens
SVGSPG

SEQ ID NO: 654 - protein, 6 aa, Homo sapiens
LPGSMG

SEQ ID NO: 655 - protein, 6 aa, Homo sapiens
PGFPGL

SEQ ID NO: 656 - protein, 6 aa, Homo sapiens
PGLPGE

SEQ ID NO: 657 - protein, 6 aa, Homo sapiens
HQGEMG

SEQ ID NO: 658 - protein, 6 aa, Homo sapiens
GPPGLV

SEQ ID NO: 659 - protein, 6 aa, Homo sapiens
PGIPGP

SEQ ID NO: 660 - protein, 6 aa, Homo sapiens
PGFPGT

SEQ ID NO: 661 - protein, 6 aa, Homo sapiens
DGIPGP

SEQ ID NO: 662 - protein, 6 aa, Homo sapiens
DGIPGP

SEQ ID NO: 663 - protein, 6 aa, Homo sapiens
PGPRGE

SEQ ID NO: 664 - protein, 6 aa, Homo sapiens
  MOD_RES (5)..(5): Proline or hydroxyproline
GQGPXG

SEQ ID NO: 665 - protein, 6 aa, Homo sapiens
KVDMGS

SEQ ID NO: 666 - protein, 6 aa, Homo sapiens
PGIDGV

SEQ ID NO: 667 - protein, 6 aa, Homo sapiens
KGHMGE

SEQ ID NO: 668 - protein, 6 aa, Homo sapiens
PGAIGP

SEQ ID NO: 669 - protein, 6 aa, Homo sapiens
KGLPGP

SEQ ID NO: 670 - protein, 6 aa, Homo sapiens
GPKGLP

SEQ ID NO: 671 - protein, 6 aa, Homo sapiens
GPKGPP

SEQ ID NO: 672 - protein, 6 aa, Homo sapiens
SPGPPG

SEQ ID NO: 673 - protein, 6 aa, Homo sapiens
GSVGYP

SEQ ID NO: 674 - protein, 6 aa, Homo sapiens
PPGSPG

SEQ ID NO: 675 - protein, 6 aa, Homo sapiens
GEPGPP

SEQ ID NO: 676 - protein, 6 aa, Homo sapiens
AGNPGP

SEQ ID NO: 677 - protein, 6 aa, Homo sapiens
PGIKGS

SEQ ID NO: 678 - protein, 6 aa, Homo sapiens
PGYTNG

SEQ ID NO: 679 - protein, 6 aa, Homo sapiens
FPGPQG

SEQ ID NO: 680 - protein, 6 aa, Homo sapiens
LSGPPG

SEQ ID NO: 681 - protein, 6 aa, Homo sapiens
GVMGTP

SEQ ID NO: 682 - protein, 6 aa, Homo sapiens
GVSGPK

SEQ ID NO: 683 - protein, 15 aa, Homo sapiens
  MOD_RES (4)..(4): Proline or hydroxyproline
  MOD_RES (6)..(6): Proline or hydroxyproline
  MOD_RES (9)..(9): Proline or hydroxyproline
KGDXGXPGXIGSLGH

SEQ ID NO: 684 - protein, 14 aa, Homo sapiens
GLRGIPGPVGEPGL

SEQ ID NO: 685 - protein, 17 aa, Homo sapiens
VIGPPGLQGLPGPPGEK

SEQ ID NO: 686 - protein, 17 aa, Homo sapiens
  MOD_RES (6)..(6): Proline or hydroxyproline
  MOD_RES (15)..(15): Proline or hydroxyproline
GKDGIXGPLGPLGPXGA

SEQ ID NO: 687 - protein, 16 aa, Homo sapiens
GLRGIPGPVGEPGLLG

SEQ ID NO: 688 - protein, 17 aa, Homo sapiens
GVLGPQGKTGEVGPLGE

SEQ ID NO: 689 - protein, 18 aa, Homo sapiens
KDGIPGPLGPLGPPGAAG

SEQ ID NO: 690 - protein, 17 aa, Homo sapiens
  MOD_RES (12)..(12): proline or hydroxyproline
GEDGERGAEGPXGPTGQ

SEQ ID NO: 691 - protein, 17 aa, Homo sapiens
  MOD_RES (6)..(6): Proline or hydroxyproline
  MOD_RES (9)..(9): Proline or hydroxyproline
  MOD_RES (11)..(11): Proline or hydroxyproline
  MOD_RES (15)..(15): Proline or hydroxyproline
GLQGPXGFXGXKGPXGH

SEQ ID NO: 692 - protein, 19 aa, Homo sapiens
PIGSLGHPGPPGVAGPLGQ

SEQ ID NO: 693 - protein, 16 aa, Homo sapiens
GIRGPPGTVIMMPFQF

SEQ ID NO: 694 - protein, 19 aa, Homo sapiens
  MOD_RES (6)..(6): proline or hydroxyproline
  MOD_RES (11)..(11): proline or hydroxyproline
  MOD_RES (15)..(15): proline or hydroxyproline
GQMGPXGPLGXSGLXGLKG

SEQ ID NO: 695 - protein, 20 aa, Homo sapiens
GLLGAPGQMGPPGPLGPSGL

SEQ ID NO: 696 - protein, 20 aa, Homo sapiens
  MOD_RES (6)..(6): proline or hydroxyproline
  MOD_RES (12)..(12): proline or hydroxyproline
  MOD_RES (18)..(18): proline or hydroxyproline
GLRGIXGPVGEXGLLGAXGQ

SEQ ID NO: 697 - protein, 20 aa, Homo sapiens
  MOD_RES (9)..(9): proline or hydroxyproline
  MOD_RES (15)..(15): proline or hydroxyproline
GLLGPRGSXGPTGRXGVTGI

SEQ ID NO: 698 - protein, 17 aa, Homo sapiens
GIRGPPGTVIMMPFQFA

SEQ ID NO: 699 - protein, 21 aa, Homo sapiens
GKDGIPGPLGPLGPPGAAGPS

SEQ ID NO: 700 - protein, 23 aa, Homo sapiens
  MOD_RES (8)..(8): proline or hydroxyproline
  MOD_RES (15)..(15): proline or hydroxyproline
GKDGIPGXLGPLGPXGAAGPSGE

SEQ ID NO: 701 - protein, 24 aa, Homo sapiens
  MOD_RES (13)..(13): lysine or hydroxylysine
  MOD_RES (19)..(19): proline or hydroxyproline
QGLPGLEGREGAXGELGPXGPLGK

SEQ ID NO: 702 - protein, 30 aa, Homo sapiens
  MOD_RES (7)..(7): lysine or hydroxylysine
  MOD_RES (16)..(16): proline or hydroxyproline
  MOD_RES (24)..(24): proline or hydroxyproline
LGPIGEXGKSGKTGQXGLEGERGXPGSRGE

SEQ ID NO: 703 - protein, 32 aa, Homo sapiens
  MOD_RES (8)..(8): proline or hydroxyproline
  MOD_RES (12)..(12): proline or hydroxyproline
  MOD_RES (18)..(18): proline or hydroxyproline
  MOD_RES (21)..(21): methionine or oxidised methionine
  MOD_RES (23)..(23): proline or hydroxyproline
GLRGIPGXVGEXGLLGAXGQXGXPGPLGPSGL

SEQ ID NO: 704 - protein, 35 aa, Homo sapiens
  MOD_RES (6)..(6): proline or hydroxyproline
  MOD_RES (21)..(21): proline or hydroxyproline
GANGSXGERGPLGPAGGIGLXGQSGSEGPVGPAGK

SEQ ID NO: 705 - protein, 38 aa, Homo sapiens
  MOD_RES (6)..(6): proline or hydroxyproline
  MOD_RES (11)..(12): proline or hydroxyproline
  MOD_RES (15)..(15): proline or hydroxyproline
  MOD_RES (18)..(18): proline or hydroxyproline
  MOD_RES (21)..(21): proline or hydroxyproline
  MOD_RES (26)..(26): proline or hydroxyproline
GLIGTXGEKGXXGNXGIXGLXGSDGXLGHPGHEGPTGE

SEQ ID NO: 706 - protein, 11 aa, Homo sapiens
  MOD_RES (3)..(3): proline or hydroxyproline
  MOD_RES (6)..(6): proline or hydroxyproline
GLXGEXGPRGL

SEQ ID NO: 707 - protein, 12 aa, Homo sapiens
  MOD_RES (10)..(10): methionine or oxidised methionine
LALRGPAGPXGL

SEQ ID NO: 708 - protein, 13 aa, Homo sapiens
  MOD_RES (11)..(11): methionine or oxidised methionine
RLALRGPAGPXGL

SEQ ID NO: 709 - protein, 17 aa, Homo sapiens
  MOD_RES (6)..(6): proline or hydroxyproline
  MOD_RES (12)..(12): proline or hydroxyproline
GLTGRXGPVGPXGSGGL

SEQ ID NO: 710 - protein, 17 aa, Homo sapiens
  MOD_RES (6)..(6): lysine or hydroxylysine
  MOD_RES (11)..(12): proline or hydroxyproline
  MOD_RES (14)..(14): proline or hydroxyproline
GLLGPXGPPGXXGXPGV

SEQ ID NO: 711 - protein, 17 aa, Homo sapiens
  MOD_RES (3)..(3): proline or hydroxyproline
  MOD_RES (6)..(6): proline or hydroxyproline
  MOD_RES (14)..(14): proline or hydroxyproline
GIXGRXGPQGPPGXAGE

SEQ ID NO: 712 - protein, 17 aa, Homo sapiens
  MOD_RES (3)..(3): proline or hydroxyproline
  MOD_RES (6)..(6): proline or hydroxyproline
  MOD_RES (13)..(13): proline or hydroxyproline
  MOD_RES (16)..(16): proline or hydroxyproline
PGXDGXPGPMGPXGLXG

SEQ ID NO: 713 - protein, 17 aa, Homo sapiens
  MOD_RES (3)..(3): proline or hydroxyproline
  MOD_RES (12)..(12): proline or hydroxyproline
GQXGPSGADGEXGPRGQ

SEQ ID NO: 714 - protein, 17 aa, Homo sapiens
  MOD_RES (12)..(12): proline or hydroxyproline
  MOD_RES (15)..(15): proline or hydroxyproline
GETGFQGKTGPXGPXGV

SEQ ID NO: 715 - protein, 16 aa, Homo sapiens
  MOD_RES (6)..(6): proline or hydroxyproline
  MOD_RES (12)..(12): proline or hydroxyproline
GLRGFXGDRGLXGPVG

SEQ ID NO: 716 - protein, 17 aa, Homo sapiens
  MOD_RES (6)..(6): proline or hydroxyproline
  MOD_RES (12)..(12): proline or hydroxyproline
GLRGFXGDRGLXGPVGA

SEQ ID NO: 717 - protein, 20 aa, Homo sapiens
  MOD_RES (12)..(12): proline or hydroxyproline
  MOD_RES (15)..(15): proline or hydroxyproline
GKTGPIGPQGAXGKXGPDGL

SEQ ID NO: 718 - protein, 20 aa, Homo sapiens
  MOD_RES (2)..(3): proline or hydroxyproline
  MOD_RES (6)..(6): proline or hydroxyproline
  MOD_RES (9)..(9): proline or hydroxyproline
  MOD_RES (17)..(18): proline or hydroxyproline
GXXGRXGLPGADGLPGXXGT

SEQ ID NO: 719 - protein, 21 aa, Homo sapiens
  MOD_RES (3)..(3): lysine or hydroxylysine
  MOD_RES (12)..(12): proline or hydroxyproline
GLXGNEGPPGPXGPAGSPGER

SEQ ID NO: 720 - protein, 20 aa, Homo sapiens
  MOD_RES (6)..(6): proline or hydroxyproline
  MOD_RES (12)..(12): proline or hydroxyproline
GLRGFXGDRGLXGPVGALGL

SEQ ID NO: 721 - protein, 20 aa, Homo sapiens
  MOD_RES (6)..(6): proline or hydroxyproline
  MOD_RES (9)..(9): proline or hydroxyproline
  MOD_RES (12)..(12): proline or hydroxyproline
  MOD_RES (18)..(18): proline or hydroxyproline
GERGHXGPXGPXGEQGLXGL

SEQ ID NO: 722 - protein, 21 aa, Homo sapiens
  MOD_RES (4)..(4): proline or hydroxyproline
  MOD_RES (10)..(10): lysine or hydroxylysine
  MOD_RES (16)..(16): proline or hydroxyproline
IGPXGEQGEXGDRGLXGPQGS

SEQ ID NO: 723 - protein, 24 aa, Homo sapiens
  MOD_RES (9)..(9): proline or hydroxyproline
  MOD_RES (11)..(12): proline or hydroxyproline
  MOD_RES (14)..(14): proline or hydroxyproline
GEAGHPGPXGXXGXPGEVIQPLPI

SEQ ID NO: 724 - protein, 26 aa, Homo sapiens
  MOD_RES (2)..(2): proline or hydroxyproline
  MOD_RES (5)..(5): lysine or hydroxylysine
  MOD_RES (22)..(22): proline or hydroxyproline
  MOD_RES (25)..(25): proline or hydroxyproline
KXGPXGNSGGDGPAGPPGERGXNGXQ

SEQ ID NO: 725 - protein, 26 aa, Homo sapiens
  MOD_RES (6)..(6): proline or hydroxyproline
  MOD_RES (9)..(9): proline or hydroxyproline
  MOD_RES (18)..(18): methionine or oxidised methionine
  MOD_RES (21)..(21): proline or hydroxyproline
  MOD_RES (24)..(24): proline or hydroxyproline
GEQGLXGSXGPDGPPGPXGPXGLXGL

SEQ ID NO: 726 - protein, 27 aa, Homo sapiens
  MOD_RES (3)..(4): proline or hydroxyproline
  MOD_RES (12)..(12): proline or hydroxyproline
  MOD_RES (24)..(24): proline or hydroxyproline
EGXXGEKGGQGXPGPQGPIGYPGXRGV

SEQ ID NO: 727 - protein, 26 aa, Homo sapiens
  MOD_RES (3)..(3): proline or hydroxyproline
  MOD_RES (5)..(5): proline or hydroxyproline
  MOD_RES (8)..(8): proline or hydroxyproline
  MOD_RES (12)..(12): proline or hydroxyproline
  MOD_RES (18)..(18): proline or hydroxyproline
  MOD_RES (21)..(21): proline or hydroxyproline
GFXGXKGXPGPXGKDGLXGHXGQRGE

SEQ ID NO: 728 - protein, 11 aa, Homo sapiens
LPFRFGGGGDA

SEQ ID NO: 729 - protein, 11 aa, Homo sapiens
GSKGPMVSAQE

SEQ ID NO: 730 - protein, 11 aa, Homo sapiens
QESQAQAILQQ

SEQ ID NO: 731 - protein, 14 aa, Homo sapiens
  MOD_RES (6)..(6): proline or hydroxyproline
  MOD_RES (9)..(9): lysine or hydroxylysine
GAIGPXGEXGPLGK

SEQ ID NO: 732 - protein, 15 aa, Homo sapiens
  MOD_RES (3)..(3): proline or hydroxyproline
  MOD_RES (13)..(13): proline or hydroxyproline
GGXNGDPGPLGPXGE

SEQ ID NO: 733 - protein, 14 aa, Homo sapiens
  MOD_RES (2)..(2): proline or hydroxyproline
  MOD_RES (4)..(5): proline or hydroxyproline
  MOD_RES (11)..(11): proline or hydroxyproline
PXGXXGEQGLXGLA

SEQ ID NO: 734 - protein, 17 aa, Homo sapiens
  MOD_RES (11)..(12): proline or hydroxyproline
  MOD_RES (14)..(14): proline or hydroxyproline
GLLGPKGPPGXXGXPGV

SEQ ID NO: 735 - protein, 17 aa, Homo sapiens
  MOD_RES (6)..(6): proline or hydroxyproline
  MOD_RES (12)..(12): proline or hydroxyproline
GQQGNXGAQGLXGPQGA

SEQ ID NO: 736 - protein, 17 aa, Homo sapiens
  MOD_RES (2)..(2): lysine or hydroxylysine
  MOD_RES (5)..(5): proline or hydroxyproline
  MOD_RES (15)..(15): proline or hydroxyproline
GXEGXPGEKGGQGPXGP

SEQ ID NO: 737 - protein, 17 aa, Homo sapiens
  MOD_RES (12)..(12): proline or hydroxyproline
  MOD_RES (15)..(15): proline or hydroxyproline
GETGFQGKTGPXGPXGV

SEQ ID NO: 738 - protein, 17 aa, Homo sapiens
  MOD_RES (3)..(3): lysine or hydroxylysine
  MOD_RES (6)..(6): proline or hydroxyproline
  MOD_RES (15)..(15): proline or hydroxyproline
GEXGHXGLIGLIGPXGE

SEQ ID NO: 739 - protein, 20 aa, Homo sapiens
  MOD_RES (12)..(12): proline or hydroxyproline
  MOD_RES (15)..(15): proline or hydroxyproline
GKTGPIGPQGAXGKXGPDGL

SEQ ID NO: 740 - protein, 20 aa, Homo sapiens
  MOD_RES (3)..(3): proline or hydroxyproline
  MOD_RES (6)..(6): proline or hydroxyproline
  MOD_RES (12)..(13): proline or hydroxyproline
  MOD_RES (16)..(16): proline or hydroxyproline
PGXDGXPGPMGXXGLXGLKG

SEQ ID NO: 741 - protein, 26 aa, Homo sapiens
  MOD_RES (15)..(15): proline or hydroxyproline
  MOD_RES (17)..(17): proline or hydroxyproline
  MOD_RES (20)..(21): proline or hydroxyproline
GERGPNGPQGPTGFXGXKGXXGPPGK

SEQ ID NO: 742 - protein, 26 aa, Homo sapiens
  MOD_RES (7)..(8): proline or hydroxyproline
LIGLIGXXGEQGEKGDRGLPGPQGSS

SEQ ID NO: 743 - protein, 31 aa, Homo sapiens
  MOD_RES (4)..(4): proline or hydroxyproline
  MOD_RES (6)..(7): proline or hydroxyproline
IGPXGXXGLPGPPGPKGAKGSSGPTGPKGEA

SEQ ID NO: 744 - protein, 30 aa, Homo sapiens
  MOD_RES (4)..(5): proline or hydroxyproline
  MOD_RES (8)..(8): lysine or hydroxylysine
  MOD_RES (14)..(14): proline or hydroxyproline
PLGXXGEXGKLGVXGLPGYPGRQGPKGSIG

SEQ ID NO: 745 - protein, 33 aa, Homo sapiens
  MOD_RES (13)..(13): proline or hydroxyproline
  MOD_RES (19)..(19): lysine or hydroxylysine
  MOD_RES (25)..(25): proline or hydroxyproline
  MOD_RES (28)..(28): proline or hydroxyproline
QGPKGSIGFPGFXGANGEXGGRGTXGKXGPRGQ

SEQ ID NO: 746 - protein, 15 aa, Homo sapiens
  MOD_RES (10)..(10): proline or hydroxyproline
PGPKGDPGPXGPIGS

SEQ ID NO: 747 - protein, 14 aa, Homo sapiens
  MOD_RES (2)..(2): proline or hydroxyproline
  MOD_RES (5)..(5): proline or hydroxyproline
  MOD_RES (11)..(11): proline or hydroxyproline
AXGIXGEKGLXGLQ

SEQ ID NO: 748 - protein, 16 aa, Homo sapiens
  MOD_RES (3)..(4): proline or hydroxyproline
  MOD_RES (6)..(6): proline or hydroxyproline
  MOD_RES (10)..(10): proline or hydroxyproline
  MOD_RES (12)..(12): proline or hydroxyproline
  MOD_RES (15)..(15): proline or hydroxyproline
QGXXGXKGDXGXPGXI

SEQ ID NO: 749 - protein, 17 aa, Homo sapiens
  MOD_RES (6)..(6): proline or hydroxyproline
  MOD_RES (9)..(9): proline or hydroxyproline
GSLGHXGPXGVAGPLGQ

SEQ ID NO: 750 - protein, 17 aa, Homo sapiens
  MOD_RES (12)..(12): proline or hydroxyproline
GELGFQGQTGPXGPAGV

SEQ ID NO: 751 - protein, 17 aa, Homo sapiens
  MOD_RES (3)..(3): lysine or hydroxylysine
  MOD_RES (15)..(15): proline or hydroxyproline
GEXGHIGLIGLIGPXGE

SEQ ID NO: 752 - protein, 20 aa, Homo sapiens
  MOD_RES (2)..(2): proline or hydroxyproline
  MOD_RES (12)..(12): proline or hydroxyproline
GXVGEPGLLGAXGQMGPPGP

SEQ ID NO: 753 - protein, 26 aa, Homo sapiens
  MOD_RES (11)..(11): proline or hydroxyproline
  MOD_RES (14)..(14): lysine or hydroxylysine
  MOD_RES (18)..(18): proline or hydroxyproline
GSRGERGPPGXTGXDGIXGPLGPLGP

SEQ ID NO: 754 - protein, 26 aa, Homo sapiens
  MOD_RES (5)..(5): lysine or hydroxylysine
  MOD_RES (12)..(12): proline or hydroxyproline
  MOD_RES (21)..(21): proline or hydroxyproline
GEKGXSGKTGQXGLEGERGPXGSRGE

SEQ ID NO: 755 - protein, 10 aa, Homo sapiens
  MOD_RES (2)..(2): proline or hydroxyproline
  MOD_RES (5)..(5): proline or hydroxyproline
LXGEXGPRGL

SEQ ID NO: 756 - protein, 11 aa, Homo sapiens
  MOD_RES (9)..(9): methionine or oxidised methionine
ALRGPAGPXGL

SEQ ID NO: 757 - protein, 35 aa, Homo sapiens
  MOD_RES (8)..(9): proline or hydroxyproline
  MOD_RES (14)..(14): proline or hydroxyproline
  MOD_RES (18)..(18): proline or hydroxyproline
  MOD_RES (21)..(21): proline or hydroxyproline
  MOD_RES (23)..(23): methionine or oxidised methionine
  MOD_RES (24)..(24): proline or hydroxyproline
  MOD_RES (29)..(30): proline or hydroxyproline
  MOD_RES (33)..(33): proline or hydroxyproline
GPQGAIGXXGEKGXLGKXGLXGXXGADGXXGHXGK

SEQ ID NO: 758 - protein, 36 aa, Homo sapiens
  MOD_RES (15)..(16): proline or hydroxyproline
  MOD_RES (22)..(22): lysine or hydroxylysine
  MOD_RES (25)..(25): proline or hydroxyproline
AGPMGLTGRPGPVGXXGSGGLXGEXGDVGPQGPRGV

SEQ ID NO: 759 - protein, 35 aa, Homo sapiens
  MOD_RES (8)..(8): proline or hydroxyproline
  MOD_RES (12)..(12): proline or hydroxyproline
  MOD_RES (18)..(18): proline or hydroxyproline
  MOD_RES (21)..(21): methionine or oxidised methionine
  MOD_RES (23)..(24): proline or hydroxyproline
GLRGIPGXVGEXGLLGAXGQXGXXGPLGPSGLPGL

SEQ ID NO: 760 - protein, 6 aa, Homo sapiens
  MOD_RES (5)..(5): proline or hydroxyproline
LRGIXG

SEQ ID NO: 761 - protein, 6 aa, Homo sapiens
IGPPGI

SEQ ID NO: 762 - protein, 6 aa, Homo sapiens
IGSLGH

SEQ ID NO: 763 - protein, 6 aa, Homo sapiens
IRGPPG

SEQ ID NO: 764 - protein, 6 aa, Homo sapiens
  MOD_RES (5)..(5): proline or hydroxyproline
ANGSXG

SEQ ID NO: 765 - protein, 6 aa, Homo sapiens
  MOD_RES (5)..(5): proline or hydroxyproline
LIGTXG

SEQ ID NO: 766 - protein, 6 aa, Homo sapiens
  MOD_RES (2)..(2): proline or hydroxyproline
  MOD_RES (5)..(5): proline or hydroxyproline
LXGEXG

SEQ ID NO: 767 - protein, 6 aa, Homo sapiens
  MOD_RES (2)..(2): proline or hydroxyproline
  MOD_RES (5)..(5): proline or hydroxyproline
IXGRXG

SEQ ID NO: 768 - protein, 6 aa, Homo sapiens
  MOD_RES (2)..(2): proline or hydroxyproline
  MOD_RES (5)..(5): proline or hydroxyproline
GXDGXP

SEQ ID NO: 769 - protein, 6 aa, Homo sapiens
  MOD_RES (2)..(2): proline or hydroxyproline
QXGPSG

SEQ ID NO: 770 - protein, 6 aa, Homo sapiens
  MOD_RES (2)..(2): lysine or hydroxylysine
LXGNEG

SEQ ID NO: 771 - protein, 6 aa, Homo sapiens
  MOD_RES (5)..(5): proline or hydroxyproline
ERGHXG

SEQ ID NO: 772 - protein, 6 aa, Homo sapiens
  MOD_RES (3)..(3): proline or hydroxyproline
GPXGEQ

SEQ ID NO: 773 - protein, 6 aa, Homo sapiens
PFRFGG

SEQ ID NO: 774 - protein, 6 aa, Homo sapiens
ESQAQA

SEQ ID NO: 775 - protein, 6 aa, Homo sapiens
  MOD_RES (5)..(5): lysine or hydroxylysine
LLGPXG

SEQ ID NO: 776 - protein, 6 aa, Homo sapiens
  MOD_RES (5)..(5): proline or hydroxyproline
QQGNXG

SEQ ID NO: 777 - protein, 6 aa, Homo sapiens
  MOD_RES (1)..(1): lysine or hydroxylysine
  MOD_RES (4)..(4): proline or hydroxyproline
XEGXPG

SEQ ID NO: 778 - protein, 6 aa, Homo sapiens
  MOD_RES (6)..(6): proline or hydroxyproline
IGLIGX

SEQ ID NO: 779 - protein, 6 aa, Homo sapiens
  MOD_RES (3)..(4): proline or hydroxyproline
LGXXGE

SEQ ID NO: 780 - protein, 6 aa, Homo sapiens
  MOD_RES (2)..(3): proline or hydroxyproline
  MOD_RES (5)..(5): proline or hydroxyproline
GXXGXK

SEQ ID NO: 781 - protein, 6 aa, Homo sapiens
  MOD_RES (5)..(5): proline or hydroxyproline
SLGHXG

SEQ ID NO: 782 - protein, 6 aa, Homo sapiens
  MOD_RES (5)..(5): proline or hydroxyproline
KDGIXG

SEQ ID NO: 783 - protein, 6 aa, Homo sapiens
  MOD_RES (5)..(5): proline or hydroxyproline
PVGEPG

SEQ ID NO: 784 - protein, 6 aa, Homo sapiens
  MOD_RES (1)..(1): proline or hydroxyproline
  MOD_RES (4)..(4): proline or hydroxyproline
XGEXGP

SEQ ID NO: 785 - protein, 6 aa, Homo sapiens
  MOD_RES (5)..(5): proline or hydroxyproline
LLGAXG

SEQ ID NO: 786 - protein, 6 aa, Homo sapiens
GLPGLE

SEQ ID NO: 787 - protein, 6 aa, Homo sapiens
GIPGEK

SEQ ID NO: 788 - protein, 6 aa, Homo sapiens
LALRGP

SEQ ID NO: 789 - protein, 6 aa, Homo sapiens
  MOD_RES (5)..(5): proline or hydroxyproline
LTGRXG

SEQ ID NO: 790 - protein, 6 aa, Homo sapiens
  MOD_RES (5)..(5): proline or hydroxyproline
LRGFXG

SEQ ID NO: 791 - protein, 6 aa, Homo sapiens
KTGPIG

SEQ ID NO: 792 - protein, 6 aa, Homo sapiens
  MOD_RES (1)..(2): proline or hydroxyproline
  MOD_RES (5)..(5): proline or hydroxyproline
XXGRXG

SEQ ID NO: 793 - protein, 6 aa, Homo sapiens
  MOD_RES (5)..(5): proline or hydroxyproline
EQGLXG

SEQ ID NO: 794 - protein, 6 aa, Homo sapiens
  MOD_RES (6)..(6): proline or hydroxyproline
AIGGPX

SEQ ID NO: 795 - protein, 6 aa, Homo sapiens
  MOD_RES (2)..(2): proline or hydroxyproline
GXNGDP

SEQ ID NO: 796 - protein, 6 aa, Homo sapiens
  MOD_RES (1)..(1): proline or hydroxyproline
  MOD_RES (3)..(4): proline or hydroxyproline
XGXXGE

SEQ ID NO: 797 - protein, 6 aa, Homo sapiens
LLGPRG

SEQ ID NO: 798 - protein, 6 aa, Homo sapiens
ERGPNG

SEQ ID NO: 799 - protein, 6 aa, Homo sapiens
GPKGDP

SEQ ID NO: 800 - protein, 6 aa, Homo sapiens
  MOD_RES (1)..(1): proline or hydroxyproline
  MOD_RES (4)..(4): proline or hydroxyproline
XGIXGE

SEQ ID NO: 801 - protein, 6 aa, Homo sapiens
  MOD_RES (2)..(2): lysine or hydroxylysine
EXGHIG

SEQ ID NO: 802 - protein, 6 aa, Homo sapiens
  MOD_RES (5)..(5): proline or hydroxyproline
QMGPXG

SEQ ID NO: 803 - protein, 6 aa, Homo sapiens
SRGERG

SEQ ID NO: 804 - protein, 6 aa, Homo sapiens
  MOD_RES (4)..(4): lysine or hydroxylysine
EKGXSG

SEQ ID NO: 805 - protein, 6 aa, Homo sapiens
  MOD_RES (6)..(6): lysine or hydroxylysine
GPIGEX

SEQ ID NO: 806 - protein, 6 aa, Homo sapiens
PQGAIG

SEQ ID NO: 807 - protein, 6 aa, Homo sapiens
GPMGLT

SEQ ID NO: 808 - protein, 6 aa, Homo sapiens
ETGFQG

SEQ ID NO: 809 - protein, 6 aa, Homo sapiens
GSKGPM

SEQ ID NO: 810 - protein, 6 aa, Homo sapiens
ALRGPA

SEQ ID NO: 811 - protein, 6 aa, Homo sapiens
EAGHPG

SEQ ID NO: 812 - protein, 6 aa, Homo sapiens
  MOD_RES (2)..(2): lysine or hydroxylysine
  MOD_RES (5)..(5): proline or hydroxyproline
EXGHXG

SEQ ID NO: 813 - protein, 5 aa, Homo sapiens
KDGIP

SEQ ID NO: 814 - protein, 6 aa, Homo sapiens
VLGPQG

SEQ ID NO: 815 - protein, 6 aa, Homo sapiens
EDGERG

SEQ ID NO: 816 - protein, 6 aa, Homo sapiens
GPKGSI

SEQ ID NO: 817 - protein, 6 aa, Homo sapiens
ELGFQG

SEQ ID NO: 818 - protein, 6 aa, Homo sapiens
LRGPAG

SEQ ID NO: 819 - protein, 6 aa, Homo sapiens
PIGSLG

SEQ ID NO: 820 - protein, 6 aa, Homo sapiens
  MOD_RES (2)..(2): proline or hydroxyproline
PXGPTG

SEQ ID NO: 821 - protein, 6 aa, Homo sapiens
  MOD_RES (1)..(1): proline or hydroxyproline
  MOD_RES (5)..(5): proline or hydroxyproline
XKGPXG

SEQ ID NO: 822 - protein, 6 aa, Homo sapiens
VAGPLG

SEQ ID NO: 823 - protein, 6 aa, Homo sapiens
  MOD_RES (2)..(2): proline or hydroxyproline
RXGVTG

SEQ ID NO: 824 - protein, 6 aa, Homo sapiens
MMPFQF

SEQ ID NO: 825 - protein, 6 aa, Homo sapiens
PGAAGP

SEQ ID NO: 826 - protein, 6 aa, Homo sapiens
PVGPAG

SEQ ID NO: 827 - protein, 6 aa, Homo sapiens
HEGPTG

SEQ ID NO: 828 - protein, 6 aa, Homo sapiens
  MOD_RES (3)..(3): proline or hydroxyproline
  MOD_RES (6)..(6): proline or hydroxyproline
GPXGLX

SEQ ID NO: 829 - protein, 6 aa, Homo sapiens
AGSPGE

SEQ ID NO: 830 - protein, 6 aa, Homo sapiens
PVGALG

SEQ ID NO: 831 - protein, 6 aa, Homo sapiens
  MOD_RES (4)..(4): proline or hydroxyproline
YPGXRG

SEQ ID NO: 832 - protein, 6 aa, Homo sapiens
  MOD_RES (2)..(2): proline or hydroxyproline
HXGQRG

SEQ ID NO: 833 - protein, 6 aa, Homo sapiens
GGGGDA

SEQ ID NO: 834 - protein, 6 aa, Homo sapiens
  MOD_RES (5)..(5): proline or hydroxyproline
LIGPXG

SEQ ID NO: 835 - protein, 6 aa, Homo sapiens
  MOD_RES (3)..(3): proline or hydroxyproline
GLXGLK

SEQ ID NO: 836 - protein, 6 aa, Homo sapiens
  MOD_RES (4)..(4): proline or hydroxyproline
KGLXGL

SEQ ID NO: 837 - protein, 6 aa, Homo sapiens
QQARLA

SEQ ID NO: 838 - protein, 6 aa, Homo sapiens
  MOD_RES (1)..(2): proline or hydroxyproline
  MOD_RES (5)..(5): proline or hydroxyproline
XXGHXG

SEQ ID NO: 839 - protein, 6 aa, Homo sapiens
  MOD_RES (5)..(5): proline or hydroxyproline
PLGPXG

SEQ ID NO: 840 - protein, 6 aa, Homo sapiens
GEPGLL

SEQ ID NO: 841 - protein, 6 aa, Homo sapiens
EVGPLG

SEQ ID NO: 842 - protein, 6 aa, Homo sapiens
IMMPFQ

SEQ ID NO: 843 - protein, 6 aa, Homo sapiens
PLGPSG

SEQ ID NO: 844 - protein, 6 aa, Homo sapiens
AAGPSG

SEQ ID NO: 845 - protein, 6 aa, Homo sapiens
  MOD_RES (2)..(2): proline or hydroxyproline
PXGPLG

SEQ ID NO: 846 - protein, 6 aa, Homo sapiens
  MOD_RES (1)..(1): proline or hydroxyproline
  MOD_RES (2)..(2): proline or hydroxyproline
XXGSRG

SEQ ID NO: 847 - protein, 6 aa, Homo sapiens
  MOD_RES (5)..(5): methionine or oxidised methionine
PAGPXG

SEQ ID NO: 848 - protein, 6 aa, Homo sapiens
  MOD_RES (2)..(2): proline or hydroxyproline
PXGSGG

SEQ ID NO: 849 - protein, 6 aa, Homo sapiens
  MOD_RES (3)..(3): proline or hydroxyproline
GLXGPV

SEQ ID NO: 850 - protein, 6 aa, Homo sapiens
  MOD_RES (2)..(2): proline or hydroxyproline
LXGPVG

SEQ ID NO: 851 - protein, 6 aa, Homo sapiens
  MOD_RES (2)..(2): proline or hydroxyproline
KXGPDG

SEQ ID NO: 852 - protein, 6 aa, Homo sapiens
  MOD_RES (2)..(2): proline or hydroxyproline
LXGPQG

SEQ ID NO: 853 - protein, 6 aa, Homo sapiens
VIQPLP

SEQ ID NO: 854 - protein, 6 aa, Homo sapiens
RGPNGP

SEQ ID NO: 855 - protein, 6 aa, Homo sapiens
PGPQGS

SEQ ID NO: 856 - protein, 6 aa, Homo sapiens
  MOD_RES (2)..(2): Lysine or hydroxylysine
EXGPLG

SEQ ID NO: 857 - protein, 6 aa, Homo sapiens
GPPGAA

SEQ ID NO: 858 - protein, 6 aa, Homo sapiens
TGPKGE

SEQ ID NO: 859 - protein, 6 aa, Homo sapiens
  MOD_RES (4)..(4): proline or hydroxyproline
QGLXGL

SEQ ID NO: 860 - protein, 6 aa, Homo sapiens
PSGLPG

SEQ ID NO: 861 - protein, 6 aa, Homo sapiens
  MOD_RES (2)..(2): proline or hydroxyproline
  MOD_RES (5)..(5): proline or hydroxyproline
PXGLXG

SEQ ID NO: 862 - protein, 6 aa, Homo sapiens
  MOD_RES (2)..(2): proline or hydroxyproline
KXGPRG

SEQ ID NO: 863 - protein, 6 aa, Homo sapiens
PLGPLG

SEQ ID NO: 864 - protein, 14 aa, Homo sapiens
GYRGPEGPQGPPGH

SEQ ID NO: 865 - protein, 16 aa, Homo sapiens
GPIGPKGYRGDEGPPG

SEQ ID NO: 866 - protein, 12 aa, Homo sapiens
IGIGIGNADITE

SEQ ID NO: 867 - protein, 14 aa, Homo sapiens
GAQGPAGPAGPPGL

SEQ ID NO: 868 - protein, 14 aa, Homo sapiens
GLIGEQGISGPRGS

SEQ ID NO: 869 - protein, 15 aa, Homo sapiens
PPGLIGEQGISGPRG

SEQ ID NO: 870 - protein, 16 aa, Homo sapiens
EPGEPGPKGGIGNRGP

SEQ ID NO: 871 - protein, 26 aa, Homo sapiens
GISGPRGSGGAAGAPGERGRTGPLGR

SEQ ID NO: 872 - protein, 14 aa, Homo sapiens
PGPAGPPGDPGLMG

SEQ ID NO: 873 - protein, 28 aa, Homo sapiens
VAAKPAAVRPPAAAAAKPVATKPEVPRP

SEQ ID NO: 874 - protein, 14 aa, Homo sapiens
GEPGLNGTTGPKGI

SEQ ID NO: 875 - protein, 17 aa, Homo sapiens
IGPKGIPGEDGYRGYPG

SEQ ID NO: 876 - protein, 26 aa, Homo sapiens
VAVVQHAPSESVDNASMPPVKVEFSL

SEQ ID NO: 877 - protein, 10 aa, Homo sapiens
LGPMGVPGRD

SEQ ID NO: 878 - protein, 28 aa, Homo sapiens
GEPGPPGEKGEAGDEGNPGPDGAPGERG

SEQ ID NO: 879 - protein, 28 aa, Homo sapiens
RGPIGSIGPKGIPGEDGYRGYPGDEGGP

SEQ ID NO: 880 - protein, 11 aa, Homo sapiens
PPPPQPARSAS

SEQ ID NO: 881 - protein, 12 aa, Homo sapiens
FGPSAATPAPPG

SEQ ID NO: 882 - protein, 29 aa, Homo sapiens
GPKGETGDLGPMGVPGRDGVPGGPGETGK

SEQ ID NO: 883 - protein, 6 aa, Homo sapiens
YRGPEG

SEQ ID NO: 884 - protein, 16 aa, Homo sapiens
SSGIENGAFQGMKKLS

SEQ ID NO: 885 - protein, 6 aa, Homo sapiens
GIGIGN

SEQ ID NO: 886 - protein, 6 aa, Homo sapiens
ISGPRG

SEQ ID NO: 887 - protein, 6 aa, Homo sapiens
PGPAGP

SEQ ID NO: 888 - protein, 6 aa, Homo sapiens
VAAKPA

SEQ ID NO: 889 - protein, 6 aa, Homo sapiens
RGPIGS

SEQ ID NO: 890 - protein, 6 aa, Homo sapiens
PPPPQP

SEQ ID NO: 891 - protein, 6 aa, Homo sapiens
AQGPAG

SEQ ID NO: 892 - protein, 6 aa, Homo sapiens
LIGEQG

SEQ ID NO: 893 - protein, 6 aa, Homo sapiens
PGLIGE

SEQ ID NO: 894 - protein, 6 aa, Homo sapiens
GEPGLN

SEQ ID NO: 895 - protein, 6 aa, Homo sapiens
IGPKGI

SEQ ID NO: 896 - protein, 6 aa, Homo sapiens
VAVVQH

SEQ ID NO: 897 - protein, 6 aa, Homo sapiens
FGPSAA

SEQ ID NO: 898 - protein, 6 aa, Homo sapiens
GPKGET

SEQ ID NO: 899 - protein, 6 aa, Homo sapiens
LGPMGV

SEQ ID NO: 900 - protein, 6 aa, Homo sapiens
GDEGPP

SEQ ID NO: 901 - protein, 6 aa, Homo sapiens
GNADIT

SEQ ID NO: 902 - protein, 6 aa, Homo sapiens
DPGLMG

SEQ ID NO: 903 - protein, 6 aa, Homo sapiens
PEVPRP

SEQ ID NO: 904 - protein, 6 aa, Homo sapiens
TGPKGI

SEQ ID NO: 905 - protein, 6 aa, Homo sapiens
GDEGGP

SEQ ID NO: 906 - protein, 6 aa, Homo sapiens
PARSAS

SEQ ID NO: 907 - protein, 6 aa, Homo sapiens
GISGPR

SEQ ID NO: 908 - protein, 6 aa, Homo sapiens
GIGNRG

SEQ ID NO: 909 - protein, 6 aa, Homo sapiens
YRGYPG

SEQ ID NO: 910 - protein, 6 aa, Homo sapiens
KVEFSL

SEQ ID NO: 911 - protein, 6 aa, Homo sapiens
GVPGRD

SEQ ID NO: 912 - protein, 6 aa, Homo sapiens
PGETGK

SEQ ID NO: 913 - protein, 6 aa, Homo sapiens
RTGPLG

SEQ ID NO: 914 - protein, 6 aa, Homo sapiens
APGERG

SEQ ID NO: 915 - protein, 6 aa, Homo sapiens
TPAPPG

SEQ ID NO: 916 - protein, 22 aa, Homo sapiens
SVPKEISPDTTLLDLQNNDISE

SEQ ID NO: 917 - protein, 23 aa, Homo sapiens
KSVPKEISPDTTLLDLQNNDISE

SEQ ID NO: 918 - protein, 23 aa, Homo sapiens
NSGFEPGAFDGLKLNYLRISEAK

SEQ ID NO: 919 - protein, 24 aa, Homo sapiens
LKSVPKEISPDTTLLDLQNNDISE

SEQ ID NO: 920 - protein, 18 aa, Homo sapiens
LRISEAKLTGIPKDLPET

SEQ ID NO: 921 - protein, 26 aa, Homo sapiens
LTGIPKDLPETLNELHLDHNKIQAIE

SEQ ID NO: 922 - protein, 20 aa, Homo sapiens
RISEAKLTGIPKDLPETLNE

SEQ ID NO: 923 - protein, 12 aa, Homo sapiens
AIELEDLLRYSK

SEQ ID NO: 924 - protein, 10 aa, Homo sapiens
AIELEDLLRY

SEQ ID NO: 925 - protein, 17 aa, Homo sapiens
EAKLTGIPKDLPETLNE

SEQ ID NO: 926 - protein, 24 aa, Homo sapiens
LKAVPKEISPDTTLLDLQNNDISE

SEQ ID NO: 927 - protein, 16 aa, Homo sapiens
LLDLQNNDISELRKDD

SEQ ID NO: 928 - protein, 10 aa, Homo sapiens
IELEDLLRYS

SEQ ID NO: 929 - protein, 13 aa, Homo sapiens
NSGFEPGAFDGLK

SEQ ID NO: 930 - protein, 11 aa, Homo sapiens
IVIELGTNPLK

SEQ ID NO: 931 - protein, 14 aa, Homo sapiens
DEASGIGPEVPDDR

SEQ ID NO: 932 - protein, 15 aa, Homo sapiens
LHLDGNKISRVDAAS

SEQ ID NO: 933 - protein, 16 aa, Homo sapiens
VNNKISKVSPGAFTPL

SEQ ID NO: 934 - protein, 24 aa, Homo sapiens
LILVNNKISKVSPGAFTPLVKLER

SEQ ID NO: 935 - protein, 15 aa, Homo sapiens
SNPVQYWEIQPSTFR

SEQ ID NO: 936 - protein, 11 aa, Homo sapiens
KITEIKDGDFK

SEQ ID NO: 937 - protein, 15 aa, Homo sapiens
GLPPSLTELHLDGNK

SEQ ID NO: 938 - protein, 10 aa, Homo sapiens
LLASDAGLYR

SEQ ID NO: 939 - protein, 12 aa, Homo sapiens
LATVGELQAAWR

SEQ ID NO: 940 - protein, 13 aa, Homo sapiens
ETTVLVAQNGNIK

SEQ ID NO: 941 - protein, 11 aa, Homo sapiens
SLEDLQLTHNK

SEQ ID NO: 942 - protein, 11 aa, Homo sapiens
LKEDAVSAAFK

SEQ ID NO: 943 - protein, 14 aa, Homo sapiens
SIEYSPQLEDAGSR

SEQ ID NO: 944 - protein, 10 aa, Homo sapiens
LEGDTLIIPR

SEQ ID NO: 945 - protein, 14 aa, Homo sapiens
VSEAVVEKLEPEYR

SEQ ID NO: 946 - protein, 16 aa, Homo sapiens
SSGIENGAFQGMKKLS

SEQ ID NO: 947 - protein, 15 aa, Homo sapiens
EVSEAVVEKLEPEYR

SEQ ID NO: 948 - protein, 17 aa, Homo sapiens
SIEYSPQLEDASAKEFR

SEQ ID NO: 949 - protein, 6 aa, Homo sapiens
SVPKEI

SEQ ID NO: 950 - protein, 6 aa, Homo sapiens
GLKLNY

SEQ ID NO: 951 - protein, 6 aa, Homo sapiens
RISEAK

SEQ ID NO: 952 - protein, 6 aa, Homo sapiens
NSGFEP

SEQ ID NO: 953 - protein, 6 aa, Homo sapiens
LKSVPK

SEQ ID NO: 954 - protein, 6 aa, Homo sapiens
AIELED

SEQ ID NO: 955 - protein, 6 aa, Homo sapiens
QCSDLG

SEQ ID NO: 956 - protein, 6 aa, Homo sapiens
EAKLTG

SEQ ID NO: 957 - protein, 6 aa, Homo sapiens
IELEDL

SEQ ID NO: 958 - protein, 6 aa, Homo sapiens
LRISEA

SEQ ID NO: 959 - protein, 6 aa, Homo sapiens
LTGIPK

SEQ ID NO: 960 - protein, 6 aa, Homo sapiens
LKAVPK

SEQ ID NO: 961 - protein, 6 aa, Homo sapiens
LLDLQN

SEQ ID NO: 962 - protein, 6 aa, Homo sapiens
IVIELG

SEQ ID NO: 963 - protein, 6 aa, Homo sapiens
DEASGI

SEQ ID NO: 964 - protein, 6 aa, Homo sapiens
VNNKIS

SEQ ID NO: 965 - protein, 6 aa, Homo sapiens
NGLNQM

SEQ ID NO: 966 - protein, 6 aa, Homo sapiens
LHLDGN

SEQ ID NO: 967 - protein, 6 aa, Homo sapiens
LILVNN

SEQ ID NO: 968 - protein, 6 aa, Homo sapiens
SSGIEN

SEQ ID NO: 969 - protein, 6 aa, Homo sapiens
KITEIK

SEQ ID NO: 970 - protein, 6 aa, Homo sapiens
GLPPSL

SEQ ID NO: 971 - protein, 6 aa, Homo sapiens
SNPVQY

SEQ ID NO: 972 - protein, 6 aa, Homo sapiens
LLASDA

SEQ ID NO: 973 - protein, 6 aa, Homo sapiens
LATVGE

SEQ ID NO: 974 - protein, 6 aa, Homo sapiens
ETTVLV

SEQ ID NO: 975 - protein, 6 aa, Homo sapiens
ENQDAR

SEQ ID NO: 976 - protein, 6 aa, Homo sapiens
NGFDQC

SEQ ID NO: 977 - protein, 6 aa, Homo sapiens
SLTVVK

SEQ ID NO: 978 - protein, 6 aa, Homo sapiens
SLEDLQ

SEQ ID NO: 979 - protein, 6 aa, Homo sapiens
LKEDAV

SEQ ID NO: 980 - protein, 6 aa, Homo sapiens
HLQHNR

SEQ ID NO: 981 - protein, 6 aa, Homo sapiens
SIEYSP

SEQ ID NO: 982 - protein, 6 aa, Homo sapiens
LVNFTR

SEQ ID NO: 983 - protein, 6 aa, Homo sapiens
VSEAVV

SEQ ID NO: 984 - protein, 6 aa, Homo sapiens
EVSEAV

SEQ ID NO: 985 - protein, 6 aa, Homo sapiens
LQHNRL

SEQ ID NO: 986 - protein, 6 aa, Homo sapiens
NNDISE

SEQ ID NO: 987 - protein, 6 aa, Homo sapiens
YWEVQP

SEQ ID NO: 988 - protein, 6 aa, Homo sapiens
EDLLRY

SEQ ID NO: 989 - protein, 6 aa, Homo sapiens
KIQAIE

SEQ ID NO: 990 - protein, 6 aa, Homo sapiens
PETLNE

SEQ ID NO: 991 - protein, 6 aa, Homo sapiens
LRKDDF

SEQ ID NO: 992 - protein, 6 aa, Homo sapiens
LLRYSK

SEQ ID NO: 993 - protein, 6 aa, Homo sapiens
ELRKDD

SEQ ID NO: 994 - protein, 6 aa, Homo sapiens
KDLPET

SEQ ID NO: 995 - protein, 6 aa, Homo sapiens
DLLRYS

SEQ ID NO: 996 - protein, 6 aa, Homo sapiens
AFDGLK

SEQ ID NO: 997 - protein, 6 aa, Homo sapiens
LNELHL

SEQ ID NO: 998 - protein, 6 aa, Homo sapiens
GTNPLK

SEQ ID NO: 999 - protein, 6 aa, Homo sapiens
EVPDDR

SEQ ID NO: 1000 - protein, 6 aa, Homo sapiens
GAFTPL

SEQ ID NO: 1001 - protein, 6 aa, Homo sapiens
RVDAAS

SEQ ID NO: 1002 - protein, 6 aa, Homo sapiens
LVKLER

SEQ ID NO: 1003 - protein, 6 aa, Homo sapiens
GMKKLS

SEQ ID NO: 1004 - protein, 6 aa, Homo sapiens
KDGDFK

SEQ ID NO: 1005 - protein, 6 aa, Homo sapiens
HLDGNK

SEQ ID NO: 1006 - protein, 6 aa, Homo sapiens
QPSTFR

SEQ ID NO: 1007 - protein, 6 aa, Homo sapiens
AFQGMK

SEQ ID NO: 1008 - protein, 6 aa, Homo sapiens
CDVMYG

SEQ ID NO: 1009 - protein, 6 aa, Homo sapiens
QNGINK

SEQ ID NO: 1010 - protein, 6 aa, Homo sapiens
IGQDYK

SEQ ID NO: 1011 - protein, 6 aa, Homo sapiens
QLTHNK

SEQ ID NO: 1012 - protein, 6 aa, Homo sapiens
VSAAFK

SEQ ID NO: 1013 - protein, 6 aa, Homo sapiens
GLKSLE

SEQ ID NO: 1014 - protein, 6 aa, Homo sapiens
EDAGSR

SEQ ID NO: 1015 - protein, 6 aa, Homo sapiens
EFREVS

SEQ ID NO: 1016 - protein, 6 aa, Homo sapiens
VAQQDS

SEQ ID NO: 1017 - protein, 6 aa, Homo sapiens
SAKEFR

SEQ ID NO: 1018 - protein, 6 aa, Homo sapiens
LEPEYR

SEQ ID NO: 1019 - protein, 16 aa, Homo sapiens
KESDTSYVSLKAPLTK

SEQ ID NO: 1020 - protein, 16 aa, Homo sapiens
GGNFEGSQSLVGDIGN

SEQ ID NO: 1021 - protein, 16 aa, Homo sapiens
ALKYEVQGEVFTKPQL

SEQ ID NO: 1022 - protein, 14 aa, Homo sapiens
GIVEFWVDGKPRVR

SEQ ID NO: 1023 - protein, 10 aa, Homo sapiens
RKAFVFPKES

SEQ ID NO: 1024 - protein, 16 aa, Homo sapiens
KYEVQGEVFTKPQLWP

SEQ ID NO: 1025 - protein, 13 aa, Homo sapiens
DSFGGNFEGSQSL

SEQ ID NO: 1026 - protein, 12 aa, Homo sapiens
DFVLSPDEINTI

SEQ ID NO: 1027 - protein, 13 aa, Homo sapiens
SLKKGYTVGAEAS

SEQ ID NO: 1028 - protein, 12 aa, Homo sapiens
AFGQTDMSRKAF

SEQ ID NO: 1029 - protein, 14 aa, Homo sapiens
SLKKGYTVGAEASI

SEQ ID NO: 1030 - protein, 11 aa, Homo sapiens
GEVFTKPQLWP

SEQ ID NO: 1031 - protein, 15 aa, Homo sapiens
SIILGQEQDSFGGNF

SEQ ID NO: 1032 - protein, 14 aa, Homo sapiens
KYEVQGEVFTKPQL

SEQ ID NO: 1033 - protein, 6 aa, Homo sapiens
AFVFPK

SEQ ID NO: 1034 - protein, 8 aa, Homo sapiens
FGQTDMSR

SEQ ID NO: 1035 - protein, 9 aa, Homo sapiens
FGQTDMSRK

SEQ ID NO: 1036 - protein, 10 aa, Homo sapiens
FGQTDMSRKA

SEQ ID NO: 1037 - protein, 11 aa, Homo sapiens
FGQTDMSRKAF

SEQ ID NO: 1038 - protein, 16 aa, Homo sapiens
FGQTDMSRKAFVFPKE

SEQ ID NO: 1039 - protein, 20 aa, Homo sapiens
FGQTDMSRKAFVFPKESDTS

SEQ ID NO: 1040 - protein, 22 aa, Homo sapiens
FGQTDMSRKAFVFPKESDTSYV

SEQ ID NO: 1041 - protein, 23 aa, Homo sapiens
FGQTDMSRKAFVFPKESDTSYVS

SEQ ID NO: 1042 - protein, 19 aa, Homo sapiens
TDMSRKAFVFPKESDTSYV

SEQ ID NO: 1043 - protein, 15 aa, Homo sapiens
MSRKAFVFPKESDTS

SEQ ID NO: 1044 - protein, 16 aa, Homo sapiens
SRKAFVFPKESDTSYV

SEQ ID NO: 1045 - protein, 9 aa, Homo sapiens
RKAFVFPKE

SEQ ID NO: 1046 - protein, 15 aa, Homo sapiens
RKAFVFPKESDTSYV

SEQ ID NO: 1047 - protein, 16 aa, Homo sapiens
RKAFVFPKESDTSYVS

SEQ ID NO: 1048 - protein, 8 aa, Homo sapiens
KAFVFPKE

SEQ ID NO: 1049 - protein, 10 aa, Homo sapiens
KAFVFPKESD

SEQ ID NO: 1050 - protein, 11 aa, Homo sapiens
KAFVFPKESDT

SEQ ID NO: 1051 - protein, 12 aa, Homo sapiens
KAFVFPKESDTS

SEQ ID NO: 1052 - protein, 14 aa, Homo sapiens
KAFVFPKESDTSYV

SEQ ID NO: 1053 - protein, 15 aa, Homo sapiens
KAFVFPKESDTSYVS

SEQ ID NO: 1054 - protein, 7 aa, Homo sapiens
AFVFPKE

SEQ ID NO: 1055 - protein, 10 aa, Homo sapiens
AFVFPKESDT

SEQ ID NO: 1056 - protein, 13 aa, Homo sapiens
AFVFPKESDTSYV

SEQ ID NO: 1057 - protein, 14 aa, Homo sapiens
AFVFPKESDTSYVS

SEQ ID NO: 1058 - protein, 15 aa, Homo sapiens
AFVFPKESDTSYVSL

SEQ ID NO: 1059 - protein, 5 aa, Homo sapiens
FVFPK

SEQ ID NO: 1060 - protein, 6 aa, Homo sapiens
FVFPKE

SEQ ID NO: 1061 - protein, 8 aa, Homo sapiens
FVFPKESD

SEQ ID NO: 1062 - protein, 10 aa, Homo sapiens
FVFPKESDTS

SEQ ID NO: 1063 - protein, 11 aa, Homo sapiens
FVFPKESDTSY

SEQ ID NO: 1064 - protein, 12 aa, Homo sapiens
FVFPKESDTSYV

SEQ ID NO: 1065 - protein, 13 aa, Homo sapiens
FVFPKESDTSYVS

SEQ ID NO: 1066 - protein, 14 aa, Homo sapiens
FVFPKESDTSYVSL

SEQ ID NO: 1067 - protein, 9 aa, Homo sapiens
VFPKESDTS

SEQ ID NO: 1068 - protein, 11 aa, Homo sapiens
VFPKESDTSYV

SEQ ID NO: 1069 - protein, 12 aa, Homo sapiens
VFPKESDTSYVS

SEQ ID NO: 1070 - protein, 13 aa, Homo sapiens
VFPKESDTSYVSL

SEQ ID NO: 1071 - protein, 11 aa, Homo sapiens
FPKESDTSYVS

SEQ ID NO: 1072 - protein, 17 aa, Homo sapiens
KESDTSYVSLKAPLTKP

SEQ ID NO: 1073 - protein, 15 aa, Homo sapiens
SDTSYVSLKAPLTKP

SEQ ID NO: 1074 - protein, 9 aa, Homo sapiens
SLKAPLTKP

SEQ ID NO: 1075 - protein, 11 aa, Homo sapiens
SLKAPLTKPLK

SEQ ID NO: 1076 - protein, 10 aa, Homo sapiens
LKAPLTKPLK

SEQ ID NO: 1077 - protein, 12 aa, Homo sapiens
FYTELSSTRGYS

SEQ ID NO: 1078 - protein, 8 aa, Homo sapiens
LSSTRGYS

SEQ ID NO: 1079 - protein, 7 aa, Homo sapiens
SSTRGYS

SEQ ID NO: 1080 - protein, 6 aa, Homo sapiens
STRGYS

SEQ ID NO: 1081 - protein, 9 aa, Homo sapiens
IFSYATKRQ

SEQ ID NO: 1082 - protein, 15 aa, Homo sapiens
IFSYATKRQDNEILI

SEQ ID NO: 1083 - protein, 13 aa, Homo sapiens
SYATKRQDNEILI

SEQ ID NO: 1084 - protein, 11 aa, Homo sapiens
YATKRQDNEIL

SEQ ID NO: 1085 - protein, 12 aa, Homo sapiens
YATKRQDNEILI

SEQ ID NO: 1086 - protein, 13 aa, Homo sapiens
YATKRQDNEILIF

SEQ ID NO: 1087 - protein, 10 aa, Homo sapiens
TKRQDNEILI

SEQ ID NO: 1088 - protein, 11 aa, Homo sapiens
TKRQDNEILIF

SEQ ID NO: 1089 - protein, 16 aa, Homo sapiens
TKRQDNEILIFWSKDI

SEQ ID NO: 1090 - protein, 9 aa, Homo sapiens
KRQDNEILI

SEQ ID NO: 1091 - protein, 10 aa, Homo sapiens
KRQDNEILIF

SEQ ID NO: 1092 - protein, 8 aa, Homo sapiens
WSKDIGYS

SEQ ID NO: 1093 - protein, 7 aa, Homo sapiens
SKDIGYS

SEQ ID NO: 1094 - protein, 12 aa, Homo sapiens
IVEFWVDGKPRV

SEQ ID NO: 1095 - protein, 9 aa, Homo sapiens
EFWVDGKPR

SEQ ID NO: 1096 - protein, 8 aa, Homo sapiens
WVDGKPRV

SEQ ID NO: 1097 - protein, 7 aa, Homo sapiens
VDGKPRV

SEQ ID NO: 1098 - protein, 11 aa, Homo sapiens
SLKKGYTVGAE

SEQ ID NO: 1099 - protein, 12 aa, Homo sapiens
SLKKGYTVGAEA

SEQ ID NO: 1100 - protein, 13 aa, Homo sapiens
SLKKGYTVGAEAS

SEQ ID NO: 1101 - protein, 7 aa, Homo sapiens
LKKGYTV

SEQ ID NO: 1102 - protein, 8 aa, Homo sapiens
LKKGYTVG

SEQ ID NO: 1103 - protein, 9 aa, Homo sapiens
LKKGYTVGA

SEQ ID NO: 1104 - protein, 10 aa, Homo sapiens
LKKGYTVGAE

SEQ ID NO: 1105 - protein, 11 aa, Homo sapiens
LKKGYTVGAEA

SEQ ID NO: 1106 - protein, 12 aa, Homo sapiens
LKKGYTVGAEAS

SEQ ID NO: 1107 - protein, 13 aa, Homo sapiens
LKKGYTVGAEASI

SEQ ID NO: 1108 - protein, 14 aa, Homo sapiens
SIILGQEQDSFGGN

SEQ ID NO: 1109 - protein, 19 aa, Homo sapiens
SIILGQEQDSFGGNFEGSQ

SEQ ID NO: 1110 - protein, 20 aa, Homo sapiens
SIILGQEQDSFGGNFEGSQS

SEQ ID NO: 1111 - protein, 17 aa, Homo sapiens
IILGQEQDSFGGNFEGS

SEQ ID NO: 1112 - protein, 19 aa, Homo sapiens
IILGQEQDSFGGNFEGSQS

SEQ ID NO: 1113 - protein, 12 aa, Homo sapiens
ILGQEQDSFGGN

SEQ ID NO: 1114 - protein, 17 aa, Homo sapiens
ILGQEQDSFGGNFEGSQ

SEQ ID NO: 1115 - protein, 18 aa, Homo sapiens
ILGQEQDSFGGNFEGSQS

SEQ ID NO: 1116 - protein, 16 aa, Homo sapiens
LGQEQDSFGGNFEGSQ

SEQ ID NO: 1117 - protein, 17 aa, Homo sapiens
LGQEQDSFGGNFEGSQS

SEQ ID NO: 1118 - protein, 16 aa, Homo sapiens
GQEQDSFGGNFEGSQS

SEQ ID NO: 1119 - protein, 11 aa, Homo sapiens
SFGGNFEGSQS

SEQ ID NO: 1120 - protein, 11 aa, Homo sapiens
QSLVGDIGNVN

SEQ ID NO: 1121 - protein, 14 aa, Homo sapiens
INTIYLGGPFSPNV

SEQ ID NO: 1122 - protein, 16 aa, Homo sapiens
INTIYLGGPFSPNVLN

SEQ ID NO: 1123 - protein, 13 aa, Homo sapiens
IYLGGPFSPNVLN

SEQ ID NO: 1124 - protein, 12 aa, Homo sapiens
YLGGPFSPNVLN

SEQ ID NO: 1125 - protein, 8 aa, Homo sapiens
LGGPFSPN

SEQ ID NO: 1126 - protein, 26 aa, Homo sapiens
SPNVLNWRALKYEVQGEVFTKPQLWP

SEQ ID NO: 1127 - protein, 5 aa, Homo sapiens
LNWRA

SEQ ID NO: 1128 - protein, 6 aa, Homo sapiens
LNWRAL

SEQ ID NO: 1129 - protein, 7 aa, Homo sapiens
LNWRALK

SEQ ID NO: 1130 - protein, 7 aa, Homo sapiens
WRALKYE

SEQ ID NO: 1131 - protein, 8 aa, Homo sapiens
WRALKYEV

SEQ ID NO: 1132 - protein, 11 aa, Homo sapiens
WRALKYEVQGE

SEQ ID NO: 1133 - protein, 6 aa, Homo sapiens
ALKYEV

SEQ ID NO: 1134 - protein, 6 aa, Homo sapiens
LKYEVQ

SEQ ID NO: 1135 - protein, 7 aa, Homo sapiens
LKYEVQG

SEQ ID NO: 1136 - protein, 8 aa, Homo sapiens
LKYEVQGE

SEQ ID NO: 1137 - protein, 13 aa, Homo sapiens
LKYEVQGEVFTKP

SEQ ID NO: 1138 - protein, 14 aa, Homo sapiens
LKYEVQGEVFTKPQ

SEQ ID NO: 1139 - protein, 17 aa, Homo sapiens
LKYEVQGEVFTKPQLWP

SEQ ID NO: 1140 - protein, 7 aa, Homo sapiens
KYEVQGE

SEQ ID NO: 1141 - protein, 13 aa, Homo sapiens
KYEVQGEVFTKPQ

SEQ ID NO: 1142 - protein, 16 aa, Homo sapiens
KYEVQGEVFTKPQLWP

SEQ ID NO: 1143 - protein, 11 aa, Homo sapiens
YEVQGEVFTKP

SEQ ID NO: 1144 - protein, 12 aa, Homo sapiens
YEVQGEVFTKPQ

SEQ ID NO: 1145 - protein, 15 aa, Homo sapiens
YEVQGEVFTKPQLWP

SEQ ID NO: 1146 - protein, 10 aa, Homo sapiens
VQGEVFTKPQ

SEQ ID NO: 1147 - protein, 13 aa, Homo sapiens
VQGEVFTKPQLWP

SEQ ID NO: 1148 - protein, 9 aa, Homo sapiens
QGEVFTKPQ

SEQ ID NO: 1149 - protein, 7 aa, Homo sapiens
GEVFTKP

SEQ ID NO: 1150 - protein, 8 aa, Homo sapiens
GEVFTKPQ

SEQ ID NO: 1151 - protein, 7 aa, Homo sapiens
EVFTKPQ

SEQ ID NO: 1152 - protein, 10 aa, Homo sapiens
EVFTKPQLWP

SEQ ID NO: 1153 - protein, 6 aa, Homo sapiens
VFTKPQ

SEQ ID NO: 1154 - protein, 5 aa, Homo sapiens
FTKPQ

SEQ ID NO: 1155 - protein, 8 aa, Homo sapiens
FTKPQLWP

SEQ ID NO: 1156 - protein, 7 aa, Homo sapiens
TKPQLWP

SEQ ID NO: 1157 - protein, 6 aa, Homo sapiens
KPQLWP

SEQ ID NO: 1158 - protein, 9 aa, Homo sapiens
MSRKAFVFP

SEQ ID NO: 1159 - protein, 11 aa, Homo sapiens
MSRKAFVFPKE

SEQ ID NO: 1160 - protein, 13 aa, Homo sapiens
MSRKAFVFPKESD

SEQ ID NO: 1161 - protein, 18 aa, Homo sapiens
MSRKAFVFPKESDTSYVS

SEQ ID NO: 1162 - protein, 8 aa, Homo sapiens
SRKAFVFP

SEQ ID NO: 1163 - protein, 12 aa, Homo sapiens
SRKAFVFPKESD

SEQ ID NO: 1164 - protein, 14 aa, Homo sapiens
SRKAFVFPKESDTS

SEQ ID NO: 1165 - protein, 7 aa, Homo sapiens
RKAFVFP

SEQ ID NO: 1166 - protein, 11 aa, Homo sapiens
RKAFVFPKESD

SEQ ID NO: 1167 - protein, 6 aa, Homo sapiens
KAFVFP

SEQ ID NO: 1168 - protein, 11 aa, Homo sapiens
AFVFPKESDTS

SEQ ID NO: 1169 - protein, 7 aa, Homo sapiens
VFPKESD

SEQ ID NO: 1170 - protein, 7 aa, Homo sapiens
KESDTSY

SEQ ID NO: 1171 - protein, 9 aa, Homo sapiens
KESDTSYVS

SEQ ID NO: 1172 - protein, 6 aa, Homo sapiens
VSLKAP

SEQ ID NO: 1173 - protein, 6 aa, Homo sapiens
LKAPLT

SEQ ID NO: 1174 - protein, 8 aa, Homo sapiens
LKAPLTKP

SEQ ID NO: 1175 - protein, 11 aa, Homo sapiens
YTELSSTRGYS

SEQ ID NO: 1176 - protein, 9 aa, Homo sapiens
YATKRQDNE

SEQ ID NO: 1177 - protein, 10 aa, Homo sapiens
YATKRQDNEI

SEQ ID NO: 1178 - protein, 9 aa, Homo sapiens
TKRQDNEIL

SEQ ID NO: 1179 - protein, 8 aa, Homo sapiens
KRQDNEIL

SEQ ID NO: 1180 - protein, 8 aa, Homo sapiens
ILIFWSKD

SEQ ID NO: 1181 - protein, 6 aa, Homo sapiens
IFWSKD

SEQ ID NO: 1182 - protein, 9 aa, Homo sapiens
WVDGKPRVR

SEQ ID NO: 1183 - protein, 16 aa, Homo sapiens
VRKSLKKGYTVGAEAS

SEQ ID NO: 1184 - protein, 7 aa, Homo sapiens
SLKKGYT

SEQ ID NO: 1185 - protein, 9 aa, Homo sapiens
SLKKGYTVG

SEQ ID NO: 1186 - protein, 10 aa, Homo sapiens
SLKKGYTVGA

SEQ ID NO: 1187 - protein, 14 aa, Homo sapiens
SLKKGYTVGAEASI

SEQ ID NO: 1188 - protein, 11 aa, Homo sapiens
KKGYTVGAEAS

SEQ ID NO: 1189 - protein, 10 aa, Homo sapiens
KGYTVGAEAS

SEQ ID NO: 1190 - protein, 11 aa, Homo sapiens
KGYTVGAEASI

SEQ ID NO: 1191 - protein, 8 aa, Homo sapiens
IILGQEQD

SEQ ID NO: 1192 - protein, 13 aa, Homo sapiens
IILGQEQDSFGGN

SEQ ID NO: 1193 - protein, 12 aa, Homo sapiens
LVGDIGNVNMWD

SEQ ID NO: 1194 - protein, 10 aa, Homo sapiens
IYLGGPFSPN

SEQ ID NO: 1195 - protein, 13 aa, Homo sapiens
IYLGGPFSPNVLN

SEQ ID NO: 1196 - protein, 11 aa, Homo sapiens
LGGPFSPNVLN

SEQ ID NO: 1197 - protein, 10 aa, Homo sapiens
EVQGEVFTKP

SEQ ID NO: 1198 - protein, 14 aa, Homo sapiens
EVQGEVFTKPQLWP

SEQ ID NO: 1199 - protein, 9 aa, Homo sapiens
VQGEVFTKP

SEQ ID NO: 1200 - protein, 11 aa, Homo sapiens
GEVFTKPQLWP

SEQ ID NO: 1201 - protein, 6 aa, Homo sapiens
EVFTKP

SEQ ID NO: 1202 - protein, 7 aa, Homo sapiens
VFTKPQL

SEQ ID NO: 1203 - protein, 9 aa, Homo sapiens
VFTKPQLWP

SEQ ID NO: 1204 - protein, 7 aa, Homo sapiens
KAFVFPK

SEQ ID NO: 1205 - protein, 6 aa, Homo sapiens
VRKSLK

SEQ ID NO: 1206 - protein, 17 aa, Homo sapiens
MSRKAFVFPKESDTSYV

SEQ ID NO: 1207 - protein, 17 aa, Homo sapiens
SRKAFVFPKESDTSYVS

SEQ ID NO: 1208 - protein, 16 aa, Homo sapiens
KAFVFPKESDTSYVSL

SEQ ID NO: 1209 - protein, 17 aa, Homo sapiens
KAFVFPKESDTSYVSLK

SEQ ID NO: 1210 - protein, 18 aa, Homo sapiens
AFVFPKESDTSYVSLKAP

SEQ ID NO: 1211 - protein, 15 aa, Homo sapiens
FVFPKESDTSYVSLK

SEQ ID NO: 1212 - protein, 14 aa, Homo sapiens
VFPKESDTSYVSLK

SEQ ID NO: 1213 - protein, 13 aa, Homo sapiens
KESDTSYVSLKAP

SEQ ID NO: 1214 - protein, 12 aa, Homo sapiens
TKRQDNEILIFW

SEQ ID NO: 1215 - protein, 15 aa, Homo sapiens
IVEFWVDGKPRVRKS

SEQ ID NO: 1216 - protein, 14 aa, Homo sapiens
LKKGYTVGAEASII

SEQ ID NO: 1217 - protein, 15 aa, Homo sapiens
QEQDSFGGNFEGSQS

SEQ ID NO: 1218 - protein, 10 aa, Homo sapiens
FVLSPDEINT

SEQ ID NO: 1219 - protein, 15 aa, Homo sapiens
SKDIGYSFTVGGSEI

SEQ ID NO: 1220 - protein, 12 aa, Homo sapiens
FGQTDMSRKAFV

SEQ ID NO: 1221 - protein, 10 aa, Homo sapiens
FPKESDTSYV

SEQ ID NO: 1222 - protein, 6 aa, Homo sapiens
SLKAPL

SEQ ID NO: 1223 - protein, 12 aa, Homo sapiens
SLKAPLTKPLKA

SEQ ID NO: 1224 - protein, 9 aa, Homo sapiens
RGYSIFSYA

SEQ ID NO: 1225 - protein, 14 aa, Homo sapiens
FSYATKRQDNEILI

SEQ ID NO: 1226 - protein, 11 aa, Homo sapiens
ATKRQDNEILI

SEQ ID NO: 1227 - protein, 9 aa, Homo sapiens
FWSKDIGYS

SEQ ID NO: 1228 - protein, 11 aa, Homo sapiens
FWSKDIGYSFT

SEQ ID NO: 1229 - protein, 12 aa, Homo sapiens
FWSKDIGYSFTV

SEQ ID NO: 1230 - protein, 11 aa, Homo sapiens
WSKDIGYSFTV

SEQ ID NO: 1231 - protein, 13 aa, Homo sapiens
KSLKKGYTVGAEA

SEQ ID NO: 1232 - protein, 10 aa, Homo sapiens
KKGYTVGAEA

SEQ ID NO: 1233 - protein, 11 aa, Homo sapiens
GAEASIILGQE

SEQ ID NO: 1234 - protein, 13 aa, Homo sapiens
GAEASIILGQEQD

SEQ ID NO: 1235 - protein, 9 aa, Homo sapiens
SIILGQEQD

SEQ ID NO: 1236 - protein, 18 aa, Homo sapiens
IILGQEQDSFGGNFEGSQ

SEQ ID NO: 1237 - protein, 16 aa, Homo sapiens
ILGQEQDSFGGNFEGS

SEQ ID NO: 1238 - protein, 11 aa, Homo sapiens
LGQEQDSFGGN

SEQ ID NO: 1239 - protein, 15 aa, Homo sapiens
LGQEQDSFGGNFEGS

SEQ ID NO: 1240 - protein, 18 aa, Homo sapiens
LGQEQDSFGGNFEGSQSL

SEQ ID NO: 1241 - protein, 19 aa, Homo sapiens
LGQEQDSFGGNFEGSQSLV

SEQ ID NO: 1242 - protein, 13 aa, Homo sapiens
QDSFGGNFEGSQS

SEQ ID NO: 1243 - protein, 10 aa, Homo sapiens
SFGGNFEGSQ

SEQ ID NO: 1244 - protein, 13 aa, Homo sapiens
SFGGNFEGSQSLV

SEQ ID NO: 1245 - protein, 11 aa, Homo sapiens
LVGDIGNVNMW

SEQ ID NO: 1246 - protein, 13 aa, Homo sapiens
INTIYLGGPFSPN

SEQ ID NO: 1247 - protein, 11 aa, Homo sapiens
TIYLGGPFSPN

SEQ ID NO: 1248 - protein, 13 aa, Homo sapiens
YLGGPFSPNVSEQ

SEQ ID NO: 1249 - protein, 6 aa, Homo sapiens
VLNWRA

SEQ ID NO: 1250 - protein, 7 aa, Homo sapiens
VLNWRAL

SEQ ID NO: 1251 - protein, 8 aa, Homo sapiens
VLNWRALK

SEQ ID NO: 1252 - protein, 10 aa, Homo sapiens
LNWRALKYEV

SEQ ID NO: 1253 - protein, 5 aa, Homo sapiens
NWRAL

SEQ ID NO: 1254 - protein, 7 aa, Homo sapiens
NWRALKY

SEQ ID NO: 1255 - protein, 9 aa, Homo sapiens
NWRALKYEV

SEQ ID NO: 1256 - protein, 10 aa, Homo sapiens
NWRALKYEVQ

SEQ ID NO: 1257 - protein, 9 aa, Homo sapiens
WRALKYEVQ

SEQ ID NO: 1258 - protein, 7 aa, Homo sapiens
RALKYEV

SEQ ID NO: 1259 - protein, 8 aa, Homo sapiens
RALKYEVQ

SEQ ID NO: 1260 - protein, 10 aa, Homo sapiens
RALKYEVQGE

SEQ ID NO: 1261 - protein, 15 aa, Homo sapiens
ALKYEVQGEVFTKPQ

SEQ ID NO: 1262 - protein, 11 aa, Homo sapiens
EVQGEVFTKPQ

SEQ ID NO: 1263 - protein, 10 aa, Homo sapiens
QGEVFTKPQL

SEQ ID NO: 1264 - protein, 12 aa, Homo sapiens
QGEVFTKPQLWP

SEQ ID NO: 1265 - protein, 10 aa, Homo sapiens
ESDTSYVSLK

SEQ ID NO: 1266 - protein, 14 aa, Homo sapiens
QEQDSFGGNFEGSQ

SEQ ID NO: 1267 - protein, 18 aa, Homo sapiens
QEQDSFGGNFEGSQSLVG

SEQ ID NO: 1268 - protein, 11 aa, Homo sapiens
GNFEGSQSLVG

SEQ ID NO: 1269 - protein, 9 aa, Homo sapiens
YEVQGEVFT

SEQ ID NO: 1270 - protein, 7 aa, Homo sapiens
EINTIYL

SEQ ID NO: 1271 - protein, 5 aa, Homo sapiens
KYEVQ

SEQ ID NO: 1272 - protein, 14 aa, Homo sapiens
ESDTSYVSLKAPLT

SEQ ID NO: 1273 - protein, 9 aa, Homo sapiens
SDTSYVSLK

SEQ ID NO: 1274 - protein, 8 aa, Homo sapiens
DTSYVSLK

SEQ ID NO: 1275 - protein, 8 aa, Homo sapiens
IFWSKDIG

SEQ ID NO: 1276 - protein, 8 aa, Homo sapiens
KGYTVGAE

SEQ ID NO: 1277 - protein, 15 aa, Homo sapiens
AEASIILGQEQDSFG

SEQ ID NO: 1278 - protein, 9 aa, Homo sapiens
LGQEQDSFG

SEQ ID NO: 1279 - protein, 13 aa, Homo sapiens
LGQEQDSFGGNFE

SEQ ID NO: 1280 - protein, 8 aa, Homo sapiens
GQEQDSFG

SEQ ID NO: 1281 - protein, 12 aa, Homo sapiens
GQEQDSFGGNFE

SEQ ID NO: 1282 - protein, 15 aa, Homo sapiens
GQEQDSFGGNFEGSQ

SEQ ID NO: 1283 - protein, 9 aa, Homo sapiens
QEQDSFGGN

SEQ ID NO: 1284 - protein, 11 aa, Homo sapiens
QEQDSFGGNFE

SEQ ID NO: 1285 - protein, 12 aa, Homo sapiens
QEQDSFGGNFEG

SEQ ID NO: 1286 - protein, 13 aa, Homo sapiens
QEQDSFGGNFEGS

SEQ ID NO: 1287 - protein, 10 aa, Homo sapiens
GNFEGSQSLV

SEQ ID NO: 1288 - protein, 14 aa, Homo sapiens
GNFEGSQSLVGDIG

SEQ ID NO: 1289 - protein, 10 aa, Homo sapiens
GSQSLVGDIG

SEQ ID NO: 1290 - protein, 13 aa, Homo sapiens
GSQSLVGDIGNVN

SEQ ID NO: 1291 - protein, 9 aa, Homo sapiens
VLSPDEINT

SEQ ID NO: 1292 - protein, 9 aa, Homo sapiens
GPFSPNVLN

SEQ ID NO: 1293 - protein, 8 aa, Homo sapiens
SPNVLNWR

SEQ ID NO: 1294 - protein, 6 aa, Homo sapiens
KYEVQG

SEQ ID NO: 1295 - protein, 11 aa, Homo sapiens
TSWESASGIVE

SEQ ID NO: 1296 - protein, 6 aa, Homo sapiens
KGYTVG

SEQ ID NO: 1297 - protein, 17 aa, Homo sapiens
QEQDSFGGNFEGSQSLV

SEQ ID NO: 1298 - protein, 14 aa, Homo sapiens
SFGGNFEGSQSLVG

SEQ ID NO: 1299 - protein, 10 aa, Homo sapiens
SPDEINTIYL

SEQ ID NO: 1300 - protein, 11 aa, Homo sapiens
SPDEINTIYLG

SEQ ID NO: 1301 - protein, 10 aa, Homo sapiens
GGPFSPNVLN

SEQ ID NO: 1302 - protein, 5 aa, Homo sapiens
ALKYE

SEQ ID NO: 1303 - protein, 7 aa, Homo sapiens
ALKYEVQ

SEQ ID NO: 1304 - protein, 8 aa, Homo sapiens
YEVQGEVF

SEQ ID NO: 1305 - protein, 6 aa, Homo sapiens
SFGGNF

SEQ ID NO: 1306 - protein, 6 aa, Homo sapiens
FGQTDM

SEQ ID NO: 1307 - protein, 6 aa, Homo sapiens
TDMSRK

SEQ ID NO: 1308 - protein, 6 aa, Homo sapiens
MSRKAF

SEQ ID NO: 1309 - protein, 6 aa, Homo sapiens
SRKAFV

SEQ ID NO: 1310 - protein, 6 aa, Homo sapiens
VFPKES

SEQ ID NO: 1311 - protein, 6 aa, Homo sapiens
FPKESD

SEQ ID NO: 1312 - protein, 6 aa, Homo sapiens
KESDTS

SEQ ID NO: 1313 - protein, 6 aa, Homo sapiens
LSSTRG

SEQ ID NO: 1314 - protein, 6 aa, Homo sapiens
SSTRGY

SEQ ID NO: 1315 - protein, 6 aa, Homo sapiens
KRQDNE

SEQ ID NO: 1316 - protein, 6 aa, Homo sapiens
WSKDIG

SEQ ID NO: 1317 - protein, 6 aa, Homo sapiens
SKDIGY

SEQ ID NO: 1318 - protein, 6 aa, Homo sapiens
SIILGQ

SEQ ID NO: 1319 - protein, 6 aa, Homo sapiens
IILGQE

SEQ ID NO: 1320 - protein, 6 aa, Homo sapiens
ILGQEQ

SEQ ID NO: 1321 - protein, 6 aa, Homo sapiens
IYLGGP

SEQ ID NO: 1322 - protein, 6 aa, Homo sapiens
YLGGPF

SEQ ID NO: 1323 - protein, 6 aa, Homo sapiens
LGGPFS

SEQ ID NO: 1324 - protein, 6 aa, Homo sapiens
VQGEVF

SEQ ID NO: 1325 - protein, 6 aa, Homo sapiens
YTELSS

SEQ ID NO: 1326 - protein, 6 aa, Homo sapiens
ILIFWS

SEQ ID NO: 1327 - protein, 6 aa, Homo sapiens
LVGDIG

SEQ ID NO: 1328 - protein, 6 aa, Homo sapiens
QEQDSF

SEQ ID NO: 1329 - protein, 6 aa, Homo sapiens
RGYSIF

SEQ ID NO: 1330 - protein, 6 aa, Homo sapiens
GAEASI

SEQ ID NO: 1331 - protein, 6 aa, Homo sapiens
QDSFGG

SEQ ID NO: 1332 - protein, 6 aa, Homo sapiens
TIYLGG

SEQ ID NO: 1333 - protein, 6 aa, Homo sapiens
EINTIY

SEQ ID NO: 1334 - protein, 6 aa, Homo sapiens
DTSYVS

SEQ ID NO: 1335 - protein, 6 aa, Homo sapiens
AEASII

SEQ ID NO: 1336 - protein, 6 aa, Homo sapiens
TSWESA

SEQ ID NO: 1337 - protein, 6 aa, Homo sapiens
SPDEIN

SEQ ID NO: 1338 - protein, 6 aa, Homo sapiens
GGPFSP

SEQ ID NO: 1339 - protein, 6 aa, Homo sapiens
YEVQGE

SEQ ID NO: 1340 - protein, 6 aa, Homo sapiens
FVLSPD

SEQ ID NO: 1341 - protein, 6 aa, Homo sapiens
LKKGYT

SEQ ID NO: 1342 - protein, 6 aa, Homo sapiens
RKAFVF

SEQ ID NO: 1343 - protein, 6 aa, Homo sapiens
IVEFWV

SEQ ID NO: 1344 - protein, 6 aa, Homo sapiens
ESDTSY

SEQ ID NO: 1345 - protein, 6 aa, Homo sapiens
TKPQLW

SEQ ID NO: 1346 - protein, 6 aa, Homo sapiens
EVQGEV

SEQ ID NO: 1347 - protein, 6 aa, Homo sapiens
SDTSYV

SEQ ID NO: 1348 - protein, 6 aa, Homo sapiens
IFSYAT

SEQ ID NO: 1349 - protein, 6 aa, Homo sapiens
SYATKR

SEQ ID NO: 1350 - protein, 6 aa, Homo sapiens
YATKRQ

SEQ ID NO: 1351 - protein, 6 aa, Homo sapiens
EFWVDG

SEQ ID NO: 1352 - protein, 6 aa, Homo sapiens
WVDGKP

SEQ ID NO: 1353 - protein, 6 aa, Homo sapiens
VDGKPR

SEQ ID NO: 1354 - protein, 6 aa, Homo sapiens
LGQEQD

SEQ ID NO: 1355 - protein, 6 aa, Homo sapiens
GQEQDS

SEQ ID NO: 1356 - protein, 6 aa, Homo sapiens
QSLVGD

SEQ ID NO: 1357 - protein, 6 aa, Homo sapiens
SPNVLN

SEQ ID NO: 1358 - protein, 6 aa, Homo sapiens
QGEVFT

SEQ ID NO: 1359 - protein, 6 aa, Homo sapiens
GEVFTK

SEQ ID NO: 1360 - protein, 6 aa, Homo sapiens
KKGYTV

SEQ ID NO: 1361 - protein, 6 aa, Homo sapiens
FSYATK

SEQ ID NO: 1362 - protein, 6 aa, Homo sapiens
ATKRQD

SEQ ID NO: 1363 - protein, 6 aa, Homo sapiens
FWSKDI

SEQ ID NO: 1364 - protein, 6 aa, Homo sapiens
NWRALK

SEQ ID NO: 1365 - protein, 6 aa, Homo sapiens
GSQSLV

SEQ ID NO: 1366 - protein, 6 aa, Homo sapiens
DFVLSP

SEQ ID NO: 1367 - protein, 6 aa, Homo sapiens
VLSPDE

SEQ ID NO: 1368 - protein, 6 aa, Homo sapiens
TKRQDN

SEQ ID NO: 1369 - protein, 6 aa, Homo sapiens
GNFEGS

SEQ ID NO: 1370 - protein, 6 aa, Homo sapiens
SLKKGY

SEQ ID NO: 1371 - protein, 6 aa, Homo sapiens
KSLKKG

SEQ ID NO: 1372 - protein, 6 aa, Homo sapiens
INTIYL

SEQ ID NO: 1373 - protein, 6 aa, Homo sapiens
RALKYE

SEQ ID NO: 1374 - protein, 6 aa, Homo sapiens
FYTELS

SEQ ID NO: 1375 - protein, 6 aa, Homo sapiens
WRALKY

SEQ ID NO: 1376 - protein, 6 aa, Homo sapiens
GPFSPN

SEQ ID NO: 1377 - protein, 6 aa, Homo sapiens
PDEINT

SEQ ID NO: 1378 - protein, 6 aa, Homo sapiens
DSFGGN

SEQ ID NO: 1379 - protein, 6 aa, Homo sapiens
LTKPLK

SEQ ID NO: 1380 - protein, 6 aa, Homo sapiens
KDIGYS

SEQ ID NO: 1381 - protein, 6 aa, Homo sapiens
DGKPRV

SEQ ID NO: 1382 - protein, 6 aa, Homo sapiens
NFEGSQ

SEQ ID NO: 1383 - protein, 6 aa, Homo sapiens
NVNMWD

SEQ ID NO: 1384 - protein, 6 aa, Homo sapiens
PRVRKS

SEQ ID NO: 1385 - protein, 6 aa, Homo sapiens
TVGSEI

SEQ ID NO: 1386 - protein, 6 aa, Homo sapiens
GYSFTV

SEQ ID NO: 1387 - protein, 6 aa, Homo sapiens
EGSQSL

SEQ ID NO: 1388 - protein, 6 aa, Homo sapiens
EQDSFG

SEQ ID NO: 1389 - protein, 6 aa, Homo sapiens
NVLNWR

SEQ ID NO: 1390 - protein, 6 aa, Homo sapiens
ASGIVE

SEQ ID NO: 1391 - protein, 6 aa, Homo sapiens
NTIYLG

SEQ ID NO: 1392 - protein, 6 aa, Homo sapiens
VGAEAS

SEQ ID NO: 1393 - protein, 6 aa, Homo sapiens
APLTKP

SEQ ID NO: 1394 - protein, 6 aa, Homo sapiens
QTDMSR

SEQ ID NO: 1395 - protein, 6 aa, Homo sapiens
PKESDT

SEQ ID NO: 1396 - protein, 6 aa, Homo sapiens
TSYVSL

SEQ ID NO: 1397 - protein, 6 aa, Homo sapiens
DNEILI

SEQ ID NO: 1398 - protein, 6 aa, Homo sapiens
QDNEIL

SEQ ID NO: 1399 - protein, 6 aa, Homo sapiens
NEILIF

SEQ ID NO: 1400 - protein, 6 aa, Homo sapiens
YTVGAE

SEQ ID NO: 1401 - protein, 6 aa, Homo sapiens
TVGAEA

SEQ ID NO: 1402 - protein, 6 aa, Homo sapiens
PFSPNV

SEQ ID NO: 1403 - protein, 6 aa, Homo sapiens
FEGSQS

SEQ ID NO: 1404 - protein, 6 aa, Homo sapiens
DIGNVN

SEQ ID NO: 1405 - protein, 6 aa, Homo sapiens
RQDNEI

SEQ ID NO: 1406 - protein, 6 aa, Homo sapiens
FTKPQL

SEQ ID NO: 1407 - protein, 6 aa, Homo sapiens
SYVSLK

SEQ ID NO: 1408 - protein, 6 aa, Homo sapiens
TKPLKA

SEQ ID NO: 1409 - protein, 6 aa, Homo sapiens
SIFSYA

SEQ ID NO: 1410 - protein, 6 aa, Homo sapiens
GNVNMW

SEQ ID NO: 1411 - protein, 6 aa, Homo sapiens
SQSLVG

SEQ ID NO: 1412 - protein, 6 aa, Homo sapiens
FGGNFE

SEQ ID NO: 1413 - protein, 6 aa, Homo sapiens
GGNFEG

SEQ ID NO: 1414 - protein, 6 aa, Homo sapiens
GKPRVR

SEQ ID NO: 1415 - protein, 6 aa, Homo sapiens
DMSRKA

SEQ ID NO: 1416 - protein, 6 aa, Homo sapiens
EILIFW

SEQ ID NO: 1417 - protein, 6 aa, Homo sapiens
IGYSFT

SEQ ID NO: 1418 - protein, 12 aa, Homo sapiens
GVPGAIPGGVPG

SEQ ID NO: 1419 - protein, 18 aa, Homo sapiens
AIPGGVPGGVFYPGAGLG

SEQ ID NO: 1420 - protein, 19 aa, Homo sapiens
AIPGGVPGGVFYPGAGLGA

SEQ ID NO: 1421 - protein, 15 aa, Homo sapiens
GVPGGVFYPGAGLGA

SEQ ID NO: 1422 - protein, 17 aa, Homo sapiens
GVPGGVFYPGAGLGALG

SEQ ID NO: 1423 - protein, 17 aa, Homo sapiens
VPGGVFYPGAGLGALGG

SEQ ID NO: 1424 - protein, 21 aa, Homo sapiens
GVFYPGAGLGALGGGALGPGG

SEQ ID NO: 1425 - protein, 9 aa, Homo sapiens
VFYPGAGLG

SEQ ID NO: 1426 - protein, 10 aa, Homo sapiens
VFYPGAGLGA

SEQ ID NO: 1427 - protein, 11 aa, Homo sapiens
VFYPGAGLGAL

SEQ ID NO: 1428 - protein, 12 aa, Homo sapiens
VFYPGAGLGALG

SEQ ID NO: 1429 - protein, 13 aa, Homo sapiens
VFYPGAGLGALGG

SEQ ID NO: 1430 - protein, 14 aa, Homo sapiens
VFYPGAGLGALGGG

SEQ ID NO: 1431 - protein, 16 aa, Homo sapiens
VFYPGAGLGALGGGAL

SEQ ID NO: 1432 - protein, 17 aa, Homo sapiens
VFYPGAGLGALGGGALG

SEQ ID NO: 1433 - protein, 19 aa, Homo sapiens
VFYPGAGLGALGGGALGPG

SEQ ID NO: 1434 - protein, 20 aa, Homo sapiens
VFYPGAGLGALGGGALGPGG

SEQ ID NO: 1435 - protein, 29 aa, Homo sapiens
VFYPGAGLGALGGGALGPGGKPLKPVPGG

SEQ ID NO: 1436 - protein, 22 aa, Homo sapiens
LGALGGGALGPGGKPLKPVPGG

SEQ ID NO: 1437 - protein, 20 aa, Homo sapiens
ALGGGALGPGGKPLKPVPGG

SEQ ID NO: 1438 - protein, 18 aa, Homo sapiens
LGGGALGPGGKPLKPVPG

SEQ ID NO: 1439 - protein, 19 aa, Homo sapiens
LGGGALGPGGKPLKPVPGG

SEQ ID NO: 1440 - protein, 17 aa, Homo sapiens
GGALGPGGKPLKPVPGG

SEQ ID NO: 1441 - protein, 14 aa, Homo sapiens
LGPGGKPLKPVPGG

SEQ ID NO: 1442 - protein, 13 aa, Homo sapiens
GPGGKPLKPVPGG

SEQ ID NO: 1443 - protein, 12 aa, Homo sapiens
PGGKPLKPVPGG

SEQ ID NO: 1444 - protein, 10 aa, Homo sapiens
GKPLKPVPGG

SEQ ID NO: 1445 - protein, 8 aa, Homo sapiens
PLKPVPGG

SEQ ID NO: 1446 - protein, 7 aa, Homo sapiens
LKPVPGG

SEQ ID NO: 1447 - protein, 15 aa, Homo sapiens
GLAGAGLGAGLGAFP

SEQ ID NO: 1448 - protein, 16 aa, Homo sapiens
GLAGAGLGAGLGAFPA

SEQ ID NO: 1449 - protein, 11 aa, Homo sapiens
LAGAGLGAGLG

SEQ ID NO: 1450 - protein, 14 aa, Homo sapiens
LAGAGLGAGLGAFP

SEQ ID NO: 1451 - protein, 15 aa, Homo sapiens
LAGAGLGAGLGAFPA

SEQ ID NO: 1452 - protein, 17 aa, Homo sapiens
LAGAGLGAGLGAFPAVT

SEQ ID NO: 1453 - protein, 20 aa, Homo sapiens
LAGAGLGAGLGAFPAVTFPG

SEQ ID NO: 1454 - protein, 21 aa, Homo sapiens
LAGAGLGAGLGAFPAVTFPGA

SEQ ID NO: 1455 - protein, 26 aa, Homo sapiens
LAGAGLGAGLGAFPAVTFPGALVPGG

SEQ ID NO: 1456 - protein, 28 aa, Homo sapiens
LAGAGLGAGLGAFPAVTFPGALVPGGVA

SEQ ID NO: 1457 - protein, 33 aa, Homo sapiens
LAGAGLGAGLGAFPAVTFPGALVPGGVADAAAA

SEQ ID NO: 1458 - protein, 25 aa, Homo sapiens
AGAGLGAGLGAFPAVTFPGALVPGG

SEQ ID NO: 1459 - protein, 13 aa, Homo sapiens
GAGLGAGLGAFPA

SEQ ID NO: 1460 - protein, 19 aa, Homo sapiens
GAGLGAGLGAFPAVTFPGA

SEQ ID NO: 1461 - protein, 12 aa, Homo sapiens
AGLGAGLGAFPA

SEQ ID NO: 1462 - protein, 11 aa, Homo sapiens
GLGAGLGAFPA

SEQ ID NO: 1463 - protein, 10 aa, Homo sapiens
LGAGLGAFPA

SEQ ID NO: 1464 - protein, 16 aa, Homo sapiens
LGAGLGAFPAVTFPGA

SEQ ID NO: 1465 - protein, 21 aa, Homo sapiens
LGAGLGAFPAVTFPGALVPGG

SEQ ID NO: 1466 - protein, 28 aa, Homo sapiens
LGAGLGAFPAVTFPGALVPGGVADAAAA

SEQ ID NO: 1467 - protein, 13 aa, Homo sapiens
AGLGAFPAVTFPG

SEQ ID NO: 1468 - protein, 12 aa, Homo sapiens
LGAFPAVTFPGA

SEQ ID NO: 1469 - protein, 19 aa, Homo sapiens
LGAFPAVTFPGALVPGGVA

SEQ ID NO: 1470 - protein, 24 aa, Homo sapiens
LGAFPAVTFPGALVPGGVADAAAA

SEQ ID NO: 1471 - protein, 15 aa, Homo sapiens
AFPAVTFPGALVPGG

SEQ ID NO: 1472 - protein, 12 aa, Homo sapiens
AVTFPGALVPGG

SEQ ID NO: 1473 - protein, 19 aa, Homo sapiens
AVTFPGALVPGGVADAAAA

SEQ ID NO: 1474 - protein, 11 aa, Homo sapiens
VTFPGALVPGG

SEQ ID NO: 1475 - protein, 18 aa, Homo sapiens
VTFPGALVPGGVADAAAA

SEQ ID NO: 1476 - protein, 12 aa, Homo sapiens
LVPGGVADAAAA

SEQ ID NO: 1477 - protein, 14 aa, Homo sapiens
LVPGGVADAAAAYK

SEQ ID NO: 1478 - protein, 9 aa, Homo sapiens
VADAAAAYK

SEQ ID NO: 1479 - protein, 7 aa, Homo sapiens
KAAKAGA

SEQ ID NO: 1480 - protein, 14 aa, Homo sapiens
LGVSAGAVVPQPGA

SEQ ID NO: 1481 - protein, 19 aa, Homo sapiens
VPGVGLPGVYPGGVLPGAR

SEQ ID NO: 1482 - protein, 18 aa, Homo sapiens
PGVGLPGVYPGGVLPGAR

SEQ ID NO: 1483 - protein, 15 aa, Homo sapiens
GLPGVYPGGVLPGAR

SEQ ID NO: 1484 - protein, 13 aa, Homo sapiens
PGVYPGGVLPGAR

SEQ ID NO: 1485 - protein, 7 aa, Homo sapiens
ARFPGVG

SEQ ID NO: 1486 - protein, 11 aa, Homo sapiens
ARFPGVGVLPG

SEQ ID NO: 1487 - protein, 16 aa, Homo sapiens
RFPGVGVLPGVPTGAG

SEQ ID NO: 1488 - protein, 13 aa, Homo sapiens
FPGVGVLPGVPTG

SEQ ID NO: 1489 - protein, 14 aa, Homo sapiens
FPGVGVLPGVPTGA

SEQ ID NO: 1490 - protein, 16 aa, Homo sapiens
FPGVGVLPGVPTGAGV

SEQ ID NO: 1491 - protein, 19 aa, Homo sapiens
FPGVGVLPGVPTGAGVKPK

SEQ ID NO: 1492 - protein, 7 aa, Homo sapiens
KPKAPGV

SEQ ID NO: 1493 - protein, 6 aa, Homo sapiens
PKAPGV

SEQ ID NO: 1494 - protein, 13 aa, Homo sapiens
GAFAGIPGVGPFG

SEQ ID NO: 1495 - protein, 16 aa, Homo sapiens
VGPFGGPQPGVPLGYP

SEQ ID NO: 1496 - protein, 11 aa, Homo sapiens
GPQPGVPLGYP

SEQ ID NO: 1497 - protein, 10 aa, Homo sapiens
PQPGVPLGYP

SEQ ID NO: 1498 - protein, 8 aa, Homo sapiens
PGVPLGYP

SEQ ID NO: 1499 - protein, 8 aa, Homo sapiens
GYPIKAPK

SEQ ID NO: 1500 - protein, 7 aa, Homo sapiens
PKLPGGY

SEQ ID NO: 1501 - protein, 13 aa, Homo sapiens
YTTGKLPYGYGPG

SEQ ID NO: 1502 - protein, 21 aa, Homo sapiens
YTTGKLPYGYGPGGVAGAAGK

SEQ ID NO: 1503 - protein, 10 aa, Homo sapiens
TTGKLPYGYG

SEQ ID NO: 1504 - protein, 20 aa, Homo sapiens
TTGKLPYGYGPGGVAGAAGK

SEQ ID NO: 1505 - protein, 16 aa, Homo sapiens
LPYGYGPGGVAGAAGK

SEQ ID NO: 1506 - protein, 13 aa, Homo sapiens
GYGPGGVAGAAGK

SEQ ID NO: 1507 - protein, 12 aa, Homo sapiens
YGPGGVAGAAGK

SEQ ID NO: 1508 - protein, 20 aa, Homo sapiens
AGYPTGTGVGPQAAAAAAAK

SEQ ID NO: 1509 - protein, 14 aa, Homo sapiens
TGVGPQAAAAAAAK

SEQ ID NO: 1510 - protein, 10 aa, Homo sapiens
PQAAAAAAAK

SEQ ID NO: 1511 - protein, 29 aa, Homo sapiens
FGAGAAGVLPGVGGAGVPGVPGAIPGIGG

SEQ ID NO: 1512 - protein, 38 aa, Homo sapiens
FGAGAAGVLPGVGGAGVPGVPGAIPGIGGIAGVGTPAA

SEQ ID NO: 1513 - protein, 16 aa, Homo sapiens
GVLPGVGGAGVPGVPG

SEQ ID NO: 1514 - protein, 22 aa, Homo sapiens
VLPGVGGAGVPGVPGAIPGIGG

SEQ ID NO: 1515 - protein, 30 aa, Homo sapiens
VLPGVGGAGVPGVPGAIPGIGGIAGVGTPA

SEQ ID NO: 1516 - protein, 31 aa, Homo sapiens
VLPGVGGAGVPGVPGAIPGIGGIAGVGTPAA

SEQ ID NO: 1517 - protein, 13 aa, Homo sapiens
GAGVPGVPGAIPG

SEQ ID NO: 1518 - protein, 14 aa, Homo sapiens
AGVPGVPGAIPGIG

SEQ ID NO: 1519 - protein, 14 aa, Homo sapiens
AGVPGVPGAIPGIG

SEQ ID NO: 1520 - protein, 15 aa, Homo sapiens
AGVPGVPGAIPGIGG

SEQ ID NO: 1521 - protein, 18 aa, Homo sapiens
AGVPGVPGAIPGIGGIAG

SEQ ID NO: 1522 - protein, 23 aa, Homo sapiens
AGVPGVPGAIPGIGGIAGVGTPA

SEQ ID NO: 1523 - protein, 14 aa, Homo sapiens
GVPGVPGAIPGIGG

SEQ ID NO: 1524 - protein, 16 aa, Homo sapiens
GVPGVPGAIPGIGGIA

SEQ ID NO: 1525 - protein, 19 aa, Homo sapiens
GVPGVPGAIPGIGGIAGVG

SEQ ID NO: 1526 - protein, 13 aa, Homo sapiens
VPGVPGAIPGIGG

SEQ ID NO: 1527 - protein, 19 aa, Homo sapiens
GVPGAIPGIGGIAGVGTPA

SEQ ID NO: 1528 - protein, 15 aa, Homo sapiens
VPGAIPGIGGIAGVG

SEQ ID NO: 1529 - protein, 18 aa, Homo sapiens
VPGAIPGIGGIAGVGTPA

SEQ ID NO: 1530 - protein, 20 aa, Homo sapiens
VPGAIPGIGGIAGVGTPAAA

SEQ ID NO: 1531 - protein, 28 aa, Homo sapiens
VPGAIPGIGGIAGVGTPAAAAAAAAAAK

SEQ ID NO: 1532 - protein, 12 aa, Homo sapiens
AIPGIGGIAGVG

SEQ ID NO: 1533 - protein, 15 aa, Homo sapiens
AIPGIGGIAGVGTPA

SEQ ID NO: 1534 - protein, 16 aa, Homo sapiens
AIPGIGGIAGVGTPAA

SEQ ID NO: 1535 - protein, 17 aa, Homo sapiens
AIPGIGGIAGVGTPAAA

SEQ ID NO: 1536 - protein, 20 aa, Homo sapiens
AIPGIGGIAGVGTPAAAAAA

SEQ ID NO: 1537 - protein, 25 aa, Homo sapiens
AIPGIGGIAGVGTPAAAAAAAAAAK

SEQ ID NO: 1538 - protein, 16 aa, Homo sapiens
IPGIGGIAGVGTPAAA

SEQ ID NO: 1539 - protein, 14 aa, Homo sapiens
IGGIAGVGTPAAAA

SEQ ID NO: 1540 - protein, 12 aa, Homo sapiens
GIAGVGTPAAAA

SEQ ID NO: 1541 - protein, 16 aa, Homo sapiens
GIAGVGTPAAAAAAAA

SEQ ID NO: 1542 - protein, 19 aa, Homo sapiens
GIAGVGTPAAAAAAAAAAK

SEQ ID NO: 1543 - protein, 15 aa, Homo sapiens
IAGVGTPAAAAAAAA

SEQ ID NO: 1544 - protein, 16 aa, Homo sapiens
IAGVGTPAAAAAAAAA

SEQ ID NO: 1545 - protein, 18 aa, Homo sapiens
IAGVGTPAAAAAAAAAAK

SEQ ID NO: 1546 - protein, 13 aa, Homo sapiens
TPAAAAAAAAAAK

SEQ ID NO: 1547 - protein, 12 aa, Homo sapiens
PAAAAAAAAAAK

SEQ ID NO: 1548 - protein, 11 aa, Homo sapiens
AAAAAAAAAAK

SEQ ID NO: 1549 - protein, 10 aa, Homo sapiens
AAAAAAAAAK

SEQ ID NO: 1550 - protein, 9 aa, Homo sapiens
AAAAAAAAK

SEQ ID NO: 1551 - protein, 10 aa, Homo sapiens
AAAAAAAAKA

SEQ ID NO: 1552 - protein, 8 aa, Homo sapiens
AAAAAAAK

SEQ ID NO: 1553 - protein, 18 aa, Homo sapiens
LVPGGPGFGPGVVGVPGA

SEQ ID NO: 1554 - protein, 13 aa, Homo sapiens
GPGFGPGVVGVPG

SEQ ID NO: 1555 - protein, 20 aa, Homo sapiens
GPGFGPGVVGVPGAGVPGVG

SEQ ID NO: 1556 - protein, 31 aa, Homo sapiens
GPGFGPGVVGVPGAGVPGVGVPGAGIPVVPG

SEQ ID NO: 1557 - protein, 12 aa, Homo sapiens
PGFGPGVVGVPG

SEQ ID NO: 1558 - protein, 13 aa, Homo sapiens
PGFGPGVVGVPGA

SEQ ID NO: 1559 - protein, 14 aa, Homo sapiens
PGFGPGVVGVPGAG

SEQ ID NO: 1560 - protein, 13 aa, Homo sapiens
PGVVGVPGAGVPG

SEQ ID NO: 1561 - protein, 18 aa, Homo sapiens
PGVVGVPGAGVPGVGVPG

SEQ ID NO: 1562 - protein, 27 aa, Homo sapiens
PGVVGVPGAGVPGVGVPGAGIPVVPGA

SEQ ID NO: 1563 - protein, 17 aa, Homo sapiens
VVGVPGAGVPGVGVPGA

SEQ ID NO: 1564 - protein, 39 aa, Homo sapiens
VGVPGAGVPGVGVPGAGIPVVPGAGIPGAAVPGVVSPEA

SEQ ID NO: 1565 - protein, 18 aa, Homo sapiens
AGVPGVGVPGAGIPVVPG

SEQ ID NO: 1566 - protein, 17 aa, Homo sapiens
GVPGVGVPGAGIPVVPG

SEQ ID NO: 1567 - protein, 18 aa, Homo sapiens
GVPGVGVPGAGIPVVPGA

SEQ ID NO: 1568 - protein, 16 aa, Homo sapiens
VPGVGVPGAGIPVVPG

SEQ ID NO: 1569 - protein, 13 aa, Homo sapiens
VGVPGAGIPVVPG

SEQ ID NO: 1570 - protein, 18 aa, Homo sapiens
VGVPGAGIPVVPGAGIPG

SEQ ID NO: 1571 - protein, 11 aa, Homo sapiens
VPGAGIPVVPG

SEQ ID NO: 1572 - protein, 13 aa, Homo sapiens
AGIPVVPGAGIPG

SEQ ID NO: 1573 - protein, 27 aa, Homo sapiens
AGIPVVPGAGIPGAAVPGVVSPEAAAK

SEQ ID NO: 1574 - protein, 12 aa, Homo sapiens
GIPVVPGAGIPG

SEQ ID NO: 1575 - protein, 17 aa, Homo sapiens
IPGAAVPGVVSPEAAAK

SEQ ID NO: 1576 - protein, 15 aa, Homo sapiens
GAAVPGVVSPEAAAK

SEQ ID NO: 1577 - protein, 13 aa, Homo sapiens
AVPGVVSPEAAAK

SEQ ID NO: 1578 - protein, 12 aa, Homo sapiens
VPGVVSPEAAAK

SEQ ID NO: 1579 - protein, 8 aa, Homo sapiens
YGARPGVG

SEQ ID NO: 1580 - protein, 10 aa, Homo sapiens
YGARPGVGVG

SEQ ID NO: 1581 - protein, 14 aa, Homo sapiens
YGARPGVGVGGIPT

SEQ ID NO: 1582 - protein, 15 aa, Homo sapiens
YGARPGVGVGGIPTY

SEQ ID NO: 1583 - protein, 16 aa, Homo sapiens
YGARPGVGVGGIPTYG

SEQ ID NO: 1584 - protein, 18 aa, Homo sapiens
YGARPGVGVGGIPTYGVG

SEQ ID NO: 1585 - protein, 19 aa, Homo sapiens
YGARPGVGVGGIPTYGVGA

SEQ ID NO: 1586 - protein, 20 aa, Homo sapiens
YGARPGVGVGGIPTYGVGAG

SEQ ID NO: 1587 - protein, 8 aa, Homo sapiens
GARPGVGV

SEQ ID NO: 1588 - protein, 10 aa, Homo sapiens
GARPGVGVGG

SEQ ID NO: 1589 - protein, 12 aa, Homo sapiens
GARPGVGVGGIP

SEQ ID NO: 1590 - protein, 14 aa, Homo sapiens
GARPGVGVGGIPTY

SEQ ID NO: 1591 - protein, 16 aa, Homo sapiens
GARPGVGVGGIPTYGV

SEQ ID NO: 1592 - protein, 17 aa, Homo sapiens
GARPGVGVGGIPTYGVG

SEQ ID NO: 1593 - protein, 21 aa, Homo sapiens
GARPGVGVGGIPTYGVGAGGF

SEQ ID NO: 1594 - protein, 24 aa, Homo sapiens
GARPGVGVGGIPTYGVGAGGFPGF

SEQ ID NO: 1595 - protein, 25 aa, Homo sapiens
GARPGVGVGGIPTYGVGAGGFPGFG

SEQ ID NO: 1596 - protein, 29 aa, Homo sapiens
GARPGVGVGGIPTYGVGAGGFPGFGVGVG

SEQ ID NO: 1597 - protein, 9 aa, Homo sapiens
ARPGVGVGG

SEQ ID NO: 1598 - protein, 11 aa, Homo sapiens
ARPGVGVGGIP

SEQ ID NO: 1599 - protein, 13 aa, Homo sapiens
ARPGVGVGGIPTY

SEQ ID NO: 1600 - protein, 17 aa, Homo sapiens
ARPGVGVGGIPTYGVGA

SEQ ID NO: 1601 - protein, 19 aa, Homo sapiens
ARPGVGVGGIPTYGVGAGG

SEQ ID NO: 1602 - protein, 22 aa, Homo sapiens
ARPGVGVGGIPTYGVGAGGFPG

SEQ ID NO: 1603 - protein, 23 aa, Homo sapiens
ARPGVGVGGIPTYGVGAGGFPGF

SEQ ID NO: 1604 - protein, 7 aa, Homo sapiens
RPGVGVG

SEQ ID NO: 1605 - protein, 8 aa, Homo sapiens
RPGVGVGG

SEQ ID NO: 1606 - protein, 11 aa, Homo sapiens
PGVGVGGIPTY

SEQ ID NO: 1607 - protein, 12 aa, Homo sapiens
PGVGVGGIPTYG

SEQ ID NO: 1608 - protein, 16 aa, Homo sapiens
PGVGVGGIPTYGVGAG

SEQ ID NO: 1609 - protein, 12 aa, Homo sapiens
VGGIPTYGVGAG

SEQ ID NO: 1610 - protein, 21 aa, Homo sapiens
GVGAGGFPGFGVGVGGIPGVA

SEQ ID NO: 1611 - protein, 14 aa, Homo sapiens
VGAGGFPGFGVGVG

SEQ ID NO: 1612 - protein, 33 aa, Homo sapiens
VGVGGIPGVAGVPSVGGVPGVGGVPGVGISPEA

SEQ ID NO: 1613 - protein, 18 aa, Homo sapiens
VAGVPSVGGVPGVGGVPG

SEQ ID NO: 1614 - protein, 25 aa, Homo sapiens
VAGVPSVGGVPGVGGVPGVGISPEA

SEQ ID NO: 1615 - protein, 20 aa, Homo sapiens
SVGGVPGVGGVPGVGISPEA

SEQ ID NO: 1616 - protein, 19 aa, Homo sapiens
VGGVPGVGGVPGVGISPEA

SEQ ID NO: 1617 - protein, 14 aa, Homo sapiens
GVPGVGGVPGVGIS

SEQ ID NO: 1618 - protein, 17 aa, Homo sapiens
GVPGVGGVPGVGISPEA

SEQ ID NO: 1619 - protein, 19 aa, Homo sapiens
GVPGVGGVPGVGISPEAQA

SEQ ID NO: 1620 - protein, 18 aa, Homo sapiens
GVPGVGISPEAQAAAAAK

SEQ ID NO: 1621 - protein, 11 aa, Homo sapiens
GVGTPAAAAAK

SEQ ID NO: 1622 - protein, 8 aa, Homo sapiens
TPAAAAAK

SEQ ID NO: 1623 - protein, 14 aa, Homo sapiens
FGLVPGVGVAPGVG

SEQ ID NO: 1624 - protein, 18 aa, Homo sapiens
FGLVPGVGVAPGVGVAPG

SEQ ID NO: 1625 - protein, 24 aa, Homo sapiens
FGLVPGVGVAPGVGVAPGVGVAPG

SEQ ID NO: 1626 - protein, 26 aa, Homo sapiens
FGLVPGVGVAPGVGVAPGVGVAPGVG

SEQ ID NO: 1627 - protein, 30 aa, Homo sapiens
FGLVPGVGVAPGVGVAPGVGVAPGVGLAPG

SEQ ID NO: 1628 - protein, 36 aa, Homo sapiens
FGLVPGVGVAPGVGVAPGVGVAPGVGLAPGVGVAPG

SEQ ID NO: 1629 - protein, 37 aa, Homo sapiens
FGLVPGVGVAPGVGVAPGVGVAPGVGLAPGVGVAPGV

SEQ ID NO: 1630 - protein, 42 aa, Homo sapiens
FGLVPGVGVAPGVGVAPGVGVAPGVGLAPGVGVAPGVGVAPG

SEQ ID NO: 1631 - protein, 11 aa, Homo sapiens
GLVPGVGVAPG

SEQ ID NO: 1632 - protein, 12 aa, Homo sapiens
GLVPGVGVAPGV

SEQ ID NO: 1633 - protein, 15 aa, Homo sapiens
GLVPGVGVAPGVGVA

SEQ ID NO: 1634 - protein, 16 aa, Homo sapiens
GLVPGVGVAPGVGVAP

SEQ ID NO: 1635 - protein, 17 aa, Homo sapiens
GLVPGVGVAPGVGVAPG

SEQ ID NO: 1636 - protein, 19 aa, Homo sapiens
GLVPGVGVAPGVGVAPGVG

SEQ ID NO: 1637 - protein, 23 aa, Homo sapiens
GLVPGVGVAPGVGVAPGVGVAPG

SEQ ID NO: 1638 - protein, 26 aa, Homo sapiens
GLVPGVGVAPGVGVAPGVGVAPGVGL

SEQ ID NO: 1639 - protein, 27 aa, Homo sapiens
GLVPGVGVAPGVGVAPGVGVAPGVGLA

SEQ ID NO: 1640 - protein, 29 aa, Homo sapiens
GLVPGVGVAPGVGVAPGVGVAPGVGLAPG

SEQ ID NO: 1641 - protein, 31 aa, Homo sapiens
GLVPGVGVAPGVGVAPGVGVAPGVGLAPGVG

SEQ ID NO: 1642 - protein, 33 aa, Homo sapiens
GLVPGVGVAPGVGVAPGVGVAPGVGLAPGVGVA

SEQ ID NO: 1643 - protein, 35 aa, Homo sapiens
GLVPGVGVAPGVGVAPGVGVAPGVGLAPGVGVAPG

SEQ ID NO: 1644 - protein, 12 aa, Homo sapiens
LVPGVGVAPGVG

SEQ ID NO: 1645 - protein, 16 aa, Homo sapiens
LVPGVGVAPGVGVAPG

SEQ ID NO: 1646 - protein, 18 aa, Homo sapiens
LVPGVGVAPGVGVAPGVG

SEQ ID NO: 1647 - protein, 24 aa, Homo sapiens
LVPGVGVAPGVGVAPGVGVAPGVG

SEQ ID NO: 1648 - protein, 36 aa, Homo sapiens
LVPGVGVAPGVGVAPGVGVAPGVGLAPGVGVAPGVG

SEQ ID NO: 1649 - protein, 14 aa, Homo sapiens
PGVGVAPGVGVAPG

SEQ ID NO: 1650 - protein, 15 aa, Homo sapiens
VGVAPGVGVAPGVGV

SEQ ID NO: 1651 - protein, 20 aa, Homo sapiens
VGVAPGVGVAPGVGVAPGVG

SEQ ID NO: 1652 - protein, 30 aa, Homo sapiens
VGVAPGVGVAPGVGVAPGVGLAPGVGVAPG

SEQ ID NO: 1653 - protein, 16 aa, Homo sapiens
VAPGVGVAPGVGVAPG

SEQ ID NO: 1654 - protein, 18 aa, Homo sapiens
VAPGVGVAPGVGVAPGVG

SEQ ID NO: 1655 - protein, 24 aa, Homo sapiens
VAPGVGVAPGVGVAPGVGLAPGVG

SEQ ID NO: 1656 - protein, 28 aa, Homo sapiens
VAPGVGVAPGVGVAPGVGLAPGVGVAPG

SEQ ID NO: 1657 - protein, 16 aa, Homo sapiens
VGVAPGVGVAPGVGLA

SEQ ID NO: 1658 - protein, 24 aa, Homo sapiens
VGVAPGVGVAPGVGLAPGVGVAPG

SEQ ID NO: 1659 - protein, 41 aa, Homo sapiens
VGVAPGVGVAPGVGLAPGVGVAPGVGVAPGVGVAPGIGPGG

SEQ ID NO: 1660 - protein, 24 aa, Homo sapiens
VAPGVGVAPGVGLAPGVGVAPGVG

SEQ ID NO: 1661 - protein, 26 aa, Homo sapiens
VAPGVGVAPGVGLAPGVGVAPGVGVA

SEQ ID NO: 1662 - protein, 28 aa, Homo sapiens
VAPGVGVAPGVGLAPGVGVAPGVGVAPG

SEQ ID NO: 1663 - protein, 37 aa, Homo sapiens
VAPGVGVAPGVGLAPGVGVAPGVGVAPGVGVAPGIGP

SEQ ID NO: 1664 - protein, 39 aa, Homo sapiens
VAPGVGVAPGVGLAPGVGVAPGVGVAPGVGVAPGIGPGG

SEQ ID NO: 1665 - protein, 14 aa, Homo sapiens
PGVGVAPGVGLAPG

SEQ ID NO: 1666 - protein, 19 aa, Homo sapiens
PGVGVAPGVGLAPGVGVAP

SEQ ID NO: 1667 - protein, 22 aa, Homo sapiens
PGVGVAPGVGLAPGVGVAPGVG

SEQ ID NO: 1668 - protein, 16 aa, Homo sapiens
VGVAPGVGLAPGVGVA

SEQ ID NO: 1669 - protein, 17 aa, Homo sapiens
VGVAPGVGLAPGVGVAP

SEQ ID NO: 1670 - protein, 24 aa, Homo sapiens
VGVAPGVGLAPGVGVAPGVGVAPG

SEQ ID NO: 1671 - protein, 26 aa, Homo sapiens
VGVAPGVGLAPGVGVAPGVGVAPGVG

SEQ ID NO: 1672 - protein, 30 aa, Homo sapiens
VGVAPGVGLAPGVGVAPGVGVAPGVGVAPG

SEQ ID NO: 1673 - protein, 35 aa, Homo sapiens
VGVAPGVGLAPGVGVAPGVGVAPGVGVAPGIGPGG

SEQ ID NO: 1674 - protein, 34 aa, Homo sapiens
GVAPGVGLAPGVGVAPGVGVAPGVGVAPGIGPGG

SEQ ID NO: 1675 - protein, 14 aa, Homo sapiens
VAPGVGLAPGVGVA

SEQ ID NO: 1676 - protein, 16 aa, Homo sapiens
VAPGVGLAPGVGVAPG

SEQ ID NO: 1677 - protein, 18 aa, Homo sapiens
VAPGVGLAPGVGVAPGVG

SEQ ID NO: 1678 - protein, 20 aa, Homo sapiens
VAPGVGLAPGVGVAPGVGVA

SEQ ID NO: 1679 - protein, 22 aa, Homo sapiens
VAPGVGLAPGVGVAPGVGVAPG

SEQ ID NO: 1680 - protein, 26 aa, Homo sapiens
VAPGVGLAPGVGVAPGVGVAPGVGVA

SEQ ID NO: 1681 - protein, 33 aa, Homo sapiens
VAPGVGLAPGVGVAPGVGVAPGVGVAPGIGPGG

SEQ ID NO: 1682 - protein, 14 aa, Homo sapiens
PGVGLAPGVGVAPG

SEQ ID NO: 1683 - protein, 19 aa, Homo sapiens
GVGLAPGVGVAPGVGVAPG

SEQ ID NO: 1684 - protein, 14 aa, Homo sapiens
VGLAPGVGVAPGVG

SEQ ID NO: 1685 - protein, 18 aa, Homo sapiens
VGLAPGVGVAPGVGVAPG

SEQ ID NO: 1686 - protein, 26 aa, Homo sapiens
VGLAPGVGVAPGVGVAPGVGVAPGIG

SEQ ID NO: 1687 - protein, 29 aa, Homo sapiens
VGLAPGVGVAPGVGVAPGVGVAPGIGPGG

SEQ ID NO: 1688 - protein, 28 aa, Homo sapiens
VGLAPGVGVAPGVGVAPGVGVAPGIGPG

SEQ ID NO: 1689 - protein, 33 aa, Homo sapiens
VGLAPGVGVAPGVGVAPGVGVAPGIGPGGVAAA

SEQ ID NO: 1690 - protein, 18 aa, Homo sapiens
LAPGVGVAPGVGVAPGVG

SEQ ID NO: 1691 - protein, 20 aa, Homo sapiens
LAPGVGVAPGVGVAPGVGVA

SEQ ID NO: 1692 - protein, 25 aa, Homo sapiens
LAPGVGVAPGVGVAPGVGVAPGIGP

SEQ ID NO: 1693 - protein, 27 aa, Homo sapiens
LAPGVGVAPGVGVAPGVGVAPGIGPGG

SEQ ID NO: 1694 - protein, 24 aa, Homo sapiens
GVGVAPGVGVAPGVGVAPGIGPGG

SEQ ID NO: 1695 - protein, 16 aa, Homo sapiens
VGVAPGVGVAPGVGVA

SEQ ID NO: 1696 - protein, 18 aa, Homo sapiens
VGVAPGVGVAPGVGVAPG

SEQ ID NO: 1697 - protein, 22 aa, Homo sapiens
VGVAPGVGVAPGVGVAPGIGPG

SEQ ID NO: 1698 - protein, 23 aa, Homo sapiens
VGVAPGVGVAPGVGVAPGIGPGG

SEQ ID NO: 1699 - protein, 27 aa, Homo sapiens
VGVAPGVGVAPGVGVAPGIGPGGVAAA

SEQ ID NO: 1700 - protein, 15 aa, Homo sapiens
VAPGVGVAPGVGVAP

SEQ ID NO: 1701 - protein, 18 aa, Homo sapiens
VAPGVGVAPGVGVAPGIG

SEQ ID NO: 1702 - protein, 21 aa, Homo sapiens
VAPGVGVAPGVGVAPGIGPGG

SEQ ID NO: 1703 - protein, 18 aa, Homo sapiens
PGVGVAPGVGVAPGIGPG

SEQ ID NO: 1704 - protein, 19 aa, Homo sapiens
PGVGVAPGVGVAPGIGPGG

SEQ ID NO: 1705 - protein, 17 aa, Homo sapiens
VGVAPGVGVAPGIGPGG

SEQ ID NO: 1706 - protein, 20 aa, Homo sapiens
VGVAPGVGVAPGIGPGGVAA

SEQ ID NO: 1707 - protein, 14 aa, Homo sapiens
VAPGVGVAPGIGPG

SEQ ID NO: 1708 - protein, 12 aa, Homo sapiens
PGVGVAPGIGPG

SEQ ID NO: 1709 - protein, 14 aa, Homo sapiens
VGVAPGIGPGGVAA

SEQ ID NO: 1710 - protein, 9 aa, Homo sapiens
PGGVAAAAK

SEQ ID NO: 1711 - protein, 7 aa, Homo sapiens
LRAAAGL

SEQ ID NO: 1712 - protein, 8 aa, Homo sapiens
LRAAAGLG

SEQ ID NO: 1713 - protein, 9 aa, Homo sapiens
LRAAAGLGA

SEQ ID NO: 1714 - protein, 15 aa, Homo sapiens
AAAGLGAGIPGLGVG

SEQ ID NO: 1715 - protein, 17 aa, Homo sapiens
AAAGLGAGIPGLGVGVG

SEQ ID NO: 1716 - protein, 11 aa, Homo sapiens
LGAGIPGLGVG

SEQ ID NO: 1717 - protein, 13 aa, Homo sapiens
LGAGIPGLGVGVG

SEQ ID NO: 1718 - protein, 20 aa, Homo sapiens
LGAGIPGLGVGVGVPGLGVG

SEQ ID NO: 1719 - protein, 16 aa, Homo sapiens
LGAGIPGLGVGVGVPG

SEQ ID NO: 1720 - protein, 21 aa, Homo sapiens
LGAGIPGLGVGVGVPGLGVGA

SEQ ID NO: 1721 - protein, 17 aa, Homo sapiens
LGAGIPGLGVGVGVPGL

SEQ ID NO: 1722 - protein, 18 aa, Homo sapiens
LGAGIPGLGVGVGVPGLG

SEQ ID NO: 1723 - protein, 25 aa, Homo sapiens
LGAGIPGLGVGVGVPGLGVGAGVPG

SEQ ID NO: 1724 - protein, 27 aa, Homo sapiens
LGAGIPGLGVGVGVPGLGVGAGVPGLG

SEQ ID NO: 1725 - protein, 29 aa, Homo sapiens
LGAGIPGLGVGVGVPGLGVGAGVPGLGVG

SEQ ID NO: 1726 - protein, 36 aa, Homo sapiens
LGAGIPGLGVGVGVPGLGVGAGVPGLGVGAGVPGFG

SEQ ID NO: 1727 - protein, 17 aa, Homo sapiens
GAGIPGLGVGVGVPGLG

SEQ ID NO: 1728 - protein, 14 aa, Homo sapiens
AGIPGLGVGVGVPG

SEQ ID NO: 1729 - protein, 18 aa, Homo sapiens
GIPGLGVGVGVPGLGVGA

SEQ ID NO: 1730 - protein, 14 aa, Homo sapiens
LGVGVGVPGLGVGA

SEQ ID NO: 1731 - protein, 14 aa, Homo sapiens
VGVPGLGVGAGVPG

SEQ ID NO: 1732 - protein, 15 aa, Homo sapiens
VGVPGLGVGAGVPGL

SEQ ID NO: 1733 - protein, 16 aa, Homo sapiens
VGVPGLGVGAGVPGLG

SEQ ID NO: 1734 - protein, 18 aa, Homo sapiens
VGVPGLGVGAGVPGLGVG

SEQ ID NO: 1735 - protein, 19 aa, Homo sapiens
VGVPGLGVGAGVPGLGVGA

SEQ ID NO: 1736 - protein, 18 aa, Homo sapiens
VGAGVPGLGVGAGVPGFG

SEQ ID NO: 1737 - protein, 8 aa, Homo sapiens
PGALAAAK

SEQ ID NO: 1738 - protein, 16 aa, Homo sapiens
AKYGAAVPGVLGGLGA

SEQ ID NO: 1739 - protein, 11 aa, Homo sapiens
YGAAVPGVLGG

SEQ ID NO: 1740 - protein, 13 aa, Homo sapiens
YGAAVPGVLGGLG

SEQ ID NO: 1741 - protein, 14 aa, Homo sapiens
YGAAVPGVLGGLGA

SEQ ID NO: 1742 - protein, 16 aa, Homo sapiens
YGAAVPGVLGGLGALG

SEQ ID NO: 1743 - protein, 23 aa, Homo sapiens
YGAAVPGVLGGLGALGGVGIPGG

SEQ ID NO: 1744 - protein, 31 aa, Homo sapiens
YGAAVPGVLGGLGALGGVGIPGGVVGAGPAA

SEQ ID NO: 1745 - protein, 12 aa, Homo sapiens
GAAVPGVLGGLG

SEQ ID NO: 1746 - protein, 22 aa, Homo sapiens
GAAVPGVLGGLGALGGVGIPGG

SEQ ID NO: 1747 - protein, 11 aa, Homo sapiens
AVPGVLGGLGA

SEQ ID NO: 1748 - protein, 20 aa, Homo sapiens
AVPGVLGGLGALGGVGIPGG

SEQ ID NO: 1749 - protein, 16 aa, Homo sapiens
VLGGLGALGGVGIPGG

SEQ ID NO: 1750 - protein, 21 aa, Homo sapiens
GGLGALGGVGIPGGVVGAGPA

SEQ ID NO: 1751 - protein, 23 aa, Homo sapiens
GGLGALGGVGIPGGVVGAGPAAA

SEQ ID NO: 1752 - protein, 12 aa, Homo sapiens
LGALGGVGIPGG

SEQ ID NO: 1753 - protein, 19 aa, Homo sapiens
LGALGGVGIPGGVVGAGPA

SEQ ID NO: 1754 - protein, 20 aa, Homo sapiens
LGALGGVGIPGGVVGAGPAA

SEQ ID NO: 1755 - protein, 21 aa, Homo sapiens
LGALGGVGIPGGVVGAGPAAA

SEQ ID NO: 1756 - protein, 22 aa, Homo sapiens
LGALGGVGIPGGVVGAGPAAAA

SEQ ID NO: 1757 - protein, 18 aa, Homo sapiens
ALGGVGIPGGVVGAGPAA

SEQ ID NO: 1758 - protein, 19 aa, Homo sapiens
ALGGVGIPGGVVGAGPAAA

SEQ ID NO: 1759 - protein, 13 aa, Homo sapiens
LGGVGIPGGVSEQ

SEQ ID NO: 1760 - protein, 16 aa, Homo sapiens
LGGVGIPGGVVGAGPA

SEQ ID NO: 1761 - protein, 18 aa, Homo sapiens
LGGVGIPGGVVGAGPAAA

SEQ ID NO: 1762 - protein, 20 aa, Homo sapiens
LGGVGIPGGVVGAGPAAAAA

SEQ ID NO: 1763 - protein, 23 aa, Homo sapiens
LGGVGIPGGVVGAGPAAAAAAAK

SEQ ID NO: 1764 - protein, 17 aa, Homo sapiens
GVGIPGGVVGAGPAAAA

SEQ ID NO: 1765 - protein, 21 aa, Homo sapiens
GVGIPGGVVGAGPAAAAAAAK

SEQ ID NO: 1766 - protein, 15 aa, Homo sapiens
VGIPGGVVGAGPAAA

SEQ ID NO: 1767 - protein, 20 aa, Homo sapiens
VGIPGGVVGAGPAAAAAAAK

SEQ ID NO: 1768 - protein, 14 aa, Homo sapiens
IPGGVVGAGPAAAA

SEQ ID NO: 1769 - protein, 14 aa, Homo sapiens
VVGAGPAAAAAAAK

SEQ ID NO: 1770 - protein, 13 aa, Homo sapiens
VGAGPAAAAAAAK

SEQ ID NO: 1771 - protein, 11 aa, Homo sapiens
AGPAAAAAAAK

SEQ ID NO: 1772 - protein, 10 aa, Homo sapiens
GPAAAAAAAK

SEQ ID NO: 1773 - protein, 9 aa, Homo sapiens
PAAAAAAAK

SEQ ID NO: 1774 - protein, 24 aa, Homo sapiens
FGLVGAAGLGGLGVGGLGVPGVGG

SEQ ID NO: 1775 - protein, 12 aa, Homo sapiens
GLVGAAGLGGLG

SEQ ID NO: 1776 - protein, 15 aa, Homo sapiens
GLVGAAGLGGLGVGG

SEQ ID NO: 1777 - protein, 22 aa, Homo sapiens
GLVGAAGLGGLGVGGLGVPGVG

SEQ ID NO: 1778 - protein, 23 aa, Homo sapiens
GLVGAAGLGGLGVGGLGVPGVGG

SEQ ID NO: 1779 - protein, 13 aa, Homo sapiens
LVGAAGLGGLGVG

SEQ ID NO: 1780 - protein, 13 aa, Homo sapiens
LVGAAGLGGLGVG

SEQ ID NO: 1781 - protein, 15 aa, Homo sapiens
LVGAAGLGGLGVGGL

SEQ ID NO: 1782 - protein, 24 aa, Homo sapiens
LVGAAGLGGLGVGGLGVPGVGGLG

SEQ ID NO: 1783 - protein, 31 aa, Homo sapiens
LVGAAGLGGLGVGGLGVPGVGGLGGIPPAAA

SEQ ID NO: 1784 - protein, 13 aa, Homo sapiens
VGAAGLGGLGVGG

SEQ ID NO: 1785 - protein, 13 aa, Homo sapiens
LGGLGVGGLGVPG

SEQ ID NO: 1786 - protein, 15 aa, Homo sapiens
LGGLGVGGLGVPGVG

SEQ ID NO: 1787 - protein, 17 aa, Homo sapiens
LGGLGVGGLGVPGVGGL

SEQ ID NO: 1788 - protein, 18 aa, Homo sapiens
LGGLGVGGLGVPGVGGLG

SEQ ID NO: 1789 - protein, 15 aa, Homo sapiens
LGVGGLGVPGVGGLG

SEQ ID NO: 1790 - protein, 20 aa, Homo sapiens
GLGVPGVGGLGGIPPAAAAK

SEQ ID NO: 1791 - protein, 11 aa, Homo sapiens
LGGIPPAAAAK

SEQ ID NO: 1792 - protein, 13 aa, Homo sapiens
LGGVLGGAGQFPL

SEQ ID NO: 1793 - protein, 19 aa, Homo sapiens
LGGVLGGAGQFPLGGVAAR

SEQ ID NO: 1794 - protein, 21 aa, Homo sapiens
LGGVLGGAGQFPLGGVAARPG

SEQ ID NO: 1795 - protein, 23 aa, Homo sapiens
LGGVLGGAGQFPLGGVAARPGFG

SEQ ID NO: 1796 - protein, 20 aa, Homo sapiens
GGVLGGAGQFPLGGVAARPG

SEQ ID NO: 1797 - protein, 13 aa, Homo sapiens
GAGQFPLGGVAAR

SEQ ID NO: 1798 - protein, 17 aa, Homo sapiens
GAGQFPLGGVAARPGFG

SEQ ID NO: 1799 - protein, 16 aa, Homo sapiens
AGQFPLGGVAARPGFG

SEQ ID NO: 1800 - protein, 11 aa, Homo sapiens
FPLGGVAARPG

SEQ ID NO: 1801 - protein, 8 aa, Homo sapiens
PLGGVAAR

SEQ ID NO: 1802 - protein, 10 aa, Homo sapiens
PLGGVAARPG

SEQ ID NO: 1803 - protein, 12 aa, Homo sapiens
PLGGVAARPGFG

SEQ ID NO: 1804 - protein, 13 aa, Homo sapiens
PLGGVAARPGFGL

SEQ ID NO: 1805 - protein, 19 aa, Homo sapiens
PLGGVAARPGFGLSPIFPG

SEQ ID NO: 1806 - protein, 7 aa, Homo sapiens
LGGVAAR

SEQ ID NO: 1807 - protein, 8 aa, Homo sapiens
LGGVAARP

SEQ ID NO: 1808 - protein, 9 aa, Homo sapiens
LGGVAARPG

SEQ ID NO: 1809 - protein, 10 aa, Homo sapiens
LGGVAARPGF

SEQ ID NO: 1810 - protein, 11 aa, Homo sapiens
LGGVAARPGFG

SEQ ID NO: 1811 - protein, 12 aa, Homo sapiens
LGGVAARPGFGL

SEQ ID NO: 1812 - protein, 14 aa, Homo sapiens
LGGVAARPGFGLSP

SEQ ID NO: 1813 - protein, 18 aa, Homo sapiens
LGGVAARPGFGLSPIFPG

SEQ ID NO: 1814 - protein, 19 aa, Homo sapiens
LGGVAARPGFGLSPIFPGG

SEQ ID NO: 1815 - protein, 20 aa, Homo sapiens
LGGVAARPGFGLSPIFPGGA

SEQ ID NO: 1816 - protein, 10 aa, Homo sapiens
GGVAARPGFG

SEQ ID NO: 1817 - protein, 11 aa, Homo sapiens
GGVAARPGFGL

SEQ ID NO: 1818 - protein, 19 aa, Homo sapiens
GGVAARPGFGLSPIFPGGA

SEQ ID NO: 1819 - protein, 14 aa, Homo sapiens
GVAARPGFGLSPIF

SEQ ID NO: 1820 - protein, 15 aa, Homo sapiens
GVAARPGFGLSPIFP

SEQ ID NO: 1821 - protein, 8 aa, Homo sapiens
VAARPGFG

SEQ ID NO: 1822 - protein, 14 aa, Homo sapiens
VAARPGFGLSPIFP

SEQ ID NO: 1823 - protein, 15 aa, Homo sapiens
VAARPGFGLSPIFPG

SEQ ID NO: 1824 - protein, 12 aa, Homo sapiens
RPGFGLSPIFPG

SEQ ID NO: 1825 - protein, 12 aa, Homo sapiens
PGFGLSPIFPGG

SEQ ID NO: 1826 - protein, 13 aa, Homo sapiens
PGFGLSPIFPGGA

SEQ ID NO: 1827 - protein, 19 aa, Homo sapiens
PGVGLPGVYPGGVLPGARF

SEQ ID NO: 1828 - protein, 18 aa, Homo sapiens
GVGLPGVYPGGVLPGARF

SEQ ID NO: 1829 - protein, 16 aa, Homo sapiens
GLPGVYPGGVLPGARF

SEQ ID NO: 1830 - protein, 14 aa, Homo sapiens
PGVYPGGVLPGARF

SEQ ID NO: 1831 - protein, 22 aa, Homo sapiens
KAGYPTGTGVGPQAAAAAAAKA

SEQ ID NO: 1832 - protein, 26 aa, Homo sapiens
GGPGFGPGVVGVPGAGVPGVGVPGAG

SEQ ID NO: 1833 - protein, 22 aa, Homo sapiens
GFGPGVVGVPGAGVPGVGVPGA

SEQ ID NO: 1834 - protein, 21 aa, Homo sapiens
FGPGVVGVPGAGVPGVGVPGA

SEQ ID NO: 1835 - protein, 18 aa, Homo sapiens
GVPGVGVPGAGIPVVPGA

SEQ ID NO: 1836 - protein, 18 aa, Homo sapiens
GARPGVGVGGIPTYGVGA

SEQ ID NO: 1837 - protein, 21 aa, Homo sapiens
GARPGVGVGGIPTYGVGAGGF

SEQ ID NO: 1838 - protein, 19 aa, Homo sapiens
ARPGVGVGGIPTYGVGAGG

SEQ ID NO: 1839 - protein, 24 aa, Homo sapiens
GGVPGVGGVPGVGISPEAQAAAAA

SEQ ID NO: 1840 - protein, 19 aa, Homo sapiens
GVPGVGISPEAQAAAAAKA

SEQ ID NO: 1841 - protein, 16 aa, Homo sapiens
GVGISPEAQAAAAAKA

SEQ ID NO: 1842 - protein, 25 aa, Homo sapiens
VPGVGVAPGVGVAPGVGVAPGVGLA

SEQ ID NO: 1843 - protein, 30 aa, Homo sapiens
GVAPGVGVAPGVGVAPGVGLAPGVGVAPGV

SEQ ID NO: 1844 - protein, 22 aa, Homo sapiens
GVGVAPGVGVAPGVGLAPGVGV

SEQ ID NO: 1845 - protein, 28 aa, Homo sapiens
GVGVAPGVGVAPGVGLAPGVGVAPGVGV

SEQ ID NO: 1846 - protein, 26 aa, Homo sapiens
APGVGVAPGVGVAPGVGVAPGIGPGG

SEQ ID NO: 1847 - protein, 22 aa, Homo sapiens
GVAPGVGVAPGVGVAPGIGPGG

SEQ ID NO: 1848 - protein, 21 aa, Homo sapiens
AAVPGVLGGLGALGGVGIPGG

SEQ ID NO: 1849 - protein, 23 aa, Homo sapiens
GAAGLGGLGVGGLGVPGVGGLGG

SEQ ID NO: 1850 - protein, 23 aa, Homo sapiens
GGAGVPGVPGAIPGIGGIAGVGT

SEQ ID NO: 1851 - protein, 22 aa, Homo sapiens
GAGVPGVPGAIPGIGGIAGVGT

SEQ ID NO: 1852 - protein, 18 aa, Homo sapiens
AGVGTPAAAAAAAAAAKA

SEQ ID NO: 1853 - protein, 17 aa, Homo sapiens
GVGTPAAAAAAAAAAKA

SEQ ID NO: 1854 - protein, 25 aa, Homo sapiens
GGPGFGPGVVGVPGAGVPGVGVPGA

SEQ ID NO: 1855 - protein, 19 aa, Homo sapiens
GARPGVGVGGIPTYGVGAG

SEQ ID NO: 1856 - protein, 20 aa, Homo sapiens
ARPGVGVGGIPTYGVGAGGF

SEQ ID NO: 1857 - protein, 28 aa, Homo sapiens
GVGVAPGVGVAPGVGVAPGVGLAPGVGV

SEQ ID NO: 1858 - protein, 26 aa, Homo sapiens
APGVGVAPGVGLAPGVGVAPGVGVAP

SEQ ID NO: 1859 - protein, 22 aa, Homo sapiens
GVGVAPGVGLAPGVGVAPGVGV

SEQ ID NO: 1860 - protein, 27 aa, Homo sapiens
LAPGVGVAPGVGVAPGVGVAPGIGPGG

SEQ ID NO: 1861 - protein, 23 aa, Homo sapiens
YGAAVPGVLGGLGALGGVGIPGG

SEQ ID NO: 1862 - protein, 20 aa, Homo sapiens
GGAGQFPLGGVAARPGFGLS

SEQ ID NO: 1863 - protein, 15 aa, Homo sapiens
LVPGGVADAAAAYKA

SEQ ID NO: 1864 - protein, 12 aa, Homo sapiens
VYPGGVLPGARF

SEQ ID NO: 1865 - protein, 26 aa, Homo sapiens
VAPGVGVAPGVGVAPGVGLAPGVGVA

SEQ ID NO: 1866 - protein, 20 aa, Homo sapiens
LAPGVGVAPGVGVAPGVGVA

SEQ ID NO: 1867 - protein, 23 aa, Homo sapiens
LAPGVGVAPGVGVAPGVGVAPGI

SEQ ID NO: 1868 - protein, 25 aa, Homo sapiens
LAPGVGVAPGVGVAPGVGVAPGIGP

SEQ ID NO: 1869 - protein, 26 aa, Homo sapiens
LAPGVGVAPGVGVAPGVGVAPGIGPG

SEQ ID NO: 1870 - protein, 31 aa, Homo sapiens
LAPGVGVAPGVGVAPGVGVAPGIGPGGVAAA

SEQ ID NO: 1871 - protein, 24 aa, Homo sapiens
GVGVAPGVGVAPGVGVAPGIGPGG

SEQ ID NO: 1872 - protein, 23 aa, Homo sapiens
GAAVPGVLGGLGALGGVGIPGGV

SEQ ID NO: 1873 - protein, 21 aa, Homo sapiens
AAVPGVLGGLGALGGVGIPGG

SEQ ID NO: 1874 - protein, 21 aa, Homo sapiens
AVPGVLGGLGALGGVGIPGGV

SEQ ID NO: 1875 - protein, 18 aa, Homo sapiens
AGQFPLGGVAARPGFGLS

SEQ ID NO: 1876 - protein, 17 aa, Homo sapiens
GALVPGGVADAAAAYKA

SEQ ID NO: 1877 - protein, 17 aa, Homo sapiens
GLPYTTGKLPYGYGPGG

SEQ ID NO: 1878 - protein, 16 aa, Homo sapiens
AAAAAAAKAAAKFGAG

SEQ ID NO: 1879 - protein, 18 aa, Homo sapiens
AAAAAAAAAAKAAKYGAA

SEQ ID NO: 1880 - protein, 26 aa, Homo sapiens
GVAPGVGVAPGVGVAPGVGLAPGVGV

SEQ ID NO: 1881 - protein, 20 aa, Homo sapiens
TFPGALVPGGVADAAAAYKA

SEQ ID NO: 1882 - protein, 21 aa, Homo sapiens
GLPGVYPGGVLPGARFPGVGV

SEQ ID NO: 1883 - protein, 20 aa, Homo sapiens
GYPTGTGVGPQAAAAAAAKA

SEQ ID NO: 1884 - protein, 18 aa, Homo sapiens
GTPAAAAAAAAAAKAAKY

SEQ ID NO: 1885 - protein, 22 aa, Homo sapiens
GVPGAGVPGVGVPGAGIPVVPG

SEQ ID NO: 1886 - protein, 28 aa, Homo sapiens
GVPGAGVPGVGVPGAGIPVVPGAGIPGA

SEQ ID NO: 1887 - protein, 17 aa, Homo sapiens
GISPEAQAAAAAKAAKY

SEQ ID NO: 1888 - protein, 20 aa, Homo sapiens
VPGVGVAPGVGVAPGVGVAP

SEQ ID NO: 1889 - protein, 25 aa, Homo sapiens
GVAPGVGVAPGVGVAPGIGPGGVAA

SEQ ID NO: 1890 - protein, 20 aa, Homo sapiens
GIPGGVVGAGPAAAAAAAKA

SEQ ID NO: 1891 - protein, 23 aa, Homo sapiens
GGVLPGARFPGVGVLPGVPTGAG

SEQ ID NO: 1892 - protein, 19 aa, Homo sapiens
GGVPGVGGVPGVGISPEAQ

SEQ ID NO: 1893 - protein, 22 aa, Homo sapiens
GVGVAPGVGVAPGVGVAPGVGL

SEQ ID NO: 1894 - protein, 20 aa, Homo sapiens
GVPGVPGAIPGIGGIAGVGT

SEQ ID NO: 1895 - protein, 22 aa, Homo sapiens
FGPGVVGVPGAGVPGVGVPGAG

SEQ ID NO: 1896 - protein, 19 aa, Homo sapiens
GVPGVGVPGAGIPVVPGAG

SEQ ID NO: 1897 - protein, 19 aa, Homo sapiens
GVGVAPGVGVAPGVGVAPG

SEQ ID NO: 1898 - protein, 6 aa, Homo sapiens
GVPGAI

SEQ ID NO: 1899 - protein, 6 aa, Homo sapiens
AIPGGV

SEQ ID NO: 1900 - protein, 6 aa, Homo sapiens
GVPGGV

SEQ ID NO: 1901 - protein, 6 aa, Homo sapiens
ALGGGA

SEQ ID NO: 1902 - protein, 6 aa, Homo sapiens
LGGGAL

SEQ ID NO: 1903 - protein, 6 aa, Homo sapiens
GGALGP

SEQ ID NO: 1904 - protein, 6 aa, Homo sapiens
PLKPVP

SEQ ID NO: 1905 - protein, 6 aa, Homo sapiens
LKPVPG

SEQ ID NO: 1906 - protein, 6 aa, Homo sapiens
GLAGAG

SEQ ID NO: 1907 - protein, 6 aa, Homo sapiens
GLGAGL

SEQ ID NO: 1908 - protein, 6 aa, Homo sapiens
LGAGLG

SEQ ID NO: 1909 - protein, 6 aa, Homo sapiens
AGLGAF

SEQ ID NO: 1910 - protein, 6 aa, Homo sapiens
LVPGGV

SEQ ID NO: 1911 - protein, 6 aa, Homo sapiens
VADAAA

SEQ ID NO: 1912 - protein, 6 aa, Homo sapiens
KAAKAG

SEQ ID NO: 1913 - protein, 6 aa, Homo sapiens
PVGYPG

SEQ ID NO: 1914 - protein, 6 aa, Homo sapiens
ARFPGV

SEQ ID NO: 1915 - protein, 6 aa, Homo sapiens
RFPGVG

SEQ ID NO: 1916 - protein, 6 aa, Homo sapiens
VGPFGG

SEQ ID NO: 1917 - protein, 6 aa, Homo sapiens
GPQPGV

SEQ ID NO: 1918 - protein, 6 aa, Homo sapiens
PQPGVP

SEQ ID NO: 1919 - protein, 6 aa, Homo sapiens
TTGKLP

SEQ ID NO: 1920 - protein, 6 aa, Homo sapiens
LPYGYG

SEQ ID NO: 1921 - protein, 6 aa, Homo sapiens
GYGPGG

SEQ ID NO: 1922 - protein, 6 aa, Homo sapiens
FGAGAA

SEQ ID NO: 1923 - protein, 6 aa, Homo sapiens
GVLPGV

SEQ ID NO: 1924 - protein, 6 aa, Homo sapiens
VLPGVG

SEQ ID NO: 1925 - protein, 6 aa, Homo sapiens
AGIPGL

SEQ ID NO: 1926 - protein, 6 aa, Homo sapiens
VPGAIP

SEQ ID NO: 1927 - protein, 6 aa, Homo sapiens
AIPGIG

SEQ ID NO: 1928 - protein, 6 aa, Homo sapiens
TPAAAA

SEQ ID NO: 1929 - protein, 6 aa, Homo sapiens
PAAAAA

SEQ ID NO: 1930 - protein, 6 aa, Homo sapiens
AAAAAA

SEQ ID NO: 1931 - protein, 6 aa, Homo sapiens
VGVPGA

SEQ ID NO: 1932 - protein, 6 aa, Homo sapiens
AVGPGV

SEQ ID NO: 1933 - protein, 6 aa, Homo sapiens
GVPGVG

SEQ ID NO: 1934 - protein, 6 aa, Homo sapiens
GIPVVP

SEQ ID NO: 1935 - protein, 6 aa, Homo sapiens
IPGAAV

SEQ ID NO: 1936 - protein, 6 aa, Homo sapiens
GAAVPG

SEQ ID NO: 1937 - protein, 6 aa, Homo sapiens
ARPGVG

SEQ ID NO: 1938 - protein, 6 aa, Homo sapiens
RPGVGV

SEQ ID NO: 1939 - protein, 6 aa, Homo sapiens
VGGIPT

SEQ ID NO: 1940 - protein, 6 aa, Homo sapiens
SVGGVP

SEQ ID NO: 1941 - protein, 6 aa, Homo sapiens
VGGVPG

SEQ ID NO: 1942 - protein, 6 aa, Homo sapiens
GVGTPA

SEQ ID NO: 1943 - protein, 6 aa, Homo sapiens
VGVAPG

SEQ ID NO: 1944 - protein, 6 aa, Homo sapiens
VAPGVG

SEQ ID NO: 1945 - protein, 6 aa, Homo sapiens
GVAPGV

SEQ ID NO: 1946 - protein, 6 aa, Homo sapiens
GVPVAP

SEQ ID NO: 1947 - protein, 6 aa, Homo sapiens
GAGIPG

SEQ ID NO: 1948 - protein, 6 aa, Homo sapiens
PGGVAA

SEQ ID NO: 1949 - protein, 6 aa, Homo sapiens
LGAGIP

SEQ ID NO: 1950 - protein, 6 aa, Homo sapiens
PGFGPG

SEQ ID NO: 1951 - protein, 6 aa, Homo sapiens
PGVVGV

SEQ ID NO: 1952 - protein, 6 aa, Homo sapiens
PGALAA

SEQ ID NO: 1953 - protein, 6 aa, Homo sapiens
AKYGAA

SEQ ID NO: 1954 - protein, 6 aa, Homo sapiens
YGAAVP

SEQ ID NO: 1955 - protein, 6 aa, Homo sapiens
ALGGVG

SEQ ID NO: 1956 - protein, 6 aa, Homo sapiens
LGGVGI

SEQ ID NO: 1957 - protein, 6 aa, Homo sapiens
GVGIPG

SEQ ID NO: 1958 - protein, 6 aa, Homo sapiens
AGPAAA

SEQ ID NO: 1959 - protein, 6 aa, Homo sapiens
GPAAAA

SEQ ID NO: 1960 - protein, 6 aa, Homo sapiens
FGLVGA

SEQ ID NO: 1961 - protein, 6 aa, Homo sapiens
GLGVPG

SEQ ID NO: 1962 - protein, 6 aa, Homo sapiens
LGGIPP

SEQ ID NO: 1963 - protein, 6 aa, Homo sapiens
LGGVLG

SEQ ID NO: 1964 - protein, 6 aa, Homo sapiens
PLGGVA

SEQ ID NO: 1965 - protein, 6 aa, Homo sapiens
LGGVAA

SEQ ID NO: 1966 - protein, 6 aa, Homo sapiens
GGVAAR

SEQ ID NO: 1967 - protein, 6 aa, Homo sapiens
GVGLPG

SEQ ID NO: 1968 - protein, 6 aa, Homo sapiens
VGLPGV

SEQ ID NO: 1969 - protein, 6 aa, Homo sapiens
LPGVYP

SEQ ID NO: 1970 - protein, 6 aa, Homo sapiens
VPGVPV

SEQ ID NO: 1971 - protein, 6 aa, Homo sapiens
VPGVGI

SEQ ID NO: 1972 - protein, 6 aa, Homo sapiens
VGISPE

SEQ ID NO: 1973 - protein, 6 aa, Homo sapiens
APGVGV

SEQ ID NO: 1974 - protein, 6 aa, Homo sapiens
VPGGVA

SEQ ID NO: 1975 - protein, 6 aa, Homo sapiens
YPGGVL

SEQ ID NO: 1976 - protein, 6 aa, Homo sapiens
GPGFGP

SEQ ID NO: 1977 - protein, 6 aa, Homo sapiens
YPTGTG

SEQ ID NO: 1978 - protein, 6 aa, Homo sapiens
VPGAGV

SEQ ID NO: 1979 - protein, 6 aa, Homo sapiens
VPGGVF

SEQ ID NO: 1980 - protein, 6 aa, Homo sapiens
GVFYPG

SEQ ID NO: 1981 - protein, 6 aa, Homo sapiens
VFYPGA

SEQ ID NO: 1982 - protein, 6 aa, Homo sapiens
LGPGGK

SEQ ID NO: 1983 - protein, 6 aa, Homo sapiens
GPGGKP

SEQ ID NO: 1984 - protein, 6 aa, Homo sapiens
PGGKPL

SEQ ID NO: 1985 - protein, 6 aa, Homo sapiens
LAGAGL

SEQ ID NO: 1986 - protein, 6 aa, Homo sapiens
AGAGLG

SEQ ID NO: 1987 - protein, 6 aa, Homo sapiens
GAGLGA

SEQ ID NO: 1988 - protein, 6 aa, Homo sapiens
LGAFPA

SEQ ID NO: 1989 - protein, 6 aa, Homo sapiens
AFPAVT

SEQ ID NO: 1990 - protein, 6 aa, Homo sapiens
AVTFPG

SEQ ID NO: 1991 - protein, 6 aa, Homo sapiens
LGVSAG

SEQ ID NO: 1992 - protein, 6 aa, Homo sapiens
VPGVGL

SEQ ID NO: 1993 - protein, 6 aa, Homo sapiens
PGVGLP

SEQ ID NO: 1994 - protein, 6 aa, Homo sapiens
FPGVGV

SEQ ID NO: 1995 - protein, 6 aa, Homo sapiens
KPGAPG

SEQ ID NO: 1996 - protein, 6 aa, Homo sapiens
PGVPLG

SEQ ID NO: 1997 - protein, 6 aa, Homo sapiens
GYPIKA

SEQ ID NO: 1998 - protein, 6 aa, Homo sapiens
PKLPGG

SEQ ID NO: 1999 - protein, 6 aa, Homo sapiens
YGPGGV

SEQ ID NO: 2000 - protein, 6 aa, Homo sapiens
AGYPTG

SEQ ID NO: 2001 - protein, 6 aa, Homo sapiens
TGVGPQ

SEQ ID NO: 2002 - protein, 6 aa, Homo sapiens
GAGVPG

SEQ ID NO: 2003 - protein, 6 aa, Homo sapiens
AGVPGV

SEQ ID NO: 2004 - protein, 6 aa, Homo sapiens
GVPGVP

SEQ ID NO: 2005 - protein, 6 aa, Homo sapiens
IPGIGG

SEQ ID NO: 2006 - protein, 6 aa, Homo sapiens
IGGIAG

SEQ ID NO: 2007 - protein, 6 aa, Homo sapiens
GIAGVG

SEQ ID NO: 2008 - protein, 6 aa, Homo sapiens
VPGVGV

SEQ ID NO: 2009 - protein, 6 aa, Homo sapiens
VPVGVA

SEQ ID NO: 2010 - protein, 6 aa, Homo sapiens
VPGAGI

SEQ ID NO: 2011 - protein, 6 aa, Homo sapiens
AVPGVV

SEQ ID NO: 2012 - protein, 6 aa, Homo sapiens
VPGVVS

SEQ ID NO: 2013 - protein, 6 aa, Homo sapiens
YGARPG

SEQ ID NO: 2014 - protein, 6 aa, Homo sapiens
GVGAGG

SEQ ID NO: 2015 - protein, 6 aa, Homo sapiens
VGAGGF

SEQ ID NO: 2016 - protein, 6 aa, Homo sapiens
VGVGGI

SEQ ID NO: 2017 - protein, 6 aa, Homo sapiens
FGLVPG

SEQ ID NO: 2018 - protein, 6 aa, Homo sapiens
GLVPGV

SEQ ID NO: 2019 - protein, 6 aa, Homo sapiens
LVPGVG

SEQ ID NO: 2020 - protein, 6 aa, Homo sapiens
PGVGLA

SEQ ID NO: 2021 - protein, 6 aa, Homo sapiens
GVGLAP

SEQ ID NO: 2022 - protein, 6 aa, Homo sapiens
VGLAPG

SEQ ID NO: 2023 - protein, 6 aa, Homo sapiens
LRAAAG

SEQ ID NO: 2024 - protein, 6 aa, Homo sapiens
LVGAAG

SEQ ID NO: 2025 - protein, 6 aa, Homo sapiens
LVPGGP

SEQ ID NO: 2026 - protein, 6 aa, Homo sapiens
GIPGLG

SEQ ID NO: 2027 - protein, 6 aa, Homo sapiens
LGVGVG

SEQ ID NO: 2028 - protein, 6 aa, Homo sapiens
VGVPGL

SEQ ID NO: 2029 - protein, 6 aa, Homo sapiens
AAAGLG

SEQ ID NO: 2030 - protein, 6 aa, Homo sapiens
AVPGVL

SEQ ID NO: 2031 - protein, 6 aa, Homo sapiens
VLGGLG

SEQ ID NO: 2032 - protein, 6 aa, Homo sapiens
VGIPGG

SEQ ID NO: 2033 - protein, 6 aa, Homo sapiens
IPGGVV

SEQ ID NO: 2034 - protein, 6 aa, Homo sapiens
VVGAGP

SEQ ID NO: 2035 - protein, 6 aa, Homo sapiens
GLVGAA

SEQ ID NO: 2036 - protein, 6 aa, Homo sapiens
VGAAGL

SEQ ID NO: 2037 - protein, 6 aa, Homo sapiens
LGGLGV

SEQ ID NO: 2038 - protein, 6 aa, Homo sapiens
GGVLGG

SEQ ID NO: 2039 - protein, 6 aa, Homo sapiens
GAGQFP

SEQ ID NO: 2040 - protein, 6 aa, Homo sapiens
AFQFPL

SEQ ID NO: 2041 - protein, 6 aa, Homo sapiens
GVAARP

SEQ ID NO: 2042 - protein, 6 aa, Homo sapiens
VAARPG

SEQ ID NO: 2043 - protein, 6 aa, Homo sapiens
RPGFGL

SEQ ID NO: 2044 - protein, 6 aa, Homo sapiens
GVYPGG

SEQ ID NO: 2045 - protein, 6 aa, Homo sapiens
LPYTTG

SEQ ID NO: 2046 - protein, 6 aa, Homo sapiens
FGPGVV

SEQ ID NO: 2047 - protein, 6 aa, Homo sapiens
AAVPGV

SEQ ID NO: 2048 - protein, 6 aa, Homo sapiens
AAGLGG

SEQ ID NO: 2049 - protein, 6 aa, Homo sapiens
FPGALV

SEQ ID NO: 2050 - protein, 6 aa, Homo sapiens
VPGVLG

SEQ ID NO: 2051 - protein, 6 aa, Homo sapiens
GQFPLG

SEQ ID NO: 2052 - protein, 6 aa, Homo sapiens
ALVPGG

SEQ ID NO: 2053 - protein, 6 aa, Homo sapiens
ISPEAQ

SEQ ID NO: 2054 - protein, 6 aa, Homo sapiens
GVLPGA

SEQ ID NO: 2055 - protein, 6 aa, Homo sapiens
VGAGVP

SEQ ID NO: 2056 - protein, 6 aa, Homo sapiens
LGALGG

SEQ ID NO: 2057 - protein, 6 aa, Homo sapiens
VPGVPG

SEQ ID NO: 2058 - protein, 6 aa, Homo sapiens
GGLGAL

SEQ ID NO: 2059 - protein, 6 aa, Homo sapiens
GKPLKP

SEQ ID NO: 2060 - protein, 6 aa, Homo sapiens
IAGVGT

SEQ ID NO: 2061 - protein, 6 aa, Homo sapiens
VGAGPA

SEQ ID NO: 2062 - protein, 6 aa, Homo sapiens
AGLGAG

SEQ ID NO: 2063 - protein, 6 aa, Homo sapiens
VVGVPG

SEQ ID NO: 2064 - protein, 6 aa, Homo sapiens
LGVGGL

SEQ ID NO: 2065 - protein, 6 aa, Homo sapiens
VTFPGA

SEQ ID NO: 2066 - protein, 6 aa, Homo sapiens
AGIPVV

SEQ ID NO: 2067 - protein, 6 aa, Homo sapiens
FPLGGV

SEQ ID NO: 2068 - protein, 6 aa, Homo sapiens
GLPGVY

SEQ ID NO: 2069 - protein, 6 aa, Homo sapiens
GARPGV

SEQ ID NO: 2070 - protein, 6 aa, Homo sapiens
PGFGLS

SEQ ID NO: 2071 - protein, 6 aa, Homo sapiens
GAFAGI

SEQ ID NO: 2072 - protein, 6 aa, Homo sapiens
VAGVPS

SEQ ID NO: 2073 - protein, 6 aa, Homo sapiens
GPGVVG

SEQ ID NO: 2074 - protein, 6 aa, Homo sapiens
YTTGKL

SEQ ID NO: 2075 - protein, 6 aa, Homo sapiens
PGVGVA

SEQ ID NO: 2076 - protein, 6 aa, Homo sapiens
VGTPAA

SEQ ID NO: 2077 - protein, 6 aa, Homo sapiens
PQAAAA

SEQ ID NO: 2078 - protein, 6 aa, Homo sapiens
LAPGVG

SEQ ID NO: 2079 - protein, 6 aa, Homo sapiens
PGGVPG

SEQ ID NO: 2080 - protein, 6 aa, Homo sapiens
PGAGLG

SEQ ID NO: 2081 - protein, 6 aa, Homo sapiens
GALGGG

SEQ ID NO: 2082 - protein, 6 aa, Homo sapiens
GGGALG

SEQ ID NO: 2083 - protein, 6 aa, Homo sapiens
GLGAFP

SEQ ID NO: 2084 - protein, 6 aa, Homo sapiens
ADAAAA

SEQ ID NO: 2085 - protein, 6 aa, Homo sapiens
PGVLGG

SEQ ID NO: 2086 - protein, 6 aa, Homo sapiens
VGVLPG

SEQ ID NO: 2087 - protein, 6 aa, Homo sapiens
VPTGAG

SEQ ID NO: 2088 - protein, 6 aa, Homo sapiens
GVGPFG

SEQ ID NO: 2089 - protein, 6 aa, Homo sapiens
VPLGYP

SEQ ID NO: 2090 - protein, 6 aa, Homo sapiens
AAAAAK

SEQ ID NO: 2091 - protein, 6 aa, Homo sapiens
AAAAKA

SEQ ID NO: 2092 - protein, 6 aa, Homo sapiens
GVGVPG

SEQ ID NO: 2093 - protein, 6 aa, Homo sapiens
PVVPGA

SEQ ID NO: 2094 - protein, 6 aa, Homo sapiens
VVSPEA

SEQ ID NO: 2095 - protein, 6 aa, Homo sapiens
GGIPTY

SEQ ID NO: 2096 - protein, 6 aa, Homo sapiens
GIPTYG

SEQ ID NO: 2097 - protein, 6 aa, Homo sapiens
GVGVGG

SEQ ID NO: 2098 - protein, 6 aa, Homo sapiens
GVGGIP

SEQ ID NO: 2099 - protein, 6 aa, Homo sapiens
GFPGFG

SEQ ID NO: 2100 - protein, 6 aa, Homo sapiens
FGVGVG

SEQ ID NO: 2101 - protein, 6 aa, Homo sapiens
PGVGIS

SEQ ID NO: 2102 - protein, 6 aa, Homo sapiens
SPEAQA

SEQ ID NO: 2103 - protein, 6 aa, Homo sapiens
GVGVAP

SEQ ID NO: 2104 - protein, 6 aa, Homo sapiens
APGVGL

SEQ ID NO: 2105 - protein, 6 aa, Homo sapiens
GIGPGG

SEQ ID NO: 2106 - protein, 6 aa, Homo sapiens
APGIGP

SEQ ID NO: 2107 - protein, 6 aa, Homo sapiens
VAPGIG

SEQ ID NO: 2108 - protein, 6 aa, Homo sapiens
RAAAGL

SEQ ID NO: 2109 - protein, 6 aa, Homo sapiens
AAGLGA

SEQ ID NO: 2110 - protein, 6 aa, Homo sapiens
GVPGLG

SEQ ID NO: 2111 - protein, 6 aa, Homo sapiens
GVPGFG

SEQ ID NO: 2112 - protein, 6 aa, Homo sapiens
AGVPGL

SEQ ID NO: 2113 - protein, 6 aa, Homo sapiens
GAGPAA

SEQ ID NO: 2114 - protein, 6 aa, Homo sapiens
VPGVGG

SEQ ID NO: 2115 - protein, 6 aa, Homo sapiens
GLGGLG

SEQ ID NO: 2116 - protein, 6 aa, Homo sapiens
PGVGGL

SEQ ID NO: 2117 - protein, 6 aa, Homo sapiens
PAAAAK

SEQ ID NO: 2118 - protein, 6 aa, Homo sapiens
AARPGF

SEQ ID NO: 2119 - protein, 6 aa, Homo sapiens
LSPIFP

SEQ ID NO: 2120 - protein, 6 aa, Homo sapiens
AQAAAA

SEQ ID NO: 2121 - protein, 6 aa, Homo sapiens
GPGIPG

SEQ ID NO: 2122 - protein, 6 aa, Homo sapiens
GPGGVA

SEQ ID NO: 2123 - protein, 6 aa, Homo sapiens
GLGALG

SEQ ID NO: 2124 - protein, 6 aa, Homo sapiens
ALGPGG

SEQ ID NO: 2125 - protein, 6 aa, Homo sapiens
GALGPG

SEQ ID NO: 2126 - protein, 6 aa, Homo sapiens
VAPVGV

SEQ ID NO: 2127 - protein, 6 aa, Homo sapiens
KPVPGG

SEQ ID NO: 2128 - protein, 6 aa, Homo sapiens
AAAAYK

SEQ ID NO: 2129 - protein, 6 aa, Homo sapiens
AAKAGA

SEQ ID NO: 2130 - protein, 6 aa, Homo sapiens
VPQPGA

SEQ ID NO: 2131 - protein, 6 aa, Homo sapiens
PGVPTG

SEQ ID NO: 2132 - protein, 6 aa, Homo sapiens
GVPTGA

SEQ ID NO: 2133 - protein, 6 aa, Homo sapiens
AGVKPK

SEQ ID NO: 2134 - protein, 6 aa, Homo sapiens
PIKAPK

SEQ ID NO: 2135 - protein, 6 aa, Homo sapiens
KLPGGY

SEQ ID NO: 2136 - protein, 6 aa, Homo sapiens
YGYGPG

SEQ ID NO: 2137 - protein, 6 aa, Homo sapiens
GIGGIA

SEQ ID NO: 2138 - protein, 6 aa, Homo sapiens
GTPAAA

SEQ ID NO: 2139 - protein, 6 aa, Homo sapiens
IPVVPG

SEQ ID NO: 2140 - protein, 6 aa, Homo sapiens
GVPGAG

SEQ ID NO: 2141 - protein, 6 aa, Homo sapiens
PEAAAK

SEQ ID NO: 2142 - protein, 6 aa, Homo sapiens
PTYGVG

SEQ ID NO: 2143 - protein, 6 aa, Homo sapiens
TYGVGA

SEQ ID NO: 2144 - protein, 6 aa, Homo sapiens
YGVGAG

SEQ ID NO: 2145 - protein, 6 aa, Homo sapiens
IPTYGV

SEQ ID NO: 2146 - protein, 6 aa, Homo sapiens
PGAIPG

SEQ ID NO: 2147 - protein, 6 aa, Homo sapiens
AGGFPG

SEQ ID NO: 2148 - protein, 6 aa, Homo sapiens
GIPGVA

SEQ ID NO: 2149 - protein, 6 aa, Homo sapiens
GISPEA

SEQ ID NO: 2150 - protein, 6 aa, Homo sapiens
VPGAPG

SEQ ID NO: 2151 - protein, 6 aa, Homo sapiens
GGVAAA

SEQ ID NO: 2152 - protein, 6 aa, Homo sapiens
PGIGPG

SEQ ID NO: 2153 - protein, 6 aa, Homo sapiens
GLGVGG

SEQ ID NO: 2154 - protein, 6 aa, Homo sapiens
PGLGVG

SEQ ID NO: 2155 - protein, 6 aa, Homo sapiens
GLGVGA

SEQ ID NO: 2156 - protein, 6 aa, Homo sapiens
ALAAAK

SEQ ID NO: 2157 - protein, 6 aa, Homo sapiens
LGGLGA

SEQ ID NO: 2158 - protein, 6 aa, Homo sapiens
GGLGVG

SEQ ID NO: 2159 - protein, 6 aa, Homo sapiens
GVGGLG

SEQ ID NO: 2160 - protein, 6 aa, Homo sapiens
AGQFPL

SEQ ID NO: 2161 - protein, 6 aa, Homo sapiens
GFGLSP

SEQ ID NO: 2162 - protein, 6 aa, Homo sapiens
PIFPGG

SEQ ID NO: 2163 - protein, 6 aa, Homo sapiens
IFPGGA

SEQ ID NO: 2164 - protein, 6 aa, Homo sapiens
AAKFGA

SEQ ID NO: 2165 - protein, 6 aa, Homo sapiens
AAKYGA

SEQ ID NO: 2166 - protein, 6 aa, Homo sapiens
AAKAAK

SEQ ID NO: 2167 - protein, 6 aa, Homo sapiens
AGLGAL

SEQ ID NO: 2168 - protein, 6 aa, Homo sapiens
GIPGGV

SEQ ID NO: 2169 - protein, 6 aa, Homo sapiens
PGVGVG

SEQ ID NO: 2170 - protein, 6 aa, Homo sapiens
IPPAAA

SEQ ID NO: 2171 - protein, 6 aa, Homo sapiens
ARPGFG

SEQ ID NO: 2172 - protein, 6 aa, Homo sapiens
VLPGAR

SEQ ID NO: 2173 - protein, 6 aa, Homo sapiens
GGFPGF

SEQ ID NO: 2174 - protein, 6 aa, Homo sapiens
GLSPIF

SEQ ID NO: 2175 - protein, 6 aa, Homo sapiens
PTGAGV

SEQ ID NO: 2176 - protein, 6 aa, Homo sapiens
AGAAGK

SEQ ID NO: 2177 - protein, 10 aa, Homo sapiens
RLRSSVPGVR

SEQ ID NO: 2178 - protein, 10 aa, Homo sapiens
RLRSSVPGVL

SEQ ID NO: 2179 - protein, 10 aa, Homo sapiens
LLQDSVDFSL

SEQ ID NO: 2180 - protein, 10 aa, Homo sapiens
FADLSEAANR

SEQ ID NO: 2181 - protein, 10 aa, Homo sapiens
ISLPLPTFSS

SEQ ID NO: 2182 - protein, 6 aa, Homo sapiens
LLQDSV

SEQ ID NO: 2183 - protein, 6 aa, Homo sapiens
FADLSE

SEQ ID NO: 2184 - protein, 6 aa, Homo sapiens
ISLPLP

SEQ ID NO: 2185 - protein, 6 aa, Homo sapiens
SVPGVR

SEQ ID NO: 2186 - protein, 6 aa, Homo sapiens
SVPGVL

SEQ ID NO: 2187 - protein, 6 aa, Homo sapiens
GPPGIC

SEQ ID NO: 2188 - protein, 6 aa, Homo sapiens
LPGAAG

SEQ ID NO: 2189 - protein, 6 aa, Homo sapiens
APGPLG

SEQ ID NO: 2190 - protein, 9 aa, Homo sapiens
ILGHVPGML

SEQ ID NO: 2191 - protein, 17 aa, Homo sapiens
PGLPGQPGPPGLPVPGQ

SEQ ID NO: 2192 - protein, 42 aa, Homo sapiens
SGYPGNPGLPGIPGQDGPPGPPGIPGCNGTKGERGPLGPPGL

SEQ ID NO: 2193 - protein, 11 aa, Homo sapiens
VSGPPGVPGQA

SEQ ID NO: 2194 - protein, 12 aa, Homo sapiens
VSGPPGVPGQAQ

SEQ ID NO: 2195 - protein, 20 aa, Homo sapiens
KRGPPGPPGLPGPPGPDGFL

SEQ ID NO: 2196 - protein, 15 aa, Homo sapiens
LHGFPGAPGQEGPLG

SEQ ID NO: 2197 - protein, 18 aa, Homo sapiens
LPGPDGPPGERGLPGEVL

SEQ ID NO: 2198 - protein, 7 aa, Homo sapiens
LRGIPGF

SEQ ID NO: 2199 - protein, 21 aa, Homo sapiens
PGFPGAPGTVGAPGIAGIPQK

SEQ ID NO: 2200 - protein, 9 aa, Homo sapiens
QQGNRGLGF

SEQ ID NO: 2201 - protein, 14 aa, Homo sapiens
VGQPGPNGIPSDTL

SEQ ID NO: 2202 - protein, 43 aa, Homo sapiens
GEPGMQGEPGPPGPPGNLGPCGPRGKPGKDGKPGTPGPAGEKG

SEQ ID NO: 2203 - protein, 39 aa, Homo sapiens
GEPGPPGPPGNLGPCGPRGKPGKDGKPGTPGPAGEKGNK

SEQ ID NO: 2204 - protein, 23 aa, Homo sapiens
PGIPGTPGPPGLPGLQGPVGPPG

SEQ ID NO: 2205 - protein, 8 aa, Homo sapiens
PGDIVFRK

SEQ ID NO: 2206 - protein, 17 aa, Homo sapiens
GNKGDPASHFGPPGPKG

SEQ ID NO: 2207 - protein, 9 aa, Homo sapiens
PGPRGKPGM

SEQ ID NO: 2208 - protein, 12 aa, Homo sapiens
PGLPGQPGTRGL

SEQ ID NO: 2209 - protein, 40 aa, Homo sapiens
PGPPGPLGIPGRSGVPGLKGDDGLQGQPGLPGPTGEKGSK

SEQ ID NO: 2210 - protein, 41 aa, Homo sapiens
PGPPGPLGIPGRSGVPGLKGDDGLQGQPGLPGPTGEKGSKG

SEQ ID NO: 2211 - protein, 40 aa, Homo sapiens
SKGEKGEPGLPGIPGVSGPKGYQGLPGDPGQPGLSGQPGL

SEQ ID NO: 2212 - protein, 6 aa, Homo sapiens
ILGHVP

SEQ ID NO: 2213 - protein, 6 aa, Homo sapiens
PGLPGQ

SEQ ID NO: 2214 - protein, 6 aa, Homo sapiens
LPGPDG

SEQ ID NO: 2215 - protein, 6 aa, Homo sapiens
PGDIVF

SEQ ID NO: 2216 - protein, 6 aa, Homo sapiens
GNKGDP

SEQ ID NO: 2217 - protein, 6 aa, Homo sapiens
SGYPGN

SEQ ID NO: 2218 - protein, 6 aa, Homo sapiens
PGFPGA

SEQ ID NO: 2219 - protein, 6 aa, Homo sapiens
PGPRGK

SEQ ID NO: 2220 - protein, 6 aa, Homo sapiens
VSGPPG

SEQ ID NO: 2221 - protein, 6 aa, Homo sapiens
QQGNRG

SEQ ID NO: 2222 - protein, 6 aa, Homo sapiens
VGQPGP

SEQ ID NO: 2223 - protein, 6 aa, Homo sapiens
KRGPPG

SEQ ID NO: 2224 - protein, 6 aa, Homo sapiens
GEPGMQ

SEQ ID NO: 2225 - protein, 6 aa, Homo sapiens
LHGFPG

SEQ ID NO: 2226 - protein, 6 aa, Homo sapiens
SKGEKG

SEQ ID NO: 2227 - protein, 6 aa, Homo sapiens
PGIPGT

SEQ ID NO: 2228 - protein, 6 aa, Homo sapiens
HVPGML

SEQ ID NO: 2229 - protein, 6 aa, Homo sapiens
LPVPGQ

SEQ ID NO: 2230 - protein, 6 aa, Homo sapiens
LGPPGL

SEQ ID NO: 2231 - protein, 6 aa, Homo sapiens
GVPGQA

SEQ ID NO: 2232 - protein, 6 aa, Homo sapiens
VPGQAQ

SEQ ID NO: 2233 - protein, 6 aa, Homo sapiens
GPDGFL

SEQ ID NO: 2234 - protein, 6 aa, Homo sapiens
QEGPLG

SEQ ID NO: 2235 - protein, 6 aa, Homo sapiens
LPGEVL

SEQ ID NO: 2236 - protein, 6 aa, Homo sapiens
RGIPGF

SEQ ID NO: 2237 - protein, 6 aa, Homo sapiens
AGIPQK

SEQ ID NO: 2238 - protein, 6 aa, Homo sapiens
NRGLGF

SEQ ID NO: 2239 - protein, 6 aa, Homo sapiens
IPSDTL

SEQ ID NO: 2240 - protein, 6 aa, Homo sapiens
PAGEKG

SEQ ID NO: 2241 - protein, 6 aa, Homo sapiens
GEKGNK

SEQ ID NO: 2242 - protein, 6 aa, Homo sapiens
PVGPPG

SEQ ID NO: 2243 - protein, 6 aa, Homo sapiens
DIVFRK

SEQ ID NO: 2244 - protein, 6 aa, Homo sapiens
RGKPGM

SEQ ID NO: 2245 - protein, 6 aa, Homo sapiens
PGTRGL

SEQ ID NO: 2246 - protein, 6 aa, Homo sapiens
GEKGSK

SEQ ID NO: 2247 - protein, 6 aa, Homo sapiens
EKGSKG

SEQ ID NO: 2248 - protein, 6 aa, Homo sapiens
SGQPGL